European Patent Application EP 4 516 897 A1, published March 5, 2025. Title: NUCLEIC ACID CONSTRUCT AND USE THEREOF. Applicant: RETROLEAD (SHANGHAI) BIOPHARMA CO., LTD. Application WO PCT/CN2023/091194, filed April 27, 2023. The sequence listing filed with the application follows.

SEQUENCE LISTING (196 sequences)

SEQ ID NO: 1 - DNA, 63 bp, synthetic construct
  source 1..63: mol_type = other DNA; note = 5'UTR I
gagttaggagttgatggcagtttcaataacaggtcattgccgagaaaaggatagcactataat

SEQ ID NO: 2 - DNA, 63 bp, synthetic construct
  source 1..63: mol_type = other DNA; note = 5'UTR I'
gagttaggagttggtggcagtttcaataacaggtcattgccgagaaaaggatagcactataat

SEQ ID NO: 3 - DNA, 43 bp, synthetic construct
  source 1..43: mol_type = other DNA; note = 5'UTR G
gcacttttctgagcagacgtccagagcagagtcagccgccacc

SEQ ID NO: 4 - DNA, 52 bp, synthetic construct
  source 1..52: mol_type = other DNA; note = 5'UTR A
acatttgcttctgacacaactgtgttcactagcaacctcaaacgccgccacc

SEQ ID NO: 5 - DNA, 55 bp, synthetic construct
  source 1..55: mol_type = other DNA; note = 5'UTR J
agagaggcaaagaaacattgtgaaatctccaactcttaaccttcaagccgccacc

SEQ ID NO: 6 - DNA, 52 bp, synthetic construct
  source 1..52: mol_type = other DNA; note = 5'UTR BNT162b2
gaataaactagtattcttctggtccccacagactcagagagaacccgccacc

SEQ ID NO: 7 - DNA, 134 bp, synthetic construct
  source 1..134: mol_type = other DNA; note = 3'UTR B
gctcgctttcttgctgtccaatttctattaaaggttcctttgttccctaagtccaactactaaactgggggatattatgaagggccttgagcatctggattctgcctaataaaaaacatttattttcattgcaa

SEQ ID NO: 8 - DNA, 180 bp, synthetic construct
  source 1..180: mol_type = other DNA; note = 3'UTR F
cagacaagacaagctactgaatacgttcacatctgtcttgatgcctaatatttttacatttctgtaaacatatttctgaaatattttttgcctttcaagcgacagatgcctcattttgtgaaaacttaatgatgattttgtgtttaagttccaaacatttgaataaaataattgacaata

SEQ ID NO: 9 - DNA, 388 bp, synthetic construct
  source 1..388: mol_type = other DNA; note = 3'UTR E
cctgaggcctcagaacacaggtttcagattgataggcctgcaggtctccaggcagcaaccagctgagcgactaaagggcccaaggccagggctctagggatggggctcagcagaggctggggtaaggggagccagggaggagctgggcctaatgcagcaccgggtccccaggatgccgtgtctcggctggaggaggagatgcggaagctccaggccacggtgcaggagctccagaagcgcttggacaggctggaggagacagtccaggccaagtagagccccgcagggcctccagcagggtcagccattcacacccatccactcacctcccattcccagccacatggcagagaaaaaaatcataataaaatggctttattttctggta

SEQ ID NO: 10 - DNA, 296 bp, synthetic construct
  source 1..296: mol_type = other DNA; note = 3'UTR D
ggggccttctgacatgagtctggcctggccccacctcctagttcctcataataaagacagattgcttcttcgcttctcactgaggggccttctgacatgagtctggcctggccccacctccccagtttctcataataaagacagattgcttcttcacttgaagctcgctttcttgctgtccaatttctattaaaggttcctttgttccctaagtccaactactaaactgggggatattatgaagggccttgagcatctggattctgcctaataaaaaacatttattttcattgcaa

SEQ ID NO: 11 - DNA, 289 bp, synthetic construct
  source 1..289: mol_type = other DNA; note = 3'UTR BNT162b2
ctcgagctggtactgcatgcacgcaatgctagctgcccctttcccgtcctgggtaccccgagtctcccccgacctcgggtcccaggtatgctcccacctccacctgccccactcaccacctctgctagttccagacacctcccaagcacgcagcaatgcagctcaaaacgcttagcctagccacacccccacgggaaacagcagtgattaacctttagcaataaacgaaagtttaactaagctatactaaccccagggttggtcaatttcgtgccagccacaccctgga

SEQ ID NO: 12 - protein, 1271 aa, synthetic construct
  source 1..1271: note = B.1.617.2(Delta)Spike
MFVFLVLLPLVSSQCVNLRTRTQLPPAYTNSFTRGVYYPDKVFRSSVLHSTQDLFLPFFSNVTWFHAIHVSGTNGTKRFDNPVLPFNDGVYFASTEKSNIIRGWIFGTTLDSKTQSLLIVNNATNVVIKVCEFQFCNDPFLDVYYHKNNKSWMESGVYSSANNCTFEYVSQPFLMDLEGKQGNFKNLREFVFKNIDGYFKIYSKHTPINLVRDLPQGFSALEPLVDLPIGINITRFQTLLALHRSYLTPGDSSSGWTAGAAAYYVGYLQPRTFLLKYNENGTITDAVDCALDPLSETKCTLKSFTVEKGIYQTSNFRVQPTESIVRFPNITNLCPFGEVFNATRFASVYAWNRKRISNCVADYSVLYNSASFSTFKCYGVSPTKLNDLCFTNVYADSFVIRGDEVRQIAPGQTGKIADYNYKLPDDFTGCVIAWNSNNLDSKVGGNYNYRYRLFRKSNLKPFERDISTEIYQAGSKPCNGVEGFNCYFPLQSYGFQPTNGVGYQPYRVVVLSFELLHAPATVCGPKKSTNLVKNKCVNFNFNGLTGTGVLTESNKKFLPFQQFGRDIADTTDAVRDPQTLEILDITPCSFGGVSVITPGTNTSNQVAVLYQGVNCTEVPVAIHADQLTPTWRVYSTGSNVFQTRAGCLIGAEHVNNSYECDIPIGAGICASYQTQTNSRRRARSVASQSIIAYTMSLGAENSVAYSNNSIAIPTNFTISVTTEILPVSMTKTSVDCTMYICGDSTECSNLLLQYGSFCTQLNRALTGIAVEQDKNTQEVFAQVKQIYKTPPIKDFGGFNFSQILPDPSKPSKRSFIEDLLFNKVTLADAGFIKQYGDCLGDIAARDLICAQKFNGLTVLPPLLTDEMIAQYTSALLAGTITSGWTFGAGAALQIPFAMQMAYRFNGIGVTQNVLYENQKLIANQFNSAIGKIQDSLSSTASALGKLQNVVNQNAQALNTLVKQLSSNFGAISSVLNDILSRLDPPEAEVQIDRLITGRLQSLQTYVTQQLIRAAEIRASANLAATKMSECVLGQSKRVDFCGKGYHLMSFPQSAPHGVVFLHVTYVPAQEKNFTTAPAICHDGKAHFPREGVFVSNGTHWFVTQRNFYEPQIITTDNTFVSGNCDVVIGIVNNTVYDPLQPELDSFKEELDKYFKNHTSPDVDLGDISGINASVVNIQKEIDRLNEVAKNLNESLIDLQELGKYEQYIKWPWYIWLGFIAGLIAIVMVTIMLCCMTSCCSCLKGCCSCGSCCKFDEDDSEPVLKGVKLHYT

SEQ ID NO: 13 - DNA, 3819 bp, synthetic construct
  source 1..3819: mol_type = other DNA; note = B.1.617.2(Delta)Spike CDS
atgttcgtgttcctggtgctgctgcccctggtgagctctcagtgcgtgaacctgaggacaagaacacagctgccccccgcctacaccaacagcttcacaagaggcgtgtactaccccgacaaggtgttcagaagcagcgtgctgcactccacccaagacctgtttctgcccttcttcagcaacgtgacctggttccacgccatccacgtcagcggcaccaacggcaccaagagattcgacaaccccgtgctgcccttcaacgacggcgtgtacttcgctagcaccgaaaagagcaacatcatcagaggctggatcttcggcaccaccctagactccaagacacaaagcctgctgatcgttaacaacgcgaccaacgtggtgatcaaggtgtgcgagtttcagttctgcaacgaccccttcctggacgtgtactaccacaagaacaacaagagctggatggagagcggggtctacagcagcgccaacaactgcaccttcgagtacgtgtctcagcccttcctgatggacctggagggcaagcaaggcaatttcaagaacctaagagagttcgtgttcaagaacatcgacggctacttcaagatctacagcaagcacacccccatcaacctggtgagagacctgccccaaggcttcagcgccctggagcccctggtggacctgcccatcggcatcaacatcacaagatttcagaccctgctggccctgcaccgtagctacctaacccccggcgatagttcctctggctggacggccggcgctgccgcctactacgtgggctacctgcagcctagaaccttcctgctgaagtacaacgagaacggcactatcactgatgccgtggactgtgccctggaccccctgagcgagaccaagtgcaccctcaagagcttcaccgtggagaagggcatctatcagacaagcaacttcagagtgcagcccaccgagagcatcgtgagattccccaacatcaccaacctgtgccccttcggcgaggtgttcaacgccacaagattcgctagcgtgtacgcgtggaacagaaagagaatcagcaactgcgtggccgactacagcgtgctgtacaacagcgctagcttcagcaccttcaagtgctatggcgtcagccccaccaagctgaacgacctgtgcttcaccaacgtgtacgccgacagcttcgtgatcagaggcgacgaggtgagacagattgcccccgggcaaaccggcaagatcgccgactacaactacaagctgcccgacgacttcaccggctgcgtgatcgcgtggaacagcaataacctggattccaaggtgggcggcaactacaactaccggtacagactgttcagaaagagcaacctgaagcccttcgagagagacatcagcaccgagatctaccaagccggcagcaagccctgcaacggcgtggagggcttcaactgctacttccccctgcagagctacggctttcagcccaccaacggcgtgggctatcagccctacagagtggtggtgctgagcttcgagctgctgcacgcccccgcaaccgtgtgcggccccaaaaagagcaccaacctggtgaagaacaagtgcgtgaacttcaactttaatggccttaccggcacgggcgtgctgaccgagagcaacaagaagttcctgccatttcagcaattcggcagagacatcgccgacaccaccgacgcggtcagagaccctcagaccctggagatcctggacatcaccccctgtagcttcggcggcgtgagcgtgatcacccccggcactaacacaagcaaccaagtggccgtgctgtaccaaggcgtgaactgcaccgaggtgcccgtggccatccacgccgatcagctgacccccacctggagagtatacagcaccggaagcaacgtgtttcagacaagagccggctgcctgatcggcgccgagcacgtgaacaacagctacgagtgcgacatccccatcggcgccggcatctgcgctagctatcagacacagaccaacagccgccggagagctagaagcgtggcttctcagagcatcatcgcctacaccatgagcctgggcgccgagaacagcgtggcctacagcaacaacagcatcgccatccccaccaacttcaccatcagcgtgaccaccgagatcctgcccgtaagtatgaccaagacaagcgtggactgcaccatgtacatctgcggcgacagcaccgagtgcagcaacctgctgctgcagtacggcagcttctgcacacagctgaacagagccctgaccggcatcgccgtggagcaagacaagaacacccaagaggtgttcgcccaagtgaagcagatctacaagaccccccccatcaaggacttcggcggcttcaacttcagccaaatcctgcccgaccctagcaagcctagcaagcggagcttcatcgaggacctgctgttcaacaaggtgaccctggccgacgccggcttcatcaagcagtacggcgactgcctaggcgacatcgcagctagagacctgatctgcgctcagaagttcaatggactcaccgtgctcccccccctgctgaccgacgagatgatcgctcagtacacctctgccctgctggcgggaaccataacaagcggttggacatttggcgccggggccgcactgcaaatccccttcgccatgcagatggcctacagattcaacggcatcggcgtgacacagaacgtgctgtacgagaatcagaagctgatcgccaatcagttcaacagcgccatcggcaagatccaagacagcctgagcagcaccgctagcgccctgggcaagctgcaaaacgtggtgaatcagaacgcccaagccctgaacaccctggtgaagcagctgagcagcaacttcggcgccatcagcagcgtattgaatgacatcctgtctagactggacccccccgaggccgaggtgcagatcgacagactgatcaccggcagactgcagagcctgcagacctacgtgacacagcagctgatcagagccgccgagatcagagctagcgccaacctggccgccaccaagatgagcgagtgcgtgctggggcagagcaagagagtggacttctgcggcaagggctaccacctgatgagcttccctcagagcgccccccacggcgtggtgttcctgcacgtgacctacgtgcccgcccaagagaagaacttcaccaccgctcccgccatctgccacgacggcaaggcccacttccctagagagggcgtgttcgtgagcaacggcacccactggttcgtgacacagagaaacttctacgagcctcagatcatcaccaccgacaacaccttcgtgagcggcaactgcgacgtggtgatcggcatagtgaacaacaccgtatacgaccccctgcagcccgagctggacagcttcaaggaggagctggacaagtacttcaaaaaccatactagccccgacgtggacctgggagacatctctggcatcaacgctagcgtggtgaacattcagaaggagatcgaccggctgaatgaggtggccaagaacctgaacgagagcctgatcgacctgcaagagctgggcaagtacgagcagtacatcaagtggccctggtacatctggctgggcttcatcgccggcctgatcgccatcgtgatggtgaccatcatgctgtgctgcatgacaagctgttgcagctgcctgaaaggttgctgcagctgtggctcgtgctgcaagttcgacgaggacgacagcgagcccgtgctgaagggcgtgaagctgcactacacctgatga

SEQ ID NO: 14 - protein, 1270 aa, synthetic construct
  source 1..1270: note = B.1.1.529(Omicron) Spike
MFVFLVLLPLVSSQCVNLTTRTQLPPAYTNSFTRGVYYPDKVFRSSVLHSTQDLFLPFFSNVTWFHVISGTNGTKRFDNPVLPFNDGVYFASIEKSNIIRGWIFGTTLDSKTQSLLIVNNATNVVIKVCEFQFCNDPFLDHKNNKSWMESEFRVYSSANNCTFEYVSQPFLMDLEGKQGNFKNLREFVFKNIDGYFKIYSKHTPIIVREPEDLPQGFSALEPLVDLPIGINITRFQTLLALHRSYLTPGDSSSGWTAGAAAYYVGYLQPRTFLLKYNENGTITDAVDCALDPLSETKCTLKSFTVEKGIYQTSNFRVQPTESIVRFPNITNLCPFDEVFNATRFASVYAWNRKRISNCVADYSVLYNLAPFFTFKCYGVSPTKLNDLCFTNVYADSFVIRGDEVRQIAPGQTGNIADYNYKLPDDFTGCVIAWNSNKLDSKVSGNYNYLYRLFRKSNLKPFERDISTEIYQAGNKPCNGVAGFNCYFPLRSYSFRPTYGVGHQPYRVVVLSFELLHAPATVCGPKKSTNLVKNKCVNFNFNGLKGTGVLTESNKKFLPFQQFGRDIADTTDAVRDPQTLEILDITPCSFGGVSVITPGTNTSNQVAVLYQGVNCTEVPVAIHADQLTPTWRVYSTGSNVFQTRAGCLIGAEYVNNSYECDIPIGAGICASYQTQTKSHRRARSVASQSIIAYTMSLGAENSVAYSNNSIAIPTNFTISVTTEILPVSMTKTSVDCTMYICGDSTECSNLLLQYGSFCTQLKRALTGIAVEQDKNTQEVFAQVKQIYKTPPIKYFGGFNFSQILPDPSKPSKRSFIEDLLFNKVTLADAGFIKQYGDCLGDIAARDLICAQKFKGLTVLPPLLTDEMIAQYTSALLAGTITSGWTFGAGAALQIPFAMQMAYRFNGIGVTQNVLYENQKLIANQFNSAIGKIQDSLSSTASALGKLQDVVNHNAQALNTLVKQLSSKFGAISSVLNDIFSRLDPPEAEVQIDRLITGRLQSLQTYVTQQLIRAAEIRASANLAATKMSECVLGQSKRVDFCGKGYHLMSFPQSAPHGVVFLHVTYVPAQEKNFTTAPAICHDGKAHFPREGVFVSNGTHWFVTQRNFYEPQIITTDNTFVSGNCDVVIGIVNNTVYDPLQPELDSFKEELDKYFKNHTSPDVDLGDISGINASVVNIQKEIDRLNEVAKNLNESLIDLQELGKYEQYIKWPWYIWLGFIAGLIAIVMVTIMLCCMTSCCSCLKGCCSCGSCCKFDEDDSEPVLKGVKLHYT

SEQ ID NO: 15 - DNA, 3816 bp, synthetic construct
  source 1..3816: mol_type = other DNA; note = B.1.1.529(Omicron)Spike CDS
atgttcgtgttcctggtgctgctgcccctggtgagctctcagtgcgtgaacctgaccacaagaacacagctgccccccgcctacaccaacagcttcacaagaggcgtgtactaccccgacaaggtgttcagaagcagcgtgctgcactccacccaagacctgtttctgcccttcttcagcaacgtgacctggttccacgtgatcagcggcaccaacggcaccaagagattcgacaaccccgtgctgcccttcaacgacggcgtgtacttcgctagcatcgaaaagagcaacatcatcagaggctggatcttcggcaccaccctagactccaagacacaaagcctgctgatcgttaacaacgcgaccaacgtggtgatcaaggtgtgcgagtttcagttctgcaacgaccccttcctggaccacaagaacaacaagagctggatggagagcgagttcagagtgtacagcagcgccaacaactgcaccttcgagtacgtgtctcagcccttcctgatggacctggagggcaagcaaggcaatttcaagaacctaagagagttcgtgttcaagaacatcgacggctacttcaagatctacagcaagcacacccccatcatcgtgagagagcccgaggacctgccccaaggcttcagcgccctggagcccctggtggacctgcccatcggcatcaacatcacaagatttcagaccctgctggccctgcaccgtagctacctaacccccggcgatagttcctctggctggacggccggcgctgccgcctactacgtgggctacctgcagcctagaaccttcctgctgaagtacaacgagaacggcactatcactgatgccgtggactgtgccctggaccccctgagcgagaccaagtgcaccctcaagagcttcaccgtggagaagggcatctatcagacaagcaacttcagagtgcagcccaccgagagcatcgtgagattccccaacatcaccaacctgtgccccttcgacgaggtgttcaacgccaccagatttgctagcgtgtacgcctggaaccggaagagaatcagcaactgcgtggccgactacagcgtgctgtacaacctggcccccttcttcaccttcaagtgctatggcgtcagccccaccaagctgaacgacctgtgcttcaccaacgtgtacgccgacagcttcgtgatcagaggcgacgaggtgagacagatcgcccccgggcagaccggcaacatcgccgactacaactacaagctgcccgacgacttcaccggctgcgtgatcgcctggaacagcaacaagctggatagcaaggtgagcggcaactacaattacctgtacagactgttcagaaagagcaacctgaagcccttcgagagagacatcagcaccgagatctaccaagccggcaacaagccctgcaacggcgtggcgggcttcaactgctacttccccctcaggagctacagcttcagacccacctacggcgtgggccatcagccctacagagtggtcgtgctgagcttcgagctgctgcacgcccctgccacagtgtgcggccccaaaaagagcaccaacctggtgaagaacaagtgcgtgaacttcaacttcaacggcctgaagggcaccggcgtgctgaccgagagcaacaagaagttcctgccatttcagcaattcggcagagacatcgccgacaccaccgacgcggtcagagaccctcagaccctggagatcctggacatcaccccctgtagcttcggcggcgtgagcgtgatcacccccggcactaacacaagcaaccaagtggccgtgctgtaccaaggcgtgaactgcaccgaggtgcccgtggccatccacgccgatcagctgacccccacctggagagtgtatagcaccggcagcaacgtgtttcagacaagagccggctgcctgatcggcgccgagtacgtgaacaacagctacgagtgcgacatccccatcggcgccggcatctgcgctagctatcagacacagaccaagagccaccggagagctagaagcgtggctagccaaagcatcatcgcctacaccatgagcctgggcgccgagaacagcgtggcctacagcaacaacagcatcgccatccccaccaacttcaccatcagcgtgaccaccgagatcctgcccgtaagtatgaccaagacaagcgtggactgcaccatgtacatctgcggcgacagcaccgagtgcagcaacctgctcctgcagtacggcagcttctgcacacagctgaagagagccctgaccggcatcgccgtggagcaagacaagaacacccaagaggtgttcgcccaagtgaagcagatctacaagaccccccccatcaagtacttcggcggcttcaacttcagccaaatcctgcccgaccctagcaagcctagcaagcggagcttcatcgaggacctgctgttcaacaaggtgaccctggccgacgccggcttcatcaagcagtacggcgactgcctaggcgacatcgcagctagagacctgatctgcgctcagaagttcaagggactcaccgtgctcccccccctgctgaccgacgagatgatcgctcagtacacctctgccctgctggcgggaaccataacaagcggttggacatttggcgccggggccgcactgcaaatccccttcgccatgcagatggcctacagattcaacggcatcggcgtgacacagaacgtgctgtacgagaatcagaagctgatcgccaatcagttcaacagcgccatcggcaagatccaagacagcctgagcagcaccgctagcgccctgggcaagctgcaagacgtggtgaaccacaacgcccaagccctgaacaccctggtgaagcagctgagcagcaagttcggcgccatcagcagcgtgctgaatgacatcttctctagactggacccccccgaggccgaggtgcagatcgacagactgatcaccggcagactgcagagcctgcagacctacgtgacacagcagctgatcagagccgccgagatcagagctagcgccaacctggccgccaccaagatgagcgagtgcgtgctggggcagagcaagagagtggacttctgcggcaagggctaccacctgatgagcttccctcagagcgccccccacggcgtggtgttcctgcacgtgacctacgtgcccgcccaagagaagaacttcaccaccgctcccgccatctgccacgacggcaaggcccacttccctagagagggcgtgttcgtgagcaacggcacccactggttcgtgacacagagaaacttctacgagcctcagatcatcaccaccgacaacaccttcgtgagcggcaactgcgacgtggtgatcggcatagtgaacaacaccgtatacgaccccctgcagcccgagctggacagcttcaaggaggagctggacaagtacttcaaaaaccatactagccccgacgtggacctgggagacatctctggcatcaacgctagcgtggtgaacattcagaaggagatcgaccggctgaatgaggtggccaagaacctgaacgagagcctgatcgacctgcaagagctgggcaagtacgagcagtacatcaagtggccctggtacatctggctgggcttcatcgccggcctgatcgccatcgtgatggtgaccatcatgctgtgctgcatgacaagctgttgcagctgcctgaaaggttgctgcagctgtggctcgtgctgcaagttcgacgaggacgacagcgagcccgtgctgaagggcgtgaagctgcactacacctgatga

SEQ ID NO: 16 - DNA, 112 bp, synthetic construct
  source 1..112: mol_type = other DNA; note = poly A
aaaaaaaaaaaaaaaaaaaaaaaaaaaaaagcatatgactaaaaaaaaaaaaaaaaaaaaaaaaaaaaaaaaaaaaaaaaaaaaaaaaaaaaaaaaaaaaaaaaaaaaaaaa

SEQ ID NO: 17 - DNA, 20 bp, synthetic construct
  source 1..20: mol_type = other DNA; note = T7 promoter
taatacgactcactataagg

SEQ ID NO: 18 - DNA, 4134 bp, synthetic construct
  source 1..4134: mol_type = other DNA; note = I'-Delta24-B
gagttaggagttggtggcagtttcaataacaggtcattgccgagaaaaggatagcactataatatgttcgtgttcctggtgctgctgcccctggtgagctctcagtgcgtgaacctgaggacaagaacacagctgccccccgcctacaccaacagcttcacaagaggcgtgtactaccccgacaaggtgttcagaagcagcgtgctgcactccacccaagacctgtttctgcccttcttcagcaacgtgacctggttccacgccatccacgtcagcggcaccaacggcaccaagagattcgacaaccccgtgctgcccttcaacgacggcgtgtacttcgctagcaccgaaaagagcaacatcatcagaggctggatcttcggcaccaccctagactccaagacacaaagcctgctgatcgttaacaacgcgaccaacgtggtgatcaaggtgtgcgagtttcagttctgcaacgaccccttcctggacgtgtactaccacaagaacaacaagagctggatggagagcggggtctacagcagcgccaacaactgcaccttcgagtacgtgtctcagcccttcctgatggacctggagggcaagcaaggcaatttcaagaacctaagagagttcgtgttcaagaacatcgacggctacttcaagatctacagcaagcacacccccatcaacctggtgagagacctgccccaaggcttcagcgccctggagcccctggtggacctgcccatcggcatcaacatcacaagatttcagaccctgctggccctgcaccgtagctacctaacccccggcgatagttcctctggctggacggccggcgctgccgcctactacgtgggctacctgcagcctagaaccttcctgctgaagtacaacgagaacggcactatcactgatgccgtggactgtgccctggaccccctgagcgagaccaagtgcaccctcaagagcttcaccgtggagaagggcatctatcagacaagcaacttcagagtgcagcccaccgagagcatcgtgagattccccaacatcaccaacctgtgccccttcggcgaggtgttcaacgccacaagattcgctagcgtgtacgcgtggaacagaaagagaatcagcaactgcgtggccgactacagcgtgctgtacaacagcgctagcttcagcaccttcaagtgctatggcgtcagccccaccaagctgaacgacctgtgcttcaccaacgtgtacgccgacagcttcgtgatcagaggcgacgaggtgagacagattgcccccgggcaaaccggcaagatcgccgactacaactacaagctgcccgacgacttcaccggctgcgtgatcgcgtggaacagcaataacctggattccaaggtgggcggcaactacaactaccggtacagactgttcagaaagagcaacctgaagcccttcgagagagacatcagcaccgagatctaccaagccggcagcaagccctgcaacggcgtggagggcttcaactgctacttccccctgcagagctacggctttcagcccaccaacggcgtgggctatcagccctacagagtggtggtgctgagcttcgagctgctgcacgcccccgcaaccgtgtgcggccccaaaaagagcaccaacctggtgaagaacaagtgcgtgaacttcaactttaatggccttaccggcacgggcgtgctgaccgagagcaacaagaagttcctgccatttcagcaattcggcagagacatcgccgacaccaccgacgcggtcagagaccctcagaccctggagatcctggacatcaccccctgtagcttcggcggcgtgagcgtgatcacccccggcactaacacaagcaaccaagtggccgtgctgtaccaaggcgtgaactgcaccgaggtgcccgtggccatccacgccgatcagctgacccccacctggagagtatacagcaccggaagcaacgtgtttcagacaagagccggctgcctgatcggcgccgagcacgtgaacaacagctacgagtgcgacatccccatcggcgccggcatctgcgctagctatcagacacagaccaacagccgccggagagctagaagcgtggcttctcagagcatcatcgcctacaccatgagcctgggcgccgagaacagcgtggcctacagcaacaacagcatcgccatccccaccaacttcaccatcagcgtgaccaccgagatcctgcccgtaagtatgaccaagacaagcgtggactgcaccatgtacatctgcggcgacagcaccgagtgcagcaacctgctgctgcagtacggcagcttctgcacacagctgaacagagccctgaccggcatcgccgtggagcaagacaagaacacccaagaggtgttcgcccaagtgaagcagatctacaagaccccccccatcaaggacttcggcggcttcaacttcagccaaatcctgcccgaccctagcaagcctagcaagcggagcttcatcgaggacctgctgttcaacaaggtgaccctggccgacgccggcttcatcaagcagtacggcgactgcctaggcgacatcgcagctagagacctgatctgcgctcagaagttcaatggactcaccgtgctcccccccctgctgaccgacgagatgatcgctcagtacacctctgccctgctggcgggaaccataacaagcggttggacatttggcgccggggccgcactgcaaatccccttcgccatgcagatggcctacagattcaacggcatcggcgtgacacagaacgtgctgtacgagaatcagaagctgatcgccaatcagttcaacagcgccatcggcaagatccaagacagcctgagcagcaccgctagcgccctgggcaagctgcaaaacgtggtgaatcagaacgcccaagccctgaacaccctggtgaagcagctgagcagcaacttcggcgccatcagcagcgtattgaatgacatcctgtctagactggacccccccgaggccgaggtgcagatcgacagactgatcaccggcagactgcagagcctgcagacctacgtgacacagcagctgatcagagccgccgagatcagagctagcgccaacctggccgccaccaagatgagcgagtgcgtgctggggcagagcaagagagtggacttctgcggcaagggctaccacctgatgagcttccctcagagcgccccccacggcgtggtgttcctgcacgtgacctacgtgcccgcccaagagaagaacttcaccaccgctcccgccatctgccacgacggcaaggcccacttccctagagagggcgtgttcgtgagcaacggcacccactggttcgtgacacagagaaacttctacgagcctcagatcatcaccaccgacaacaccttcgtgagcggcaactgcgacgtggtgatcggcatagtgaacaacaccgtatacgaccccctgcagcccgagctggacagcttcaaggaggagctggacaagtacttcaaaaaccatactagccccgacgtggacctgggagacatctctggcatcaacgctagcgtggtgaacattcagaaggagatcgaccggctgaatgaggtggccaagaacctgaacgagagcctgatcgacctgcaagagctgggcaagtacgagcagtacatcaagtggccctggtacatctggctgggcttcatcgccggcctgatcgccatcgtgatggtgaccatcatgctgtgctgcatgacaagctgttgcagctgcctgaaaggttgctgcagctgtggctcgtgctgcaagttcgacgaggacgacagcgagcccgtgctgaagggcgtgaagctgcactacacctgatgactcgaggctcgctttcttgctgtccaatttctattaaaggttcctttgttccctaagtccaactactaaactgggggatattatgaagggccttgagcatctggattctgcctaataaaaaacatttattttcattgcaaaaaaaaaaaaaaaaaaaaaaaaaaaaaaaagcatatgactaaaaaaaaaaaaaaaaaaaaaaaaaaaaaaaaaaaaaaaaaaaaaaaaaaaaaaaaaaaaaaaaaaaaaaaa

SEQ ID NO: 19 - DNA, 4131 bp, synthetic construct
  source 1..4131: mol_type = other DNA; note = I'-OC24-B
gagttaggagttggtggcagtttcaataacaggtcattgccgagaaaaggatagcactataatatgttcgtgttcctggtgctgctgcccctggtgagctctcagtgcgtgaacctgaccacaagaacacagctgccccccgcctacaccaacagcttcacaagaggcgtgtactaccccgacaaggtgttcagaagcagcgtgctgcactccacccaagacctgtttctgcccttcttcagcaacgtgacctggttccacgtgatcagcggcaccaacggcaccaagagattcgacaaccccgtgctgcccttcaacgacggcgtgtacttcgctagcatcgaaaagagcaacatcatcagaggctggatcttcggcaccaccctagactccaagacacaaagcctgctgatcgttaacaacgcgaccaacgtggtgatcaaggtgtgcgagtttcagttctgcaacgaccccttcctggaccacaagaacaacaagagctggatggagagcgagttcagagtgtacagcagcgccaacaactgcaccttcgagtacgtgtctcagcccttcctgatggacctggagggcaagcaaggcaatttcaagaacctaagagagttcgtgttcaagaacatcgacggctacttcaagatctacagcaagcacacccccatcatcgtgagagagcccgaggacctgccccaaggcttcagcgccctggagcccctggtggacctgcccatcggcatcaacatcacaagatttcagaccctgctggccctgcaccgtagctacctaacccccggcgatagttcctctggctggacggccggcgctgccgcctactacgtgggctacctgcagcctagaaccttcctgctgaagtacaacgagaacggcactatcactgatgccgtggactgtgccctggaccccctgagcgagaccaagtgcaccctcaagagcttcaccgtggagaagggcatctatcagacaagcaacttcagagtgcagcccaccgagagcatcgtgagattccccaacatcaccaacctgtgccccttcgacgaggtgttcaacgccaccagatttgctagcgtgtacgcctggaaccggaagagaatcagcaactgcgtggccgactacagcgtgctgtacaacctggcccccttcttcaccttcaagtgctatggcgtcagccccaccaagctgaacgacctgtgcttcaccaacgtgtacgccgacagcttcgtgatcagaggcgacgaggtgagacagatcgcccccgggcagaccggcaacatcgccgactacaactacaagctgcccgacgacttcaccggctgcgtgatcgcctggaacagcaacaagctggatagcaaggtgagcggcaactacaattacctgtacagactgttcagaaagagcaacctgaagcccttcgagagagacatcagcaccgagatctaccaagccggcaacaagccctgcaacggcgtggcgggcttcaactgctacttccccctcaggagctacagcttcagacccacctacggcgtgggccatcagccctacagagtggtcgtgctgagcttcgagctgctgcacgcccctgccacagtgtgcggccccaaaaagagcaccaacctggtgaagaacaagtgcgtgaacttcaacttcaacggcctgaagggcaccggcgtgctgaccgagagcaacaagaagttcctgccatttcagcaattcggcagagacatcgccgacaccaccgacgcggtcagagaccctcagaccctggagatcctggacatcaccccctgtagcttcggcggcgtgagcgtgatcacccccggcactaacacaagcaaccaagtggccgtgctgtaccaaggcgtgaactgcaccgaggtgcccgtggccatccacgccgatcagctgacccccacctggagagtgtatagcaccggcagcaacgtgtttcagacaagagccggctgcctgatcggcgccgagtacgtgaacaacagctacgagtgcgacatccccatcggcgccggcatctgcgctagctatcagacacagaccaagagccaccggagagctagaagcgtggctagccaaagcatcatcgcctacaccatgagcctgggcgccgagaacagcgtggcctacagcaacaacagcatcgccatccccaccaacttcaccatcagcgtgaccaccgagatcctgcccgtaagtatgaccaagacaagcgtggactgcaccatgtacatctgcggcgacagcaccgagtgcagcaacctgctcctgcagtacggcagcttctgcacacagctgaagagagccctgaccggcatcgccgtggagcaagacaagaacacccaagaggtgttcgcccaagtgaagcagatctacaagaccccccccatcaagtacttcggcggcttcaacttcagccaaatcctgcccgaccctagcaagcctagcaagcggagcttcatcgaggacctgctgttcaacaaggtgaccctggccgacgccggcttcatcaagcagtacggcgactgcctaggcgacatcgcagctagagacctgatctgcgctcagaagttcaagggactcaccgtgctcccccccctgctgaccgacgagatgatcgctcagtacacctctgccctgctggcgggaaccataacaagcggttggacatttggcgccggggccgcactgcaaatccccttcgccatgcagatggcctacagattcaacggcatcggcgtgacacagaacgtgctgtacgagaatcagaagctgatcgccaatcagttcaacagcgccatcggcaagatccaagacagcctgagcagcaccgctagcgccctgggcaagctgcaagacgtggtgaaccacaacgcccaagccctgaacaccctggtgaagcagctgagcagcaagttcggcgccatcagcagcgtgctgaatgacatcttctctagactggacccccccgaggccgaggtgcagatcgacagactgatcaccggcagactgcagagcctgcagacctacgtgacacagcagctgatcagagccgccgagatcagagctagcgccaacctggccgccaccaagatgagcgagtgcgtgctggggcagagcaagagagtggacttctgcggcaagggctaccacctgatgagcttccctcagagcgccccccacggcgtggtgttcctgcacgtgacctacgtgcccgcccaagagaagaacttcaccaccgctcccgccatctgccacgacggcaaggcccacttccctagagagggcgtgttcgtgagcaacggcacccactggttcgtgacacagagaaacttctacgagcctcagatcatcaccaccgacaacaccttcgtgagcggcaactgcgacgtggtgatcggcatagtgaacaacaccgtatacgaccccctgcagcccgagctggacagcttcaaggaggagctggacaagtacttcaaaaaccatactagccccgacgtggacctgggagacatctctggcatcaacgctagcgtggtgaacattcagaaggagatcgaccggctgaatgaggtggccaagaacctgaacgagagcctgatcgacctgcaagagctgggcaagtacgagcagtacatcaagtggccctggtacatctggctgggcttcatcgccggcctgatcgccatcgtgatggtgaccatcatgctgtgctgcatgacaagctgttgcagctgcctgaaaggttgctgcagctgtggctcgtgctgcaagttcgacgaggacgacagcgagcccgtgctgaagggcgtgaagctgcactacacctgatgactcgaggctcgctttcttgctgtccaatttctattaaaggttcctttgttccctaagtccaactactaaactgggggatattatgaagggccttgagcatctggattctgcctaataaaaaacatttattttcattgcaaaaaaaaaaaaaaaaaaaaaaaaaaaaaaaagcatatgactaaaaaaaaaaaaaaaaaaaaaaaaaaaaaaaaaaaaaaaaaaaaaaaaaaaaaaaaaaaaaaaaaaaaaaaa

SEQ ID NO: 20 - DNA, 3816 bp, synthetic construct
  source 1..3816: mol_type = other DNA; note = B.1.351 Spike CDS
atgttcgtgttcctggtgctgctgcccctggtgagctctcagtgcgtgaacttcacgacaagaacacagctgccccccgcctacaccaacagcttcacaagaggcgtgtactaccccgacaaggtgttcagaagcagcgtgctgcactccacccaagacctgtttctgcccttcttcagcaacgtgacctggttccacgccatccacgtgagcggcaccaacggcaccaagagattcgccaaccccgtgctgcccttcaacgacggcgtgtacttcgctagcaccgaaaagagcaacatcatcagaggctggatcttcggcaccaccctagactccaagacacaaagcctgctgatcgttaacaacgcgaccaacgtggtgatcaaggtgtgcgagtttcagttctgcaacgaccccttcctgggcgtgtactaccacaagaacaacaagagctggatggagagcgagttccgtgtctacagcagcgccaacaactgcaccttcgagtacgtgtctcagcccttcctgatggacctggagggcaagcaaggcaatttcaagaacctaagagagttcgtgttcaagaacatcgacggctacttcaagatctacagcaagcacacccccatcaacctggtgagaggcctgccccaaggcttcagcgccctggagcccctggtggacctgcccatcggcatcaacatcacaagatttcagaccctgcaccgtagctacctaacccccggcgatagttcctctggctggacggccggcgctgccgcctactacgtgggctacctgcagcctagaaccttcctgctgaagtacaacgagaacggcactatcactgatgccgtggactgtgccctggaccccctgagcgagaccaagtgcaccctcaagagcttcaccgtggagaagggcatctatcagacaagcaacttcagagtgcagcccaccgagagcatcgtgagattccccaacatcaccaacctgtgccccttcggcgaggtgttcaacgccacaagattcgctagcgtgtacgcgtggaacagaaagagaatcagcaactgcgtggccgactacagcgtgctgtacaacagcgctagcttcagcaccttcaagtgctatggcgtcagccccaccaagctgaacgacctgtgcttcaccaacgtgtacgccgacagcttcgtgatcagaggcgacgaggtgagacagattgcccccgggcaaaccggcaacatcgccgactacaactacaagctgcccgacgacttcaccggctgcgtgatcgcgtggaacagcaataacctggattccaaggtgggcggcaactacaactacctgtacagactgttcagaaagagcaacctgaagcccttcgagagagacatcagcaccgagatctaccaagccggcagcaccccctgcaacggcgtgaagggcttcaactgctacttccccctgcagagctacggctttcagcccacctacggcgtgggctatcagccctacagagtggtggtgctgagcttcgagctgctgcacgcccccgcaaccgtgtgcggccccaaaaagagcaccaacctggtgaagaacaagtgcgtgaacttcaactttaatggccttaccggcacgggcgtgctgaccgagagcaacaagaagttcctgccatttcagcaattcggcagagacatcgccgacaccaccgacgcggtcagagaccctcagaccctggagatcctggacatcaccccctgtagcttcggcggcgtgagcgtgatcacccccggcactaacacaagcaaccaagtggccgtgctgtaccaaggcgtgaactgcaccgaggtgcccgtggccatccacgccgatcagctgacccccacctggagagtatacagcaccggaagcaacgtgtttcagacaagagccggctgcctgatcggcgccgagcacgtgaacaacagctacgagtgcgacatccccatcggcgccggcatctgcgctagctatcagacacagaccaacagcccccggagagctagaagcgtggcttctcagagcatcatcgcctacaccatgagcctgggcgtcgagaacagcgtggcctacagcaacaacagcatcgccatccccaccaacttcaccatcagcgtgaccaccgagatcctgcccgtaagtatgaccaagacaagcgtggactgcaccatgtacatctgcggcgacagcaccgagtgcagcaacctgctgctgcagtacggcagcttctgcacacagctgaacagagccctgaccggcatcgccgtggagcaagacaagaacacccaagaggtgttcgcccaagtgaagcagatctacaagaccccccccatcaaggacttcggcggcttcaacttcagccaaatcctgcccgaccctagcaagcctagcaagcggagcttcatcgaggacctgctgttcaacaaggtgaccctggccgacgccggcttcatcaagcagtacggcgactgcctaggcgacatcgcagctagagacctgatctgcgctcagaagttcaatggactcaccgtgctcccccccctgctgaccgacgagatgatcgctcagtacacctctgccctgctggcgggaaccataacaagcggttggacatttggcgccggggccgcactgcaaatccccttcgccatgcagatggcctacagattcaacggcatcggcgtgacacagaacgtgctgtacgagaatcagaagctgatcgccaatcagttcaacagcgccatcggcaagatccaagacagcctgagcagcaccgctagcgccctgggcaagctgcaagacgtggtgaatcagaacgcccaagccctgaacaccctggtgaagcagctgagcagcaacttcggcgccatcagcagcgtattgaatgacatcctgtctagactggacccccccgaggccgaggtgcagatcgacagactgatcaccggcagactgcagagcctgcagacctacgtgacacagcagctgatcagagccgccgagatcagagctagcgccaacctggccgccaccaagatgagcgagtgcgtgctggggcagagcaagagagtggacttctgcggcaagggctaccacctgatgagcttccctcagagcgccccccacggcgtggtgttcctgcacgtgacctacgtgcccgcccaagagaagaacttcaccaccgctcccgccatctgccacgacggcaaggcccacttccctagagagggcgtgttcgtgagcaacggcacccactggttcgtgacacagagaaacttctacgagcctcagatcatcaccaccgacaacaccttcgtgagcggcaactgcgacgtggtgatcggcatagtgaacaacaccgtatacgaccccctgcagcccgagctggacagcttcaaggaggagctggacaagtacttcaaaaaccatactagccccgacgtggacctgggagacatctctggcatcaacgctagcgtggtgaacattcagaaggagatcgaccggctgaatgaggtggccaagaacctgaacgagagcctgatcgacctgcaagagctgggcaagtacgagcagtacatcaagtggccctggtacatctggctgggcttcatcgccggcctgatcgccatcgtgatggtgaccatcatgctgtgctgcatgacaagctgttgcagctgcctgaaaggttgctgcagctgtggctcgtgctgcaagttcgacgaggacgacagcgagcccgtgctgaagggcgtgaagctgcactacacctgatga

SEQ ID NO: 21 - protein, 1270 aa, synthetic construct
  source 1..1270: note = B.1.351 Spike
MFVFLVLLPLVSSQCVNFTTRTQLPPAYTNSFTRGVYYPDKVFRSSVLHSTQDLFLPFFSNVTWFHAIHVSGTNGTKRFANPVLPFNDGVYFASTEKSNIIRGWIFGTTLDSKTQSLLIVNNATNVVIKVCEFQFCNDPFLGVYYHKNNKSWMESEFRVYSSANNCTFEYVSQPFLMDLEGKQGNFKNLREFVFKNIDGYFKIYSKHTPINLVRGLPQGFSALEPLVDLPIGINITRFQTLHRSYLTPGDSSSGWTAGAAAYYVGYLQPRTFLLKYNENGTITDAVDCALDPLSETKCTLKSFTVEKGIYQTSNFRVQPTESIVRFPNITNLCPFGEVFNATRFASVYAWNRKRISNCVADYSVLYNSASFSTFKCYGVSPTKLNDLCFTNVYADSFVIRGDEVRQIAPGQTGNIADYNYKLPDDFTGCVIAWNSNNLDSKVGGNYNYLYRLFRKSNLKPFERDISTEIYQAGSTPCNGVKGFNCYFPLQSYGFQPTYGVGYQPYRVVVLSFELLHAPATVCGPKKSTNLVKNKCVNFNFNGLTGTGVLTESNKKFLPFQQFGRDIADTTDAVRDPQTLEILDITPCSFGGVSVITPGTNTSNQVAVLYQGVNCTEVPVAIHADQLTPTWRVYSTGSNVFQTRAGCLIGAEHVNNSYECDIPIGAGICASYQTQTNSPRRARSVASQSIIAYTMSLGVENSVAYSNNSIAIPTNFTISVTTEILPVSMTKTSVDCTMYICGDSTECSNLLLQYGSFCTQLNRALTGIAVEQDKNTQEVFAQVKQIYKTPPIKDFGGFNFSQILPDPSKPSKRSFIEDLLFNKVTLADAGFIKQYGDCLGDIAARDLICAQKFNGLTVLPPLLTDEMIAQYTSALLAGTITSGWTFGAGAALQIPFAMQMAYRFNGIGVTQNVLYENQKLIANQFNSAIGKIQDSLSSTASALGKLQDVVNQNAQALNTLVKQLSSNFGAISSVLNDILSRLDPPEAEVQIDRLITGRLQSLQTYVTQQLIRAAEIRASANLAATKMSECVLGQSKRVDFCGKGYHLMSFPQSAPHGVVFLHVTYVPAQEKNFTTAPAICHDGKAHFPREGVFVSNGTHWFVTQRNFYEPQIITTDNTFVSGNCDVVIGIVNNTVYDPLQPELDSFKEELDKYFKNHTSPDVDLGDISGINASVVNIQKEIDRLNEVAKNLNESLIDLQELGKYEQYIKWPWYIWLGFIAGLIAIVMVTIMLCCMTSCCSCLKGCCSCGSCCKFDEDDSEPVLKGVKLHYT

SEQ ID NO: 22 - DNA, 3816 bp, synthetic construct
  source 1..3816: mol_type = other DNA; note = B.1.1.7 Spike CDS
atgttcgtgttcctggtgctgctgcccctggtgagctctcagtgcgtgaacctgaccacaagaacacagctgccccccgcctacaccaacagcttcacaagaggcgtgtactaccccgacaaggtgttcagaagcagcgtgctgcactccacccaagacctgtttctgcccttcttcagcaacgtgacctggttccacgccatcagcggcaccaacggcaccaagagattcgacaaccccgtgctgcccttcaacgacggcgtgtacttcgctagcaccgaaaagagcaacatcatcagaggctggatcttcggcaccaccctagactccaagacacaaagcctgctgatcgttaacaacgcgaccaacgtggtgatcaaggtgtgcgagtttcagttctgcaacgaccccttcctgggcgtgtaccacaagaacaacaagagctggatggagagcgagttccgtgtctacagcagcgccaacaactgcaccttcgagtacgtgtctcagcccttcctgatggacctggagggcaagcaaggcaatttcaagaacctaagagagttcgtgttcaagaacatcgacggctacttcaagatctacagcaagcacacccccatcaacctggtgagagacctgccccaaggcttcagcgccctggagcccctggtggacctgcccatcggcatcaacatcacaagatttcagaccctgctggccctgcaccgtagctacctaacccccggcgatagttcctctggctggacggccggcgctgccgcctactacgtgggctacctgcagcctagaaccttcctgctgaagtacaacgagaacggcactatcactgatgccgtggactgtgccctggaccccctgagcgagaccaagtgcaccctcaagagcttcaccgtggagaagggcatctatcagacaagcaacttcagagtgcagcccaccgagagcatcgtgagattccccaacatcaccaacctgtgccccttcggcgaggtgttcaacgccacaagattcgctagcgtgtacgcgtggaacagaaagagaatcagcaactgcgtggccgactacagcgtgctgtacaacagcgctagcttcagcaccttcaagtgctatggcgtcagccccaccaagctgaacgacctgtgcttcaccaacgtgtacgccgacagcttcgtgatcagaggcgacgaggtgagacagattgcccccgggcaaaccggcaagatcgccgactacaactacaagctgcccgacgacttcaccggctgcgtgatcgcgtggaacagcaataacctggattccaaggtgggcggcaactacaactacctgtacagactgttcagaaagagcaacctgaagcccttcgagagagacatcagcaccgagatctaccaagccggcagcaccccctgcaacggcgtggagggcttcaactgctacttccccctgcagagctacggctttcagcccacctacggcgtgggctatcagccctacagagtggtggtgctgagcttcgagctgctgcacgcccccgcaaccgtgtgcggccccaaaaagagcaccaacctggtgaagaacaagtgcgtgaacttcaactttaatggccttaccggcacgggcgtgctgaccgagagcaacaagaagttcctgccatttcagcaattcggcagagacatcgacgacaccaccgacgcggtcagagaccctcagaccctggagatcctggacatcaccccctgtagcttcggcggcgtgagcgtgatcacccccggcactaacacaagcaaccaagtggccgtgctgtaccaaggcgtgaactgcaccgaggtgcccgtggccatccacgccgatcagctgacccccacctggagagtatacagcaccggaagcaacgtgtttcagacaagagccggctgcctgatcggcgccgagcacgtgaacaacagctacgagtgcgacatccccatcggcgccggcatctgcgctagctatcagacacagaccaacagccaccggagagctagaagcgtggcttctcagagcatcatcgcctacaccatgagcctgggcgccgagaacagcgtggcctacagcaacaacagcatcgccatccccatcaacttcaccatcagcgtgaccaccgagatcctgcccgtaagtatgaccaagacaagcgtggactgcaccatgtacatctgcggcgacagcaccgagtgcagcaacctgctgctgcagtacggcagcttctgcacacagctgaacagagccctgaccggcatcgccgtggagcaagacaagaacacccaagaggtgttcgcccaagtgaagcagatctacaagaccccccccatcaaggacttcggcggcttcaacttcagccaaatcctgcccgaccctagcaagcctagcaagcggagcttcatcgaggacctgctgttcaacaaggtgaccctggccgacgccggcttcatcaagcagtacggcgactgcctaggcgacatcgcagctagagacctgatctgcgctcagaagttcaatggactcaccgtgctcccccccctgctgaccgacgagatgatcgctcagtacacctctgccctgctggcgggaaccataacaagcggttggacatttggcgccggggccgcactgcaaatccccttcgccatgcagatggcctacagattcaacggcatcggcgtgacacagaacgtgctgtacgagaatcagaagctgatcgccaatcagttcaacagcgccatcggcaagatccaagacagcctgagcagcaccgctagcgccctgggcaagctgcaagacgtggtgaatcagaacgcccaagccctgaacaccctggtgaagcagctgagcagcaacttcggcgccatcagcagcgtattgaatgacatcctggctagactggacccccccgaggccgaggtgcagatcgacagactgatcaccggcagactgcagagcctgcagacctacgtgacacagcagctgatcagagccgccgagatcagagctagcgccaacctggccgccaccaagatgagcgagtgcgtgctggggcagagcaagagagtggacttctgcggcaagggctaccacctgatgagcttccctcagagcgccccccacggcgtggtgttcctgcacgtgacctacgtgcccgcccaagagaagaacttcaccaccgctcccgccatctgccacgacggcaaggcccacttccctagagagggcgtgttcgtgagcaacggcacccactggttcgtgacacagagaaacttctacgagcctcagatcatcaccacccacaacaccttcgtgagcggcaactgcgacgtggtgatcggcatagtgaacaacaccgtatacgaccccctgcagcccgagctggacagcttcaaggaggagctggacaagtacttcaaaaaccatactagccccgacgtggacctgggagacatctctggcatcaacgctagcgtggtgaacattcagaaggagatcgaccggctgaatgaggtggccaagaacctgaacgagagcctgatcgacctgcaagagctgggcaagtacgagcagtacatcaagtggccctggtacatctggctgggcttcatcgccggcctgatcgccatcgtgatggtgaccatcatgctgtgctgcatgacaagctgttgcagctgcctgaaaggttgctgcagctgtggctcgtgctgcaagttcgacgaggacgacagcgagcccgtgctgaagggcgtgaagctgcactacacctgatga

SEQ ID NO: 23 - protein, 1270 aa, synthetic construct
  source 1..1270: note = B.1.1.7 Spike
MFVFLVLLPLVSSQCVNLTTRTQLPPAYTNSFTRGVYYPDKVFRSSVLHSTQDLFLPFFSNVTWFHAISGTNGTKRFDNPVLPFNDGVYFASTEKSNIIRGWIFGTTLDSKTQSLLIVNNATNVVIKVCEFQFCNDPFLGVYHKNNKSWMESEFRVYSSANNCTFEYVSQPFLMDLEGKQGNFKNLREFVFKNIDGYFKIYSKHTPINLVRDLPQGFSALEPLVDLPIGINITRFQTLLALHRSYLTPGDSSSGWTAGAAAYYVGYLQPRTFLLKYNENGTITDAVDCALDPLSETKCTLKSFTVEKGIYQTSNFRVQPTESIVRFPNITNLCPFGEVFNATRFASVYAWNRKRISNCVADYSVLYNSASFSTFKCYGVSPTKLNDLCFTNVYADSFVIRGDEVRQIAPGQTGKIADYNYKLPDDFTGCVIAWNSNNLDSKVGGNYNYLYRLFRKSNLKPFERDISTEIYQAGSTPCNGVEGFNCYFPLQSYGFQPTYGVGYQPYRVVVLSFELLHAPATVCGPKKSTNLVKNKCVNFNFNGLTGTGVLTESNKKFLPFQQFGRDIDDTTDAVRDPQTLEILDITPCSFGGVSVITPGTNTSNQVAVLYQGVNCTEVPVAIHADQLTPTWRVYSTGSNVFQTRAGCLIGAEHVNNSYECDIPIGAGICASYQTQTNSHRRARSVASQSIIAYTMSLGAENSVAYSNNSIAIPINFTISVTTEILPVSMTKTSVDCTMYICGDSTECSNLLLQYGSFCTQLNRALTGIAVEQDKNTQEVFAQVKQIYKTPPIKDFGGFNFSQILPDPSKPSKRSFIEDLLFNKVTLADAGFIKQYGDCLGDIAARDLICAQKFNGLTVLPPLLTDEMIAQYTSALLAGTITSGWTFGAGAALQIPFAMQMAYRFNGIGVTQNVLYENQKLIANQFNSAIGKIQDSLSSTASALGKLQDVVNQNAQALNTLVKQLSSNFGAISSVLNDILARLDPPEAEVQIDRLITGRLQSLQTYVTQQLIRAAEIRASANLAATKMSECVLGQSKRVDFCGKGYHLMSFPQSAPHGVVFLHVTYVPAQEKNFTTAPAICHDGKAHFPREGVFVSNGTHWFVTQRNFYEPQIITTHNTFVSGNCDVVIGIVNNTVYDPLQPELDSFKEELDKYFKNHTSPDVDLGDISGINASVVNIQKEIDRLNEVAKNLNESLIDLQELGKYEQYIKWPWYIWLGFIAGLIAIVMVTIMLCCMTSCCSCLKGCCSCGSCCKFDEDDSEPVLKGVKLHYT

SEQ ID NO: 24 - DNA, 3825 bp, synthetic construct
  source 1..3825: mol_type = other DNA; note = SARS-COV-2 Spike CDS
atgttcgtgttcctggtgctgctgcccctggtgagctctcagtgcgtgaacctgaccacaagaacacagctgccccccgcctacaccaacagcttcacaagaggcgtgtactaccccgacaaggtgttcagaagcagcgtgctgcactccacccaagacctgtttctgcccttcttcagcaacgtgacctggttccacgccatccacgtgagcggcaccaacggcaccaagagattcgacaaccccgtgctgcccttcaacgacggcgtgtacttcgctagcaccgaaaagagcaacatcatcagaggctggatcttcggcaccaccctagactccaagacacaaagcctgctgatcgttaacaacgcgaccaacgtggtgatcaaggtgtgcgagtttcagttctgcaacgaccccttcctgggcgtgtactaccacaagaacaacaagagctggatggagagcgagttccgtgtctacagcagcgccaacaactgcaccttcgagtacgtgtctcagcccttcctgatggacctggagggcaagcaaggcaatttcaagaacctaagagagttcgtgttcaagaacatcgacggctacttcaagatctacagcaagcacacccccatcaacctggtgagagacctgccccaaggcttcagcgccctggagcccctggtggacctgcccatcggcatcaacatcacaagatttcagaccctgctggccctgcaccgtagctacctaacccccggcgatagttcctctggctggacggccggcgctgccgcctactacgtgggctacctgcagcctagaaccttcctgctgaagtacaacgagaacggcactatcactgatgccgtggactgtgccctggaccccctgagcgagaccaagtgcaccctcaagagcttcaccgtggagaagggcatctatcagacaagcaacttcagagtgcagcccaccgagagcatcgtgagattccccaacatcaccaacctgtgccccttcggcgaggtgttcaacgccacaagattcgctagcgtgtacgcgtggaacagaaagagaatcagcaactgcgtggccgactacagcgtgctgtacaacagcgctagcttcagcaccttcaagtgctatggcgtcagccccaccaagctgaacgacctgtgcttcaccaacgtgtacgccgacagcttcgtgatcagaggcgacgaggtgagacagattgcccccgggcaaaccggcaagatcgccgactacaactacaagctgcccgacgacttcaccggctgcgtgatcgcgtggaacagcaataacctggattccaaggtgggcggcaactacaactacctgtacagactgttcagaaagagcaacctgaagcccttcgagagagacatcagcaccgagatctaccaagccggcagcaccccctgcaacggcgtggagggcttcaactgctacttccccctgcagagctacggctttcagcccaccaatggcgtgggctatcagccctacagagtggtggtgctgagcttcgagctgctgcacgcccccgcaaccgtgtgcggccccaaaaagagcaccaacctggtgaagaacaagtgcgtgaacttcaactttaatggccttaccggcacgggcgtgctgaccgagagcaacaagaagttcctgccatttcagcaattcggcagagacatcgccgacaccaccgacgcggtcagagaccctcagaccctggagatcctggacatcaccccctgtagcttcggcggcgtgagcgtgatcacccccggcactaacacaagcaaccaagtggccgtgctgtaccaagacgtgaactgcaccgaggtgcccgtggccatccacgccgatcagctgacccccacctggagagtatacagcaccggaagcaacgtgtttcagacaagagccggctgcctgatcggcgccgagcacgtgaacaacagctacgagtgcgacatccccatcggcgccggcatctgcgctagctatcagacacagaccaacagccctcggagagctagaagcgtggcttctcagagcatcatcgcctacaccatgagcctgggcgccgagaacagcgtggcctacagcaacaacagcatcgccatccccaccaacttcaccatcagcgtgaccaccgagatcctgcccgtaagtatgaccaagacaagcgtggactgcaccatgtacatctgcggcgacagcaccgagtgcagcaacctgctgctgcagtacggcagcttctgcacacagctgaacagagccctgaccggcatcgccgtggagcaagacaagaacacccaagaggtgttcgcccaagtgaagcagatctacaagaccccccccatcaaggacttcggcggcttcaacttcagccaaatcctgcccgaccctagcaagcctagcaagcggagcttcatcgaggacctgctgttcaacaaggtgaccctggccgacgccggcttcatcaagcagtacggcgactgcctaggcgacatcgcagctagagacctgatctgcgctcagaagttcaatggactcaccgtgctcccccccctgctgaccgacgagatgatcgctcagtacacctctgccctgctggcgggaaccataacaagcggttggacatttggcgccggggccgcactgcaaatccccttcgccatgcagatggcctacagattcaacggcatcggcgtgacacagaacgtgctgtacgagaatcagaagctgatcgccaatcagttcaacagcgccatcggcaagatccaagacagcctgagcagcaccgctagcgccctgggcaagctgcaagacgtggtgaatcagaacgcccaagccctgaacaccctggtgaagcagctgagcagcaacttcggcgccatcagcagcgtattgaatgacatcctgagcagactggacccccccgaggccgaggtgcagatcgacagactgatcaccggcagactgcagagcctgcagacctacgtgacacagcagctgatcagagccgccgagatcagagctagcgccaacctggccgccaccaagatgagcgagtgcgtgctggggcagagcaagagagtggacttctgcggcaagggctaccacctgatgagcttccctcagagcgccccccacggcgtggtgttcctgcacgtgacctacgtgcccgcccaagagaagaacttcaccaccgctcccgccatctgccacgacggcaaggcccacttccctagagagggcgtgttcgtgagcaacggcacccactggttcgtgacacagagaaacttctacgagcctcagatcatcaccaccgacaacaccttcgtgagcggcaactgcgacgtggtgatcggcatagtgaacaacaccgtatacgaccccctgcagcccgagctggacagcttcaaggaggagctggacaagtacttcaaaaaccatactagccccgacgtggacctgggagacatctctggcatcaacgctagcgtggtgaacattcagaaggagatcgaccggctgaatgaggtggccaagaacctgaacgagagcctgatcgacctgcaagagctgggcaagtacgagcagtacatcaagtggccctggtacatctggctgggcttcatcgccggcctgatcgccatcgtgatggtgaccatcatgctgtgctgcatgacaagctgttgcagctgcctgaaaggttgctgcagctgtggctcgtgctgcaagttcgacgaggacgacagcgagcccgtgctgaagggcgtgaagctgcactacacctgatga

SEQ ID NO: 25 - protein, 1273 aa, synthetic construct
  source 1..1273: note = SARS-COV-2 Spike
MFVFLVLLPLVSSQCVNLTTRTQLPPAYTNSFTRGVYYPDKVFRSSVLHSTQDLFLPFFSNVTWFHAIHVSGTNGTKRFDNPVLPFNDGVYFASTEKSNIIRGWIFGTTLDSKTQSLLIVNNATNVVIKVCEFQFCNDPFLGVYYHKNNKSWMESEFRVYSSANNCTFEYVSQPFLMDLEGKQGNFKNLREFVFKNIDGYFKIYSKHTPINLVRDLPQGFSALEPLVDLPIGINITRFQTLLALHRSYLTPGDSSSGWTAGAAAYYVGYLQPRTFLLKYNENGTITDAVDCALDPLSETKCTLKSFTVEKGIYQTSNFRVQPTESIVRFPNITNLCPFGEVFNATRFASVYAWNRKRISNCVADYSVLYNSASFSTFKCYGVSPTKLNDLCFTNVYADSFVIRGDEVRQIAPGQTGKIADYNYKLPDDFTGCVIAWNSNNLDSKVGGNYNYLYRLFRKSNLKPFERDISTEIYQAGSTPCNGVEGFNCYFPLQSYGFQPTNGVGYQPYRVVVLSFELLHAPATVCGPKKSTNLVKNKCVNFNFNGLTGTGVLTESNKKFLPFQQFGRDIADTTDAVRDPQTLEILDITPCSFGGVSVITPGTNTSNQVAVLYQDVNCTEVPVAIHADQLTPTWRVYSTGSNVFQTRAGCLIGAEHVNNSYECDIPIGAGICASYQTQTNSPRRARSVASQSIIAYTMSLGAENSVAYSNNSIAIPTNFTISVTTEILPVSMTKTSVDCTMYICGDSTECSNLLLQYGSFCTQLNRALTGIAVEQDKNTQEVFAQVKQIYKTPPIKDFGGFNFSQILPDPSKPSKRSFIEDLLFNKVTLADAGFIKQYGDCLGDIAARDLICAQKFNGLTVLPPLLTDEMIAQYTSALLAGTITSGWTFGAGAALQIPFAMQMAYRFNGIGVTQNVLYENQKLIANQFNSAIGKIQDSLSSTASALGKLQDVVNQNAQALNTLVKQLSSNFGAISSVLNDILSRLDPPEAEVQIDRLITGRLQSLQTYVTQQLIRAAEIRASANLAATKMSECVLGQSKRVDFCGKGYHLMSFPQSAPHGVVFLHVTYVPAQEKNFTTAPAICHDGKAHFPREGVFVSNGTHWFVTQRNFYEPQIITTDNTFVSGNCDVVIGIVNNTVYDPLQPELDSFKEELDKYFKNHTSPDVDLGDISGINASVVNIQKEIDRLNEVAKNLNESLIDLQELGKYEQYIKWPWYIWLGFIAGLIAIVMVTIMLCCMTSCCSCLKGCCSCGSCCKFDEDDSEPVLKGVKLHYT

SEQ ID NO: 26 - DNA, 1653 bp, synthetic construct
  source 1..1653: mol_type = other DNA; note = Luciferase CDS
atggaggacgccaagaacatcaagaaaggccccgcccccttctaccccctggaggacggcaccgccggcgagcagctgcacaaagccatgaaaagatacgctctggtgcccggcaccatcgccttcaccgacgcccacatcgaggtgaacatcacctacgccgagtacttcgagatgagcgtgagactggccgaggctatgaagagatacggcttgaacaccaaccacagaatcgtggtgtgcagcgagaacagcctgcagttcttcatgcccgtgctgggcgccctgttcatcggcgtggccgttgcccccgccaacgacatctacaacgagagagagctgctgaacagcatgaacatctctcagcccaccgtggttttcgtgtccaaaaagggcctgcagaagatcctgaacgtgcagaagaagctgcccatcattcagaagatcatcatcatggacagcaagaccgactaccaaggctttcagagcatgtacaccttcgtgacaagccacctgccccccggcttcaacgagtacgacttcgtgcccgagagcttcgacagagacaagaccatcgccctgatcatgaacagcagcggcagcaccggcctgcccaagggcgtggccctgccccacagaaccgcctgcgtgagattcagccacgctagagaccccatcttcggcaatcagatcatccccgacaccgccatcctgagcgtagtgcctttccatcatggcttcggcatgttcaccaccctgggctacctgatctgcggcttcagagtggtgctgatgtacagattcgaggaggagctgttcctgagaagcctgcaagactacaagattcagagcgccctgctggtgcccaccctgttcagcttcttcgccaagagcaccctgatcgacaagtatgacctgagcaacctgcacgaaattgcgagcggcggagcgccgctcagcaaagaggtgggcgaggccgtggccaagagattccacctgcccggcatcagacaaggctacggcctgaccgagaccacaagcgccatcctgatcacccccgagggcgacgataagcccggcgccgtgggcaaggtggtaccattcttcgaggccaaggtggtggacctggacaccggcaagaccctgggcgtgaatcagagaggcgagctgtgcgtgagaggccccatgatcatgagcggctacgtgaacaaccccgaggccaccaacgccctcatcgataaggatgggtggctgcacagcggcgacatcgcctactgggacgaggacgagcacttcttcatcgtggacagactcaagagcctgatcaagtacaagggctaccaagtggcccccgccgagttggagagcatcctgctgcagcaccccaatatcttcgacgctggcgtggccggactacccgacgacgacgccggcgagttacccgccgccgtggtggtgctggagcacggcaagaccatgaccgagaaggagatcgtggactacgtggctagccaagtgaccaccgccaagaagctgagaggcggcgtggtgttcgttgacgaagtgcccaagggcctgaccggcaagctggacgctagaaagatcagagagatcctgatcaaggccaagaagggcggcaagagcaagctgtga

SEQ ID NO: 27 - protein, 550 aa, synthetic construct
  source 1..550: note = Luciferase
MEDAKNIKKGPAPFYPLEDGTAGEQLHKAMKRYALVPGTIAFTDAHIEVNITYAEYFEMSVRLAEAMKRYGLNTNHRIVVCSENSLQFFMPVLGALFIGVAVAPANDIYNERELLNSMNISQPTVVFVSKKGLQKILNVQKKLPIIQKIIIMDSKTDYQGFQSMYTFVTSHLPPGFNEYDFVPESFDRDKTIALIMNSSGSTGLPKGVALPHRTACVRFSHARDPIFGNQIIPDTAILSVVPFHHGFGMFTTLGYLICGFRVVLMYRFEEELFLRSLQDYKIQSALLVPTLFSFFAKSTLIDKYDLSNLHEIASGGAPLSKEVGEAVAKRFHLPGIRQGYGLTETTSAILITPEGDDKPGAVGKVVPFFEAKVVDLDTGKTLGVNQRGELCVRGPMIMSGYVNNPEATNALIDKDGWLHSGDIAYWDEDEHFFIVDRLKSLIKYKGYQVAPAELESILLQHPNIFDAGVAGLPDDDAGELPAAVVVLEHGKTMTEKEIVDYVASQVTTAKKLRGGVVFVDEVPKGLTGKLDARKIREILIKAKKGGKSKL

SEQ ID NO: 28 - DNA, 59 bp, synthetic construct
  source 1..59: mol_type = other DNA; note; note (original language) = LUC1- I' truncation
taggagttggtggcagtttcaataacaggtcattgccgagaaaaggatagcactataat

SEQ ID NO: 29 - DNA, 55 bp, synthetic construct
  source 1..55: mol_type = other DNA; note; note (original language) = LUC2- I' truncation
agttggtggcagtttcaataacaggtcattgccgagaaaaggatagcactataat

SEQ ID NO: 30 - DNA, 51 bp, synthetic construct
  source 1..51: mol_type = other DNA; note; note (original language) = LUC3- I' truncation
ggtggcagtttcaataacaggtcattgccgagaaaaggatagcactataat

SEQ ID NO: 31 - DNA, 47 bp, synthetic construct
  source 1..47: mol_type = other DNA; note; note (original language) = LUC4- I' truncation
gcagtttcaataacaggtcattgccgagaaaaggatagcactataat

SEQ ID NO: 32 - DNA, 43 bp, synthetic construct
  source 1..43: mol_type = other DNA; note; note (original language) = LUC5- I' truncation
tttcaataacaggtcattgccgagaaaaggatagcactataat

SEQ ID NO: 33 - DNA, 39 bp, synthetic construct
  source 1..39: mol_type = other DNA; note; note (original language) = LUC6- I' truncation
aataacaggtcattgccgagaaaaggatagcactataat

SEQ ID NO: 34 - DNA, 35 bp, synthetic construct
  source 1..35: mol_type = other DNA; note; note (original language) = LUC7- I' truncation
acaggtcattgccgagaaaaggatagcactataat

SEQ ID NO: 35 - DNA, 31 bp, synthetic construct
  source 1..31: mol_type = other DNA; note; note (original language) = LUC8- I' truncation
gtcattgccgagaaaaggatagcactataat

SEQ ID NO: 36 - DNA, 27 bp, synthetic construct
  source 1..27: mol_type = other DNA; note; note (original language) = LUC9- I' truncation
ttgccgagaaaaggatagcactataat

SEQ ID NO: 37 - DNA, 23 bp, synthetic construct
  source 1..23: mol_type = other DNA; note; note (original language) = LUC10- I' truncation
cgagaaaaggatagcactataat

SEQ ID NO: 38 - DNA, 19 bp, synthetic construct
  source 1..19: mol_type = other DNA; note; note (original language) = LUC11- I' truncation
aaaaggatagcactataat

SEQ ID NO: 39 - DNA, 15 bp, synthetic construct
  source 1..15: mol_type = other DNA; note; note (original language) = LUC12- I' truncation
ggatagcactataat

SEQ ID NO: 40 - DNA, 11 bp, synthetic construct
  source 1..11: mol_type = other DNA; note; note (original language) = LUC13- I' truncation
agcactataat

SEQ ID NO: 41 - DNA, 21 bp, synthetic construct
  source 1..21: mol_type = other DNA; note; note (original language) = 5'UTR truncation
tcaataacaggtcattgccga

SEQ ID NO: 42 - DNA, 63 bp, synthetic construct
  source 1..63: mol_type = other DNA; note; note (original language) = LUC15- I' mutant
gagttaggagttgctggcagtttcaataacaggtcattgccgagaaaaggatagcactataat

SEQ ID NO: 43 - DNA, 63 bp, synthetic construct
  source 1..63: mol_type = other DNA; note; note (original language) = LUC16- I' mutant
gagttaggagttgttggcagtttcaataacaggtcattgccgagaaaaggatagcactataat

SEQ ID NO: 44 - DNA, 63 bp, synthetic construct
  source 1..63: mol_type = other DNA; note; note (original language) = 5'UTR I general formula
  misc_difference 14: note; note (original language) = N is selected from the group consisting of A, G, C, and T
gagttaggagttgntggcagtttcaataacaggtcattgccgagaaaaggatagcactataat

SEQ ID NO: 45 - RNA, 63 nt, synthetic construct
  source 1..63: mol_type = other RNA; note = 5'UTR I
gagttaggagttgatggcagtttcaataacaggtcattgccgagaaaaggatagcactataat

SEQ ID NO: 46 - RNA, 63 nt, synthetic construct
  source 1..63: mol_type = other RNA; note = 5'UTR I'
gagttaggagttggtggcagtttcaataacaggtcattgccgagaaaaggatagcactataat

SEQ ID NO: 47 - RNA, 43 nt, synthetic construct
  source 1..43: mol_type = other RNA; note = 5'UTR G
gcacttttctgagcagacgtccagagcagagtcagccgccacc

SEQ ID NO: 48 - RNA, 52 nt, synthetic construct
  source 1..52: mol_type = other RNA; note = 5'UTR A
acatttgcttctgacacaactgtgttcactagcaacctcaaacgccgccacc

SEQ ID NO: 49 - RNA, 55 nt, synthetic construct
  source 1..55: mol_type = other RNA; note = 5'UTR J
agagaggcaaagaaacattgtgaaatctccaactcttaaccttcaagccgccacc

SEQ ID NO: 50 - RNA, 134 nt, synthetic construct
  source 1..134: mol_type = other RNA; note = 3'UTR B
gctcgctttcttgctgtccaatttctattaaaggttcctttgttccctaagtccaactactaaactgggggatattatgaagggccttgagcatctggattctgcctaataaaaaacatttattttcattgcaa

SEQ ID NO: 51 - RNA, 180 nt, synthetic construct
  source 1..180: mol_type = other RNA; note = 3'UTR F
cagacaagacaagctactgaatacgttcacatctgtcttgatgcctaatatttttacatttctgtaaacatatttctgaaatattttttgcctttcaagcgacagatgcctcattttgtgaaaacttaatgatgattttgtgtttaagttccaaacatttgaataaaataattgacaata

SEQ ID NO: 52 - RNA, 388 nt, synthetic construct
  source 1..388: mol_type = other RNA; note = 3'UTR E
cctgaggcctcagaacacaggtttcagattgataggcctgcaggtctccaggcagcaaccagctgagcgactaaagggcccaaggccagggctctagggatggggctcagcagaggctggggtaaggggagccagggaggagctgggcctaatgcagcaccgggtccccaggatgccgtgtctcggctggaggaggagatgcggaagctccaggccacggtgcaggagctccagaagcgcttggacaggctggaggagacagtccaggccaagtagagccccgcagggcctccagcagggtcagccattcacacccatccactcacctcccattcccagccacatggcagagaaaaaaatcataataaaatggctttattttctggta

SEQ ID NO: 53 - RNA, 296 nt, synthetic construct
  source 1..296: mol_type = other RNA; note = 3'UTR D
ggggccttctgacatgagtctggcctggccccacctcctagttcctcataataaagacagattgcttcttcgcttctcactgaggggccttctgacatgagtctggcctggccccacctccccagtttctcataataaagacagattgcttcttcacttgaagctcgctttcttgctgtccaatttctattaaaggttcctttgttccctaagtccaactactaaactgggggatattatgaagggccttgagcatctggattctgcctaataaaaaacatttattttcattgcaa

SEQ ID NO: 54 - RNA, 3819 nt, synthetic construct
  source 1..3819: mol_type = other RNA; note = B.1.617.2(Delta) spike mRNA
atgttcgtgttcctggtgctgctgcccctggtgagctctcagtgcgtgaacctgaggacaagaacacagctgccccccgcctacaccaacagcttcacaagaggcgtgtactaccccgacaaggtgttcagaagcagcgtgctgcactccacccaagacctgtttctgcccttcttcagcaacgtgacctggttccacgccatccacgtcagcggcaccaacggcaccaagagattcgacaaccccgtgctgcccttcaacgacggcgtgtacttcgctagcaccgaaaagagcaacatcatcagaggctggatcttcggcaccaccctagactccaagacacaaagcctgctgatcgttaacaacgcgaccaacgtggtgatcaaggtgtgcgagtttcagttctgcaacgaccccttcctggacgtgtactaccacaagaacaacaagagctggatggagagcggggtctacagcagcgccaacaactgcaccttcgagtacgtgtctcagcccttcctgatggacctggagggcaagcaaggcaatttcaagaacctaagagagttcgtgttcaagaacatcgacggctacttcaagatctacagcaagcacacccccatcaacctggtgagagacctgccccaaggcttcagcgccctggagcccctggtggacctgcccatcggcatcaacatcacaagatttcagaccctgctggccctgcaccgtagctacctaacccccggcgatagttcctctggctggacggccggcgctgccgcctactacgtgggctacctgcagcctagaaccttcctgctgaagtacaacgagaacggcactatcactgatgccgtggactgtgccctggaccccctgagcgagaccaagtgcaccctcaagagcttcaccgtggagaagggcatctatcagacaagcaacttcagagtgcagcccaccgagagcatcgtgagattccccaacatcaccaacctgtgccccttcggcgaggtgttcaacgccacaagattcgctagcgtgtacgcgtggaacagaaagagaatcagcaactgcgtggccgactacagcgtgctgtacaacagcgctagcttcagcaccttcaagtgctatggcgtcagccccaccaagctgaacgacctgtgcttcaccaacgtgtacgccgacagcttcgtgatcagaggcgacgaggtgagacagattgcccccgggcaaaccggcaagatcgccgactacaactacaagctgcccgacgacttcaccggctgcgtgatcgcgtggaacagcaataacctggattccaaggtgggcggcaactacaactaccggtacagactgttcagaaagagcaacctgaagcccttcgagagagacatcagcaccgagatctaccaagccggcagcaagccctgcaacggcgtggagggcttcaactgctacttccccctgcagagctacggctttcagcccaccaacggcgtgggctatcagccctacagagtggtggtgctgagcttcgagctgctgcacgcccccgcaaccgtgtgcggccccaaaaagagcaccaacctggtgaagaacaagtgcgtgaacttcaactttaatggccttaccggcacgggcgtgctgaccgagagcaacaagaagttcctgccatttcagcaattcggcagagacatcgccgacaccaccgacgcggtcagagaccctcagaccctggagatcctggacatcaccccctgtagcttcggcggcgtgagcgtgatcacccccggcactaacacaagcaaccaagtggccgtgctgtaccaaggcgtgaactgcaccgaggtgcccgtggccatccacgccgatcagctgacccccacctggagagtatacagcaccggaagcaacgtgtttcagacaagagccggctgcctgatcggcgccgagcacgtgaacaacagctacgagtgcgacatccccatcggcgccggcatctgcgctagctatcagacacagaccaacagccgccggagagctagaagcgtggcttctcagagcatcatcgcctacaccatgagcctgggcgccgagaacagcgtggcctacagcaacaacagcatcgccatccccaccaacttcaccatcagcgtgaccaccgagatcctgcccgtaagtatgaccaagacaagcgtggactgcaccatgtacatctgcggcgacagcaccgagtgcagcaacctgctgctgcagtacggcagcttctgcacacagctgaacagagccctgaccggcatcgccgtggagcaagacaagaacacccaagaggtgttcgcccaagtgaagcagatctacaagaccccccccatcaaggacttcggcggcttcaacttcagccaaatcctgcccgaccctagcaagcctagcaagcggagcttcatcgaggacctgctgttcaacaaggtgaccctggccgacgccggcttcatcaagcagtacggcgactgcctaggcgacatcgcagctagagacctgatctgcgctcagaagttcaatggactcaccgtgctcccccccctgctgaccgacgagatgatcgctcagtacacctctgccctgctggcgggaaccataacaagcggttggacatttggcgccggggccgcactgcaaatccccttcgccatgcagatggcctacagattcaacggcatcggcgtgacacagaacgtgctgtacgagaatcagaagctgatcgccaatcagttcaacagcgccatcggcaagatccaagacagcctgagcagcaccgctagcgccctgggcaagctgcaaaacgtggtgaatcagaacgcccaagccctgaacaccctggtgaagcagctgagcagcaacttcggcgccatcagcagcgtattgaatgacatcctgtctagactggacccccccgaggccgaggtgcagatcgacagactgatcaccggcagactgcagagcctgcagacctacgtgacacagcagctgatcagagccgccgagatcagagctagcgccaacctggccgccaccaagatgagcgagtgcgtgctggggcagagcaagagagtggacttctgcggcaagggctaccacctgatgagcttccctcagagcgccccccacggcgtggtgttcctgcacgtgacctacgtgcccgcccaagagaagaacttcaccaccgctcccgccatctgccacgacggcaaggcccacttccctagagagggcgtgttcgtgagcaacggcacccactggttcgtgacacagagaaacttctacgagcctcagatcatcaccaccgacaacaccttcgtgagcggcaactgcgacgtggtgatcggcatagtgaacaacaccgtatacgaccccctgcagcccgagctggacagcttcaaggaggagctggacaagtacttcaaaaaccatactagccccgacgtggacctgggagacatctctggcatcaacgctagcgtggtgaacattcagaaggagatcgaccggctgaatgaggtggccaagaacctgaacgagagcctgatcgacctgcaagagctgggcaagtacgagcagtacatcaagtggccctggtacatctggctgggcttcatcgccggcctgatcgccatcgtgatggtgaccatcatgctgtgctgcatgacaagctgttgcagctgcctgaaaggttgctgcagctgtggctcgtgctgcaagttcgacgaggacgacagcgagcccgtgctgaagggcgtgaagctgcactacacctgatga

SEQ ID NO: 55 - RNA, 3816 nt, synthetic construct
  source 1..3816: mol_type = other RNA; note = B.1.1.529(Omicron) spike mRNA
atgttcgtgttcctggtgctgctgcccctggtgagctctcagtgcgtgaacctgaccacaagaacacagctgccccccgcctacaccaacagcttcacaagaggcgtgtactaccccgacaaggtgttcagaagcagcgtgctgcactccacccaagacctgtttctgcccttcttcagcaacgtgacctggttccacgtgatcagcggcaccaacggcaccaagagattcgacaaccccgtgctgcccttcaacgacggcgtgtacttcgctagcatcgaaaagagcaacatcatcagaggctggatcttcggcaccaccctagactccaagacacaaagcctgctgatcgttaacaacgcgaccaacgtggtgatcaaggtgtgcgagtttcagttctgcaacgaccccttcctggaccacaagaacaacaagagctggatggagagcgagttcagagtgtacagcagcgccaacaactgcaccttcgagtacgtgtctcagcccttcctgatggacctggagggcaagcaaggcaatttcaagaacctaagagagttcgtgttcaagaacatcgacggctacttcaagatctacagcaagcacacccccatcatcgtgagagagcccgaggacctgccccaaggcttcagcgccctggagcccctggtggacctgcccatcggcatcaacatcacaagatttcagaccctgctggccctgcaccgtagctacctaacccccggcgatagttcctctggctggacggccggcgctgccgcctactacgtgggctacctgcagcctagaaccttcctgctgaagtacaacgagaacggcactatcactgatgccgtggactgtgccctggaccccctgagcgagaccaagtgcaccctcaagagcttcaccgtggagaagggcatctatcagacaagcaacttcagagtgcagcccaccgagagcatcgtgagattccccaacatcaccaacctgtgccccttcgacgaggtgttcaacgccaccagatttgctagcgtgtacgcctggaaccggaagagaatcagcaactgcgtggccgactacagcgtgctgtacaacctggcccccttcttcaccttcaagtgctatggcgtcagccccaccaagctgaacgacctgtgcttcaccaacgtgtacgccgacagcttcgtgatcagaggcgacgaggtgagacagatcgcccccgggcagaccggcaacatcgccgactacaactacaagctgcccgacgacttcaccggctgcgtgatcgcctggaacagcaacaagctggatagcaaggtgagcggcaactacaattacctgtacagactgttcagaaagagcaacctgaagcccttcgagagagacatcagcaccgagatctaccaagccggcaacaagccctgcaacggcgtggcgggcttcaactgctacttccccctcaggagctacagcttcagacccacctacggcgtgggccatcagccctacagagtggtcgtgctgagcttcgagctgctgcacgcccctgccacagtgtgcggccccaaaaagagcaccaacctggtgaagaacaagtgcgtgaacttcaacttcaacggcctgaagggcaccggcgtgctgaccgagagcaacaagaagttcctgccatttcagcaattcggcagagacatcgccgacaccaccgacgcggtcagagaccctcagaccctggagatcctggacatcaccccctgtagcttcggcggcgtgagcgtgatcacccccggcactaacacaagcaaccaagtggccgtgctgtaccaaggcgtgaactgcaccgaggtgcccgtggccatccacgccgatcagctgacccccacctggagagtgtatagcaccggcagcaacgtgtttcagacaagagccggctgcctgatcggcgccgagtacgtgaacaacagctacgagtgcgacatccccatcggcgccggcatctgcgctagctatcagacacagaccaagagccaccggagagctagaagcgtggctagccaaagcatcatcgcctacaccatgagcctgggcgccgagaacagcgtggcctacagcaacaacagcatcgccatccccaccaacttcaccatcagcgtgaccaccgagatcctgcccgtaagtatgaccaagacaagcgtggactgcaccatgtacatctgcggcgacagcaccgagtgcagcaacctgctcctgcagtacggcagcttctgcacacagctgaagagagccctgaccggcatcgccgtggagcaagacaagaacacccaagaggtgttcgcccaagtgaagcagatctacaagaccccccccatcaagtacttcggcggcttcaacttcagccaaatcctgcccgaccctagcaagcctagcaagcggagcttcatcgaggacctgctgttcaacaaggtgaccctggccgacgccggcttcatcaagcagtacggcgactgcctaggcgacatcgcagctagagacctgatctgcgctcagaagttcaagggactcaccgtgctcccccccctgctgaccgacgagatgatcgctcagtacacctctgccctgctggcgggaaccataacaagcggttggacatttggcgccggggccgcactgcaaatccccttcgccatgcagatggcctacagattcaacggcatcggcgtgacacagaacgtgctgtacgagaatcagaagctgatcgccaatcagttcaacagcgccatcggcaagatccaagacagcctgagcagcaccgctagcgccctgggcaagctgcaagacgtggtgaaccacaacgcccaagccctgaacaccctggtgaagcagctgagcagcaagttcggcgccatcagcagcgtgctgaatgacatcttctctagactggacccccccgaggccgaggtgcagatcgacagactgatcaccggcagactgcagagcctgcagacctacgtgacacagcagctgatcagagccgccgagatcagagctagcgccaacctggccgccaccaagatgagcgagtgcgtgctggggcagagcaagagagtggacttctgcggcaagggctaccacctgatgagcttccctcagagcgccccccacggcgtggtgttcctgcacgtgacctacgtgcccgcccaagagaagaacttcaccaccgctcccgccatctgccacgacggcaaggcccacttccctagagagggcgtgttcgtgagcaacggcacccactggttcgtgacacagagaaacttctacgagcctcagatcatcaccaccgacaacaccttcgtgagcggcaactgcgacgtggtgatcggcatagtgaacaacaccgtatacgaccccctgcagcccgagctggacagcttcaaggaggagctggacaagtacttcaaaaaccatactagccccgacgtggacctgggagacatctctggcatcaacgctagcgtggtgaacattcagaaggagatcgaccggctgaatgaggtggccaagaacctgaacgagagcctgatcgacctgcaagagctgggcaagtacgagcagtacatcaagtggccctggtacatctggctgggcttcatcgccggcctgatcgccatcgtgatggtgaccatcatgctgtgctgcatgacaagctgttgcagctgcctgaaaggttgctgcagctgtggctcgtgctgcaagttcgacgaggacgacagcgagcccgtgctgaagggcgtgaagctgcactacacctgatga

SEQ ID NO: 56 - RNA, 112 nt, synthetic construct
  source 1..112: mol_type = other RNA; note = poly A
aaaaaaaaaaaaaaaaaaaaaaaaaaaaaagcatatgactaaaaaaaaaaaaaaaaaaaaaaaaaaaaaaaaaaaaaaaaaaaaaaaaaaaaaaaaaaaaaaaaaaaaaaaa

SEQ ID NO: 57 - RNA, 4134 nt, synthetic construct
  source 1..4134: mol_type = other RNA; note = I'-Delta24-B mRNA
gagttaggagttggtggcagtttcaataacaggtcattgccgagaaaaggatagcactataatatgttcgtgttcctggtgctgctgcccctggtgagctctcagtgcgtgaacctgaggacaagaacacagctgccccccgcctacaccaacagcttcacaagaggcgtgtactaccccgacaaggtgttcagaagcagcgtgctgcactccacccaagacctgtttctgcccttcttcagcaacgtgacctggttccacgccatccacgtcagcggcaccaacggcaccaagagattcgacaaccccgtgctgcccttcaacgacggcgtgtacttcgctagcaccgaaaagagcaacatcatcagaggctggatcttcggcaccaccctagactccaagacacaaagcctgctgatcgttaacaacgcgaccaacgtggtgatcaaggtgtgcgagtttcagttctgcaacgaccccttcctggacgtgtactaccacaagaacaacaagagctggatggagagcggggtctacagcagcgccaacaactgcaccttcgagtacgtgtctcagcccttcctgatggacctggagggcaagcaaggcaatttcaagaacctaagagagttcgtgttcaagaacatcgacggctacttcaagatctacagcaagcacacccccatcaacctggtgagagacctgccccaaggcttcagcgccctggagcccctggtggacctgcccatcggcatcaacatcacaagatttcagaccctgctggccctgcaccgtagctacctaacccccggcgatagttcctctggctggacggccggcgctgccgcctactacgtgggctacctgcagcctagaaccttcctgctgaagtacaacgagaacggcactatcactgatgccgtggactgtgccctggaccccctgagcgagaccaagtgcaccctcaagagcttcaccgtggagaagggcatctatcagacaagcaacttcagagtgcagcccaccgagagcatcgtgagattccccaacatcaccaacctgtgccccttcggcgaggtgttcaacgccacaagattcgctagcgtgtacgcgtggaacagaaagagaatcagcaactgcgtggccgactacagcgtgctgtacaacagcgctagcttcagcaccttcaagtgctatggcgtcagccccaccaagctgaacgacctgtgcttcaccaacgtgtacgccgacagcttcgtgatcagaggcgacgaggtgagacagattgcccccgggcaaaccggcaagatcgccgactacaactacaagctgcccgacgacttcaccggctgcgtgatcgcgtggaacagcaataacctggattccaaggtgggcggcaactacaactaccggtacagactgttcagaaagagcaacctgaagcccttcgagagagacatcagcaccgagatctaccaagccggcagcaagccctgcaacggcgtggagggcttcaactgctacttccccctgcagagctacggctttcagcccaccaacggcgtgggctatcagccctacagagtggtggtgctgagcttcgagctgctgcacgcccccgcaaccgtgtgcggccccaaaaagagcaccaacctggtgaagaacaagtgcgtgaacttcaactttaatggccttaccggcacgggcgtgctgaccgagagcaacaagaagttcctgccatttcagcaattcggcagagacatcgccgacaccaccgacgcggtcagagaccctcagaccctggagatcctggacatcaccccctgtagcttcggcggcgtgagcgtgatcacccccggcactaacacaagcaaccaagtggccgtgctgtaccaaggcgtgaactgcaccgaggtgcccgtggccatccacgccgatcagctgacccccacctggagagtatacagcaccggaagcaacgtgtttcagacaagagccggctgcctgatcggcgccgagcacgtgaacaacagctacgagtgcgacatccccatcggcgccggcatctgcgctagctatcagacacagaccaacagccgccggagagctagaagcgtggcttctcagagcatcatcgcctacaccatgagcctgggcgccgagaacagcgtggcctacagcaacaacagcatcgccatccccaccaacttcaccatcagcgtgaccaccgagatcctgcccgtaagtatgaccaagacaagcgtggactgcaccatgtacatctgcggcgacagcaccgagtgcagcaacctgctgctgcagtacggcagcttctgcacacagctgaacagagccctgaccggcatcgccgtggagcaagacaagaacacccaagaggtgttcgcccaagtgaagcagatctacaagaccccccccatcaaggacttcggcggcttcaacttcagccaaatcctgcccgaccctagcaagcctagcaagcggagcttcatcgaggacctgctgttcaacaaggtgaccctggccgacgccggcttcatcaagcagtacggcgactgcctaggcgacatcgcagctagagacctgatctgcgctcagaagttcaatggactcaccgtgctcccccccctgctgaccgacgagatgatcgctcagtacacctctgccctgctggcgggaaccataacaagcggttggacatttggcgccggggccgcactgcaaatccccttcgccatgcagatggcctacagattcaacggcatcggcgtgacacagaacgtgctgtacgagaatcagaagctgatcgccaatcagttcaacagcgccatcggcaagatccaagacagcctgagcagcaccgctagcgccctgggcaagctgcaaaacgtggtgaatcagaacgcccaagccctgaacaccctggtgaagcagctgagcagcaacttcggcgccatcagcagcgtattgaatgacatcctgtctagactggacccccccgaggccgaggtgcagatcgacagactgatcaccggcagactgcagagcctgcagacctacgtgacacagcagctgatcagagccgccgagatcagagctagcgccaacctggccgccaccaagatgagcgagtgcgtgctggggcagagcaagagagtggacttctgcggcaagggctaccacctgatgagcttccctcagagcgccccccacggcgtggtgttcctgcacgtgacctacgtgcccgcccaagagaagaacttcaccaccgctcccgccatctgccacgacggcaaggcccacttccctagagagggcgtgttcgtgagcaacggcacccactggttcgtgacacagagaaacttctacgagcctcagatcatcaccaccgacaacaccttcgtgagcggcaactgcgacgtggtgatcggcatagtgaacaacaccgtatacgaccccctgcagcccgagctggacagcttcaaggaggagctggacaagtacttcaaaaaccatactagccccgacgtggacctgggagacatctctggcatcaacgctagcgtggtgaacattcagaaggagatcgaccggctgaatgaggtggccaagaacctgaacgagagcctgatcgacctgcaagagctgggcaagtacgagcagtacatcaagtggccctggtacatctggctgggcttcatcgccggcctgatcgccatcgtgatggtgaccatcatgctgtgctgcatgacaagctgttgcagctgcctgaaaggttgctgcagctgtggctcgtgctgcaagttcgacgaggacgacagcgagcccgtgctgaagggcgtgaagctgcactacacctgatgactcgaggctcgctttcttgctgtccaatttctattaaaggttcctttgttccctaagtccaactactaaactgggggatattatgaagggccttgagcatctggattctgcctaataaaaaacatttattttcattgcaaaaaaaaaaaaaaaaaaaaaaaaaaaaaaaagcatatgactaaaaaaaaaaaaaaaaaaaaaaaaaaaaaaaaaaaaaaaaaaaaaaaaaaaaaaaaaaaaaaaaaaaaaaaa

SEQ ID NO: 58 - RNA, 4131 nt, synthetic construct
  source 1..4131: mol_type = other RNA; note = I'-OC24-B mRNA
gagttaggagttggtggcagtttcaataacaggtcattgccgagaaaaggatagcactataatatgttcgtgttcctggtgctgctgcccctggtgagctctcagtgcgtgaacctgaccacaagaacacagctgccccccgcctacaccaacagcttcacaagaggcgtgtactaccccgacaaggtgttcagaagcagcgtgctgcactccacccaagacctgtttctgcccttcttcagcaacgtgacctggttccacgtgatcagcggcaccaacggcaccaagagattcgacaaccccgtgctgcccttcaacgacggcgtgtacttcgctagcatcgaaaagagcaacatcatcagaggctggatcttcggcaccaccctagactccaagacacaaagcctgctgatcgttaacaacgcgaccaacgtggtgatcaaggtgtgcgagtttcagttctgcaacgaccccttcctggaccacaagaacaacaagagctggatggagagcgagttcagagtgtacagcagcgccaacaactgcaccttcgagtacgtgtctcagcccttcctgatggacctggagggcaagcaaggcaatttcaagaacctaagagagttcgtgttcaagaacatcgacggctacttcaagatctacagcaagcacacccccatcatcgtgagagagcccgaggacctgccccaaggcttcagcgccctggagcccctggtggacctgcccatcggcatcaacatcacaagatttcagaccctgctggccctgcaccgtagctacctaacccccggcgatagttcctctggctggacggccggcgctgccgcctactacgtgggctacctgcagcctagaaccttcctgctgaagtacaacgagaacggcactatcactgatgccgtggactgtgccctggaccccctgagcgagaccaagtgcaccctcaagagcttcaccgtggagaagggcatctatcagacaagcaacttcagagtgcagcccaccgagagcatcgtgagattccccaacatcaccaacctgtgccccttcgacgaggtgttcaacgccaccagatttgctagcgtgtacgcctggaaccggaagagaatcagcaactgcgtggccgactacagcgtgctgtacaacctggcccccttcttcaccttcaagtgctatggcgtcagccccaccaagctgaacgacctgtgcttcaccaacgtgtacgccgacagcttcgtgatcagaggcgacgaggtgagacagatcgcccccgggcagaccggcaacatcgccgactacaactacaagctgcccgacgacttcaccggctgcgtgatcgcctggaacagcaacaagctggatagcaaggtgagcggcaactacaattacctgtacagactgttcagaaagagcaacctgaagcccttcgagagagacatcagcaccgagatctaccaagccggcaacaagccctgcaacggcgtggcgggcttcaactgctacttccccctcaggagctacagcttcagacccacctacggcgtgggccatcagccctacagagtggtcgtgctgagcttcgagctgctgcacgcccctgccacagtgtgcggccccaaaaagagcaccaacctggtgaagaacaagtgcgtgaacttcaacttcaacggcctgaagggcaccggcgtgctgaccgagagcaacaagaagttcctgccatttcagcaattcggcagagacatcgccgacaccaccgacgcggtcagagaccctcagaccctggagatcctggacatcaccccctgtagcttcggcggcgtgagcgtgatcacccccggcactaacacaagcaaccaagtggccgtgctgtaccaaggcgtgaactgcaccgaggtgcccgtggccatccacgccgatcagctgacccccacctggagagtgtatagcaccggcagcaacgtgtttcagacaagagccggctgcctgatcggcgccgagtacgtgaacaacagctacgagtgcgacatccccatcggcgccggcatctgcgctagctatcagacacagaccaagagccaccggagagctagaagcgtggctagccaaagcatcatcgcctacaccatgagcctgggcgccgagaacagcgtggcctacagcaacaacagcatcgccatccccaccaacttcaccatcagcgtgaccaccgagatcctgcccgtaagtatgaccaagacaagcgtggactgcaccatgtacatctgcggcgacagcaccgagtgcagcaacctgctcctgcagtacggcagcttctgcacacagctgaagagagccctgaccggcatcgccgtggagcaagacaagaacacccaagaggtgttcgcccaagtgaagcagatctacaagaccccccccatcaagtacttcggcggcttcaacttcagccaaatcctgcccgaccctagcaagcctagcaagcggagcttcatcgaggacctgctgttcaacaaggtgaccctggccgacgccggcttcatcaagcagtacggcgactgcctaggcgacatcgcagctagagacctgatctgcgctcagaagttcaagggactcaccgtgctcccccccctgctgaccgacgagatgatcgctcagtacacctctgccctgctggcgggaaccataacaagcggttggacatttggcgccggggccgcactgcaaatccccttcgccatgcagatggcctacagattcaacggcatcggcgtgacacagaacgtgctgtacgagaatcagaagctgatcgccaatcagttcaacagcgccatcggcaagatccaagacagcctgagcagcaccgctagcgccctgggcaagctgcaagacgtggtgaaccacaacgcccaagccctgaacaccctggtgaagcagctgagcagcaagttcggcgccatcagcagcgtgctgaatgacatcttctctagactggacccccccgaggccgaggtgcagatcgacagactgatcaccggcagactgcagagcctgcagacctacgtgacacagcagctgatcagagccgccgagatcagagctagcgccaacctggccgccaccaagatgagcgagtgcgtgctggggcagagcaagagagtggacttctgcggcaagggctaccacctgatgagcttccctcagagcgccccccacggcgtggtgttcctgcacgtgacctacgtgcccgcccaagagaagaacttcaccaccgctcccgccatctgccacgacggcaaggcccacttccctagagagggcgtgttcgtgagcaacggcacccactggttcgtgacacagagaaacttctacgagcctcagatcatcaccaccgacaacaccttcgtgagcggcaactgcgacgtggtgatcggcatagtgaacaacaccgtatacgaccccctgcagcccgagctggacagcttcaaggaggagctggacaagtacttcaaaaaccatactagccccgacgtggacctgggagacatctctggcatcaacgctagcgtggtgaacattcagaaggagatcgaccggctgaatgaggtggccaagaacctgaacgagagcctgatcgacctgcaagagctgggcaagtacgagcagtacatcaagtggccctggtacatctggctgggcttcatcgccggcctgatcgccatcgtgatggtgaccatcatgctgtgctgcatgacaagctgttgcagctgcctgaaaggttgctgcagctgtggctcgtgctgcaagttcgacgaggacgacagcgagcccgtgctgaagggcgtgaagctgcactacacctgatgactcgaggctcgctttcttgctgtccaatttctattaaaggttcctttgttccctaagtccaactactaaactgggggatattatgaagggccttgagcatctggattctgcctaataaaaaacatttattttcattgcaaaaaaaaaaaaaaaaaaaaaaaaaaaaaaaagcatatgactaaaaaaaaaaaaaaaaaaaaaaaaaaaaaaaaaaaaaaaaaaaaaaaaaaaaaaaaaaaaaaaaaaaaaaaa

SEQ ID NO: 59 - RNA, 3816 nt, synthetic construct
  source 1..3816: mol_type = other RNA; note = B.1.351 Spike mRNA
atgttcgtgttcctggtgctgctgcccctggtgagctctcagtgcgtgaacttcacgacaagaacacagctgccccccgcctacaccaacagcttcacaagaggcgtgtactaccccgacaaggtgttcagaagcagcgtgctgcactccacccaagacctgtttctgcccttcttcagcaacgtgacctggttccacgccatccacgtgagcggcaccaacggcaccaagagattcgccaaccccgtgctgcccttcaacgacggcgtgtacttcgctagcaccgaaaagagcaacatcatcagaggctggatcttcggcaccaccctagactccaagacacaaagcctgctgatcgttaacaacgcgaccaacgtggtgatcaaggtgtgcgagtttcagttctgcaacgaccccttcctgggcgtgtactaccacaagaacaacaagagctggatggagagcgagttccgtgtctacagcagcgccaacaactgcaccttcgagtacgtgtctcagcccttcctgatggacctggagggcaagcaaggcaatttcaagaacctaagagagttcgtgttcaagaacatcgacggctacttcaagatctacagcaagcacacccccatcaacctggtgagaggcctgccccaaggcttcagcgccctggagcccctggtggacctgcccatcggcatcaacatcacaagatttcagaccctgcaccgtagctacctaacccccggcgatagttcctctggctggacggccggcgctgccgcctactacgtgggctacctgcagcctagaaccttcctgctgaagtacaacgagaacggcactatcactgatgccgtggactgtgccctggaccccctgagcgagaccaagtgcaccctcaagagcttcaccgtggagaagggcatctatcagacaagcaacttcagagtgcagcccaccgagagcatcgtgagattccccaacatcaccaacctgtgccccttcggcgaggtgttcaacgccacaagattcgctagcgtgtacgcgtggaacagaaagagaatcagcaactgcgtggccgactacagcgtgctgtacaacagcgctagcttcagcaccttcaagtgctatggcgtcagccccaccaagctgaacgacctgtgcttcaccaacgtgtacgccgacagcttcgtgatcagaggcgacgaggtgagacagattgcccccgggcaaaccggcaacatcgccgactacaactacaagctgcccgacgacttcaccggctgcgtgatcgcgtggaacagcaataacctggattccaaggtgggcggcaactacaactacctgtacagactgttcagaaagagcaacctgaagcccttcgagagagacatcagcaccgagatctaccaagccggcagcaccccctgcaacggcgtgaagggcttcaactgctacttccccctgcagagctacggctttcagcccacctacggcgtgggctatcagccctacagagtggtggtgctgagcttcgagctgctgcacgcccccgcaaccgtgtgcggccccaaaaagagcaccaacctggtgaagaacaagtgcgtgaacttcaactttaatggccttaccggcacgggcgtgctgaccgagagcaacaagaagttcctgccatttcagcaattcggcagagacatcgccgacaccaccgacgcggtcagagaccctcagaccctggagatcctggacatcaccccctgtagcttcggcggcgtgagcgtgatcacccccggcactaacacaagcaaccaagtggccgtgctgtaccaaggcgtgaactgcaccgaggtgcccgtggccatccacgccgatcagctgacccccacctggagagtatacagcaccggaagcaacgtgtttcagacaagagccggctgcctgatcggcgccgagcacgtgaacaacagctacgagtgcgacatccccatcggcgccggcatctgcgctagctatcagacacagaccaacagcccccggagagctagaagcgtggcttctcagagcatcatcgcctacaccatgagcctgggcgtcgagaacagcgtggcctacagcaacaacagcatcgccatccccaccaacttcaccatcagcgtgaccaccgagatcctgcccgtaagtatgaccaagacaagcgtggactgcaccatgtacatctgcggcgacagcaccgagtgcagcaacctgctgctgcagtacggcagcttctgcacacagctgaacagagccctgaccggcatcgccgtggagcaagacaagaacacccaagaggtgttcgcccaagtgaagcagatctacaagaccccccccatcaaggacttcggcggcttcaacttcagccaaatcctgcccgaccctagcaagcctagcaagcggagcttcatcgaggacctgctgttcaacaaggtgaccctggccgacgccggcttcatcaagcagtacggcgactgcctaggcgacatcgcagctagagacctgatctgcgctcagaagttcaatggactcaccgtgctcccccccctgctgaccgacgagatgatcgctcagtacacctctgccctgctggcgggaaccataacaagcggttggacatttggcgccggggccgcactgcaaatccccttcgccatgcagatggcctacagattcaacggcatcggcgtgacacagaacgtgctgtacgagaatcagaagctgatcgccaatcagttcaacagcgccatcggcaagatccaagacagcctgagcagcaccgctagcgccctgggcaagctgcaagacgtggtgaatcagaacgcccaagccctgaacaccctggtgaagcagctgagcagcaacttcggcgccatcagcagcgtattgaatgacatcctgtctagactggacccccccgaggccgaggtgcagatcgacagactgatcaccggcagactgcagagcctgcagacctacgtgacacagcagctgatcagagccgccgagatcagagctagcgccaacctggccgccaccaagatgagcgagtgcgtgctggggcagagcaagagagtggacttctgcggcaagggctaccacctgatgagcttccctcagagcgccccccacggcgtggtgttcctgcacgtgacctacgtgcccgcccaagagaagaacttcaccaccgctcccgccatctgccacgacggcaaggcccacttccctagagagggcgtgttcgtgagcaacggcacccactggttcgtgacacagagaaacttctacgagcctcagatcatcaccaccgacaacaccttcgtgagcggcaactgcgacgtggtgatcggcatagtgaacaacaccgtatacgaccccctgcagcccgagctggacagcttcaaggaggagctggacaagtacttcaaaaaccatactagccccgacgtggacctgggagacatctctggcatcaacgctagcgtggtgaacattcagaaggagatcgaccggctgaatgaggtggccaagaacctgaacgagagcctgatcgacctgcaagagctgggcaagtacgagcagtacatcaagtggccctggtacatctggctgggcttcatcgccggcctgatcgccatcgtgatggtgaccatcatgctgtgctgcatgacaagctgttgcagctgcctgaaaggttgctgcagctgtggctcgtgctgcaagttcgacgaggacgacagcgagcccgtgctgaagggcgtgaagctgcactacacctgatga

SEQ ID NO: 60 - RNA, 3816 nt, synthetic construct
  source 1..3816: mol_type = other RNA; note = B.1.1.7 Spike mRNA
atgttcgtgttcctggtgctgctgcccctggtgagctctcagtgcgtgaacctgaccacaagaacacagctgccccccgcctacaccaacagcttcacaagaggcgtgtactaccccgacaaggtgttcagaagcagcgtgctgcactccacccaagacctgtttctgcccttcttcagcaacgtgacctggttccacgccatcagcggcaccaacggcaccaagagattcgacaaccccgtgctgcccttcaacgacggcgtgtacttcgctagcaccgaaaagagcaacatcatcagaggctggatcttcggcaccaccctagactccaagacacaaagcctgctgatcgttaacaacgcgaccaacgtggtgatcaaggtgtgcgagtttcagttctgcaacgaccccttcctgggcgtgtaccacaagaacaacaagagctggatggagagcgagttccgtgtctacagcagcgccaacaactgcaccttcgagtacgtgtctcagcccttcctgatggacctggagggcaagcaaggcaatttcaagaacctaagagagttcgtgttcaagaacatcgacggctacttcaagatctacagcaagcacacccccatcaacctggtgagagacctgccccaaggcttcagcgccctggagcccctggtggacctgcccatcggcatcaacatcacaagatttcagaccctgctggccctgcaccgtagctacctaacccccggcgatagttcctctggctggacggccggcgctgccgcctactacgtgggctacctgcagcctagaaccttcctgctgaagtacaacgagaacggcactatcactgatgccgtggactgtgccctggaccccctgagcgagaccaagtgcaccctcaagagcttcaccgtggagaagggcatctatcagacaagcaacttcagagtgcagcccaccgagagcatcgtgagattccccaacatcaccaacctgtgccccttcggcgaggtgttcaacgccacaagattcgctagcgtgtacgcgtggaacagaaagagaatcagcaactgcgtggccgactacagcgtgctgtacaacagcgctagcttcagcaccttcaagtgctatggcgtcagccccaccaagctgaacgacctgtgcttcaccaacgtgtacgccgacagcttcgtgatcagaggcgacgaggtgagacagattgcccccgggcaaaccggcaagatcgccgactacaactacaagctgcccgacgacttcaccggctgcgtgatcgcgtggaacagcaataacctggattccaaggtgggcggcaactacaactacctgtacagactgttcagaaagagcaacctgaagcccttcgagagagacatcagcaccgagatctaccaagccggcagcaccccctgcaacggcgtggagggcttcaactgctacttccccctgcagagctacggctttcagcccacctacggcgtgggctatcagccctacagagtggtggtgctgagcttcgagctgctgcacgcccccgcaaccgtgtgcggccccaaaaagagcaccaacctggtgaagaacaagtgcgtgaacttcaactttaatggccttaccggcacgggcgtgctgaccgagagcaacaagaagttcctgccatttcagcaattcggcagagacatcgacgacaccaccgacgcggtcagagaccctcagaccctggagatcctggacatcaccccctgtagcttcggcggcgtgagcgtgatcacccccggcactaacacaagcaaccaagtggccgtgctgtaccaaggcgtgaactgcaccgaggtgcccgtggccatccacgccgatcagctgacccccacctggagagtatacagcaccggaagcaacgtgtttcagacaagagccggctgcctgatcggcgccgagcacgtgaacaacagctacgagtgcgacatccccatcggcgccggcatctgcgctagctatcagacacagaccaacagccaccggagagctagaagcgtggcttctcagagcatcatcgcctacaccatgagcctgggcgccgagaacagcgtggcctacagcaacaacagcatcgccatccccatcaacttcaccatcagcgtgaccaccgagatcctgcccgtaagtatgaccaagacaagcgtggactgcaccatgtacatctgcggcgacagcaccgagtgcagcaacctgctgctgcagtacggcagcttctgcacacagctgaacagagccctgaccggcatcgccgtggagcaagacaagaacacccaagaggtgttcgcccaagtgaagcagatctacaagaccccccccatcaaggacttcggcggcttcaacttcagccaaatcctgcccgaccctagcaagcctagcaagcggagcttcatcgaggacctgctgttcaacaaggtgaccctggccgacgccggcttcatcaagcagtacggcgactgcctaggcgacatcgcagctagagacctgatctgcgctcagaagttcaatggactcaccgtgctcccccccctgctgaccgacgagatgatcgctcagtacacctctgccctgctggcgggaaccataacaagcggttggacatttggcgccggggccgcactgcaaatccccttcgccatgcagatggcctacagattcaacggcatcggcgtgacacagaacgtgctgtacgagaatcagaagctgatcgccaatcagttcaacagcgccatcggcaagatccaagacagcctgagcagcaccgctagcgccctgggcaagctgcaagacgtggtgaatcagaacgcccaagccctgaacaccctggtgaagcagctgagcagcaacttcggcgccatcagcagcgtattgaatgacatcctggctagactggacccccccgaggccgaggtgcagatcgacagactgatcaccggcagactgcagagcctgcagacctacgtgacacagcagctgatcagagccgccgagatcagagctagcgccaacctggccgccaccaagatgagcgagtgcgtgctggggcagagcaagagagtggacttctgcggcaagggctaccacctgatgagcttccctcagagcgccccccacggcgtggtgttcctgcacgtgacctacgtgcccgcccaagagaagaacttcaccaccgctcccgccatctgccacgacggcaaggcccacttccctagagagggcgtgttcgtgagcaacggcacccactggttcgtgacacagagaaacttctacgagcctcagatcatcaccacccacaacaccttcgtgagcggcaactgcgacgtggtgatcggcatagtgaacaacaccgtatacgaccccctgcagcccgagctggacagcttcaaggaggagctggacaagtacttcaaaaaccatactagccccgacgtggacctgggagacatctctggcatcaacgctagcgtggtgaacattcagaaggagatcgaccggctgaatgaggtggccaagaacctgaacgagagcctgatcgacctgcaagagctgggcaagtacgagcagtacatcaagtggccctggtacatctggctgggcttcatcgccggcctgatcgccatcgtgatggtgaccatcatgctgtgctgcatgacaagctgttgcagctgcctgaaaggttgctgcagctgtggctcgtgctgcaagttcgacgaggacgacagcgagcccgtgctgaagggcgtgaagctgcactacacctgatga

SEQ ID NO: 61 - RNA, 3825 nt, synthetic construct
  source 1..3825: mol_type = other RNA; note = SARS-COV-2 Spike mRNA
atgttcgtgttcctggtgctgctgcccctggtgagctctcagtgcgtgaacctgaccacaagaacacagctgccccccgcctacaccaacagcttcacaagaggcgtgtactaccccgacaaggtgttcagaagcagcgtgctgcactccacccaagacctgtttctgcccttcttcagcaacgtgacctggttccacgccatccacgtgagcggcaccaacggcaccaagagattcgacaaccccgtgctgcccttcaacgacggcgtgtacttcgctagcaccgaaaagagcaacatcatcagaggctggatcttcggcaccaccctagactccaagacacaaagcctgctgatcgttaacaacgcgaccaacgtggtgatcaaggtgtgcgagtttcagttctgcaacgaccccttcctgggcgtgtactaccacaagaacaacaagagctggatggagagcgagttccgtgtctacagcagcgccaacaactgcaccttcgagtacgtgtctcagcccttcctgatggacctggagggcaagcaaggcaatttcaagaacctaagagagttcgtgttcaagaacatcgacggctacttcaagatctacagcaagcacacccccatcaacctggtgagagacctgccccaaggcttcagcgccctggagcccctggtggacctgcccatcggcatcaacatcacaagatttcagaccctgctggccctgcaccgtagctacctaacccccggcgatagttcctctggctggacggccggcgctgccgcctactacgtgggctacctgcagcctagaaccttcctgctgaagtacaacgagaacggcactatcactgatgccgtggactgtgccctggaccccctgagcgagaccaagtgcaccctcaagagcttcaccgtggagaagggcatctatcagacaagcaacttcagagtgcagcccaccgagagcatcgtgagattccccaacatcaccaacctgtgccccttcggcgaggtgttcaacgccacaagattcgctagcgtgtacgcgtggaacagaaagagaatcagcaactgcgtggccgactacagcgtgctgtacaacagcgctagcttcagcaccttcaagtgctatggcgtcagccccaccaagctgaacgacctgtgcttcaccaacgtgtacgccgacagcttcgtgatcagaggcgacgaggtgagacagattgcccccgggcaaaccggcaagatcgccgactacaactacaagctgcccgacgacttcaccggctgcgtgatcgcgtggaacagcaataacctggattccaaggtgggcggcaactacaactacctgtacagactgttcagaaagagcaacctgaagcccttcgagagagacatcagcaccgagatctaccaagccggcagcaccccctgcaacggcgtggagggcttcaactgctacttccccctgcagagctacggctttcagcccaccaatggcgtgggctatcagccctacagagtggtggtgctgagcttcgagctgctgcacgcccccgcaaccgtgtgcggccccaaaaagagcaccaacctggtgaagaacaagtgcgtgaacttcaactttaatggccttaccggcacgggcgtgctgaccgagagcaacaagaagttcctgccatttcagcaattcggcagagacatcgccgacaccaccgacgcggtcagagaccctcagaccctggagatcctggacatcaccccctgtagcttcggcggcgtgagcgtgatcacccccggcactaacacaagcaaccaagtggccgtgctgtaccaagacgtgaactgcaccgaggtgcccgtggccatccacgccgatcagctgacccccacctggagagtatacagcaccggaagcaacgtgtttcagacaagagccggctgcctgatcggcgccgagcacgtgaacaacagctacgagtgcgacatccccatcggcgccggcatctgcgctagctatcagacacagaccaacagccctcggagagctagaagcgtggcttctcagagcatcatcgcctacaccatgagcctgggcgccgagaacagcgtggcctacagcaacaacagcatcgccatccccaccaacttcaccatcagcgtgaccaccgagatcctgcccgtaagtatgaccaagacaagcgtggactgcaccatgtacatctgcggcgacagcaccgagtgcagcaacctgctgctgcagtacggcagcttctgcacacagctgaacagagccctgaccggcatcgccgtggagcaagacaagaacacccaagaggtgttcgcccaagtgaagcagatctacaagaccccccccatcaaggacttcggcggcttcaacttcagccaaatcctgcccgaccctagcaagcctagcaagcggagcttcatcgaggacctgctgttcaacaaggtgaccctggccgacgccggcttcatcaagcagtacggcgactgcctaggcgacatcgcagctagagacctgatctgcgctcagaagttcaatggactcaccgtgctcccccccctgctgaccgacgagatgatcgctcagtacacctctgccctgctggcgggaaccataacaagcggttggacatttggcgccggggccgcactgcaaatccccttcgccatgcagatggcctacagattcaacggcatcggcgtgacacagaacgtgctgtacgagaatcagaagctgatcgccaatcagttcaacagcgccatcggcaagatccaagacagcctgagcagcaccgctagcgccctgggcaagctgcaagacgtggtgaatcagaacgcccaagccctgaacaccctggtgaagcagctgagcagcaacttcggcgccatcagcagcgtattgaatgacatcctgagcagactggacccccccgaggccgaggtgcagatcgacagactgatcaccggcagactgcagagcctgcagacctacgtgacacagcagctgatcagagccgccgagatcagagctagcgccaacctggccgccaccaagatgagcgagtgcgtgctggggcagagcaagagagtggacttctgcggcaagggctaccacctgatgagcttccctcagagcgccccccacggcgtggtgttcctgcacgtgacctacgtgcccgcccaagagaagaacttcaccaccgctcccgccatctgccacgacggcaaggcccacttccctagagagggcgtgttcgtgagcaacggcacccactggttcgtgacacagagaaacttctacgagcctcagatcatcaccaccgacaacaccttcgtgagcggcaactgcgacgtggtgatcggcatagtgaacaacaccgtatacgaccccctgcagcccgagctggacagcttcaaggaggagctggacaagtacttcaaaaaccatactagccccgacgtggacctgggagacatctctggcatcaacgctagcgtggtgaacattcagaaggagatcgaccggctgaatgaggtggccaagaacctgaacgagagcctgatcgacctgcaagagctgggcaagtacgagcagtacatcaagtggccctggtacatctggctgggcttcatcgccggcctgatcgccatcgtgatggtgaccatcatgctgtgctgcatgacaagctgttgcagctgcctgaaaggttgctgcagctgtggctcgtgctgcaagttcgacgaggacgacagcgagcccgtgctgaagggcgtgaagctgcactacacctgatga

SEQ ID NO: 62 - RNA, 1653 nt, synthetic construct
  source 1..1653: mol_type = other RNA; note = Luciferase mRNA
atggaggacgccaagaacatcaagaaaggccccgcccccttctaccccctggaggacggcaccgccggcgagcagctgcacaaagccatgaaaagatacgctctggtgcccggcaccatcgccttcaccgacgcccacatcgaggtgaacatcacctacgccgagtacttcgagatgagcgtgagactggccgaggctatgaagagatacggcttgaacaccaaccacagaatcgtggtgtgcagcgagaacagcctgcagttcttcatgcccgtgctgggcgccctgttcatcggcgtggccgttgcccccgccaacgacatctacaacgagagagagctgctgaacagcatgaacatctctcagcccaccgtggttttcgtgtccaaaaagggcctgcagaagatcctgaacgtgcagaagaagctgcccatcattcagaagatcatcatcatggacagcaagaccgactaccaaggctttcagagcatgtacaccttcgtgacaagccacctgccccccggcttcaacgagtacgacttcgtgcccgagagcttcgacagagacaagaccatcgccctgatcatgaacagcagcggcagcaccggcctgcccaagggcgtggccctgccccacagaaccgcctgcgtgagattcagccacgctagagaccccatcttcggcaatcagatcatccccgacaccgccatcctgagcgtagtgcctttccatcatggcttcggcatgttcaccaccctgggctacctgatctgcggcttcagagtggtgctgatgtacagattcgaggaggagctgttcctgagaagcctgcaagactacaagattcagagcgccctgctggtgcccaccctgttcagcttcttcgccaagagcaccctgatcgacaagtatgacctgagcaacctgcacgaaattgcgagcggcggagcgccgctcagcaaagaggtgggcgaggccgtggccaagagattccacctgcccggcatcagacaaggctacggcctgaccgagaccacaagcgccatcctgatcacccccgagggcgacgataagcccggcgccgtgggcaaggtggtaccattcttcgaggccaaggtggtggacctggacaccggcaagaccctgggcgtgaatcagagaggcgagctgtgcgtgagaggccccatgatcatgagcggctacgtgaacaaccccgaggccaccaacgccctcatcgataaggatgggtggctgcacagcggcgacatcgcctactgggacgaggacgagcacttcttcatcgtggacagactcaagagcctgatcaagtacaagggctaccaagtggcccccgccgagttggagagcatcctgctgcagcaccccaatatcttcgacgctggcgtggccggactacccgacgacgacgccggcgagttacccgccgccgtggtggtgctggagcacggcaagaccatgaccgagaaggagatcgtggactacgtggctagccaagtgaccaccgccaagaagctgagaggcggcgtggtgttcgttgacgaagtgcccaagggcctgaccggcaagctggacgctagaaagatcagagagatcctgatcaaggccaagaagggcggcaagagcaagctgtga

SEQ ID NO: 63 - RNA, 59 nt, synthetic construct
  source 1..59: mol_type = other RNA; note; note (original language) = LUC1- I' truncation
taggagttggtggcagtttcaataacaggtcattgccgagaaaaggatagcactataat

SEQ ID NO: 64 - RNA, 55 nt, synthetic construct
  source 1..55: mol_type = other RNA; note; note (original language) = LUC2- I' truncation
agttggtggcagtttcaataacaggtcattgccgagaaaaggatagcactataat

SEQ ID NO: 65 - RNA, 51 nt, synthetic construct
  source 1..51: mol_type = other RNA; note; note (original language) = LUC3- I' truncation
ggtggcagtttcaataacaggtcattgccgagaaaaggatagcactataat

SEQ ID NO: 66 - RNA, 47 nt, synthetic construct
  source 1..47: mol_type = other RNA; note; note (original language) = LUC4- I' truncation
gcagtttcaataacaggtcattgccgagaaaaggatagcactataat

SEQ ID NO: 67 - RNA, 43 nt, synthetic construct
  source 1..43: mol_type = other RNA; note; note (original language) = LUC5- I' truncation
tttcaataacaggtcattgccgagaaaaggatagcactataat

SEQ ID NO: 68 - RNA, 39 nt, synthetic construct
  source 1..39: mol_type = other RNA; note; note (original language) = LUC6- I' truncation
aataacaggtcattgccgagaaaaggatagcactataat

SEQ ID NO: 69 - RNA, 35 nt, synthetic construct
  source 1..35: mol_type = other RNA; note; note (original language) = LUC7- I' truncation
acaggtcattgccgagaaaaggatagcactataat

SEQ ID NO: 70 - RNA, 31 nt, synthetic construct
  source 1..31: mol_type = other RNA; note; note (original language) = LUC8- I' truncation
gtcattgccgagaaaaggatagcactataat

SEQ ID NO: 71 - RNA, 27 nt, synthetic construct
  source 1..27: mol_type = other RNA; note; note (original language) = LUC9- I' truncation
ttgccgagaaaaggatagcactataat

SEQ ID NO: 72 - RNA, 23 nt, synthetic construct
  source 1..23: mol_type = other RNA; note; note (original language) = LUC10- I' truncation
cgagaaaaggatagcactataat

SEQ ID NO: 73 - RNA, 19 nt, synthetic construct
  source 1..19: mol_type = other RNA; note; note (original language) = LUC11- I' truncation
aaaaggatagcactataat

SEQ ID NO: 74 - RNA, 15 nt, synthetic construct
  source 1..15: mol_type = other RNA; note; note (original language) = LUC12- I' truncation
ggatagcactataat

SEQ ID NO: 75 - RNA, 11 nt, synthetic construct
  source 1..11: mol_type = other RNA; note; note (original language) = LUC13- I' truncation
agcactataat

SEQ ID NO: 76 - DNA, 18 bp, synthetic construct
  source 1..18: mol_type = other DNA; note; note (original language) = 5'UTR truncation
tcaataacaggtcattgc

SEQ ID NO: 77 - RNA, 63 nt, synthetic construct
  source 1..63: mol_type = other RNA; note; note (original language) = LUC15- I' mutant
gagttaggagttgctggcagtttcaataacaggtcattgccgagaaaaggatagcactataat

SEQ ID NO: 78 - RNA, 63 nt, synthetic construct
  source 1..63: mol_type = other RNA; note; note (original language) = LUC16- I' mutant
gagttaggagttgttggcagtttcaataacaggtcattgccgagaaaaggatagcactataat

SEQ ID NO: 79 - RNA, 63 nt, synthetic construct
  source 1..63: mol_type = other RNA; note; note (original language) = 5'UTR I general formula
  misc_difference 14: note; note (original language) = N is selected from the group consisting of A, G, C, and U
gagttaggagttgntggcagtttcaataacaggtcattgccgagaaaaggatagcactataat

SEQ ID NO: 80 - protein, 1273 aa, Severe acute respiratory syndrome coronavirus2
  source 1..1273: note = Wild SARS-COV-2 Spike
MFVFLVLLPLVSSQCVNLTTRTQLPPAYTNSFTRGVYYPDKVFRSSVLHSTQDLFLPFFSNVTWFHAIHVSGTNGTKRFDNPVLPFNDGVYFASTEKSNIIRGWIFGTTLDSKTQSLLIVNNATNVVIKVCEFQFCNDPFLGVYYHKNNKSWMESEFRVYSSANNCTFEYVSQPFLMDLEGKQGNFKNLREFVFKNIDGYFKIYSKHTPINLVRDLPQGFSALEPLVDLPIGINITRFQTLLALHRSYLTPGDSSSGWTAGAAAYYVGYLQPRTFLLKYNENGTITDAVDCALDPLSETKCTLKSFTVEKGIYQTSNFRVQPTESIVRFPNITNLCPFGEVFNATRFASVYAWNRKRISNCVADYSVLYNSASFSTFKCYGVSPTKLNDLCFTNVYADSFVIRGDEVRQIAPGQTGKIADYNYKLPDDFTGCVIAWNSNNLDSKVGGNYNYLYRLFRKSNLKPFERDISTEIYQAGSTPCNGVEGFNCYFPLQSYGFQPTNGVGYQPYRVVVLSFELLHAPATVCGPKKSTNLVKNKCVNFNFNGLTGTGVLTESNKKFLPFQQFGRDIADTTDAVRDPQTLEILDITPCSFGGVSVITPGTNTSNQVAVLYQDVNCTEVPVAIHADQLTPTWRVYSTGSNVFQTRAGCLIGAEHVNNSYECDIPIGAGICASYQTQTNSPRRARSVASQSIIAYTMSLGAENSVAYSNNSIAIPTNFTISVTTEILPVSMTKTSVDCTMYICGDSTECSNLLLQYGSFCTQLNRALTGIAVEQDKNTQEVFAQVKQIYKTPPIKDFGGFNFSQILPDPSKPSKRSFIEDLLFNKVTLADAGFIKQYGDCLGDIAARDLICAQKFNGLTVLPPLLTDEMIAQYTSALLAGTITSGWTFGAGAALQIPFAMQMAYRFNGIGVTQNVLYENQKLIANQFNSAIGKIQDSLSSTASALGKLQDVVNQNAQALNTLVKQLSSNFGAISSVLNDILSRLDKVEAEVQIDRLITGRLQSLQTYVTQQLIRAAEIRASANLAATKMSECVLGQSKRVDFCGKGYHLMSFPQSAPHGVVFLHVTYVPAQEKNFTTAPAICHDGKAHFPREGVFVSNGTHWFVTQRNFYEPQIITTDNTFVSGNCDVVIGIVNNTVYDPLQPELDSFKEELDKYFKNHTSPDVDLGDISGINASVVNIQKEIDRLNEVAKNLNESLIDLQELGKYEQYIKWPWYIWLGFIAGLIAIVMVTIMLCCMTSCCSCLKGCCSCGSCCKFDEDDSEPVLKGVKLHYT

SEQ ID NO: 81 - DNA, 3822 bp, synthetic construct
  source 1..3822: mol_type = other DNA; note = Wild SARS-COV-2 Spike CDS
atgtttgtttttcttgttttattgccactagtctctagtcagtgtgttaatcttacaaccagaactcaattaccccctgcatacactaattctttcacacgtggtgtttattaccctgacaaagttttcagatcctcagttttacattcaactcaggacttgttcttacctttcttttccaatgttacttggttccatgctatacatgtctctgggaccaatggtactaagaggtttgataaccctgtcctaccatttaatgatggtgtttattttgcttccactgagaagtctaacataataagaggctggatttttggtactactttagattcgaagacccagtccctacttattgttaataacgctactaatgttgttattaaagtctgtgaatttcaattttgtaatgatccatttttgggtgtttattaccacaaaaacaacaaaagttggatggaaagtgagttcagagtttattctagtgcgaataattgcacttttgaatatgtctctcagccttttcttatggaccttgaaggaaaacagggtaatttcaaaaatcttagggaatttgtgtttaagaatattgatggttattttaaaatatattctaagcacacgcctattaatttagtgcgtgatctccctcagggtttttcggctttagaaccattggtagatttgccaataggtattaacatcactaggtttcaaactttacttgctttacatagaagttatttgactcctggtgattcttcttcaggttggacagctggtgctgcagcttattatgtgggttatcttcaacctaggacttttctattaaaatataatgaaaatggaaccattacagatgctgtagactgtgcacttgaccctctctcagaaacaaagtgtacgttgaaatccttcactgtagaaaaaggaatctatcaaacttctaactttagagtccaaccaacagaatctattgttagatttcctaatattacaaacttgtgcccttttggtgaagtttttaacgccaccagatttgcatctgtttatgcttggaacaggaagagaatcagcaactgtgttgctgattattctgtcctatataattccgcatcattttccacttttaagtgttatggagtgtctcctactaaattaaatgatctctgctttactaatgtctatgcagattcatttgtaattagaggtgatgaagtcagacaaatcgctccagggcaaactggaaagattgctgattataattataaattaccagatgattttacaggctgcgttatagcttggaattctaacaatcttgattctaaggttggtggtaattataattacctgtatagattgtttaggaagtctaatctcaaaccttttgagagagatatttcaactgaaatctatcaggccggtagcacaccttgtaatggtgttgaaggttttaattgttactttcctttacaatcatatggtttccaacccactaatggtgttggttaccaaccatacagagtagtagtactttcttttgaacttctacatgcaccagcaactgtttgtggacctaaaaagtctactaatttggttaaaaacaaatgtgtcaatttcaacttcaatggtttaacaggcacaggtgttcttactgagtctaacaaaaagtttctgcctttccaacaatttggcagagacattgctgacactactgatgctgtccgtgatccacagacacttgagattcttgacattacaccatgttcttttggtggtgtcagtgttataacaccaggaacaaatacttctaaccaggttgctgttctttatcaggatgttaactgcacagaagtccctgttgctattcatgcagatcaacttactcctacttggcgtgtttattctacaggttctaatgtttttcaaacacgtgcaggctgtttaataggggctgaacatgtcaacaactcatatgagtgtgacatacccattggtgcaggtatatgcgctagttatcagactcagactaattctcctcggcgggcacgtagtgtagctagtcaatccatcattgcctacactatgtcacttggtgcagaaaattcagttgcttactctaataactctattgccatacccacaaattttactattagtgttaccacagaaattctaccagtgtctatgaccaagacatcagtagattgtacaatgtacatttgtggtgattcaactgaatgcagcaatcttttgttgcaatatggcagtttttgtacacaattaaaccgtgctttaactggaatagctgttgaacaagacaaaaacacccaagaagtttttgcacaagtcaaacaaatttacaaaacaccaccaattaaagattttggtggttttaatttttcacaaatattaccagatccatcaaaaccaagcaagaggtcatttattgaagatctacttttcaacaaagtgacacttgcagatgctggcttcatcaaacaatatggtgattgccttggtgatattgctgctagagacctcatttgtgcacaaaagtttaacggccttactgttttgccacctttgctcacagatgaaatgattgctcaatacacttctgcactgttagcgggtacaatcacttctggttggacctttggtgcaggtgctgcattacaaataccatttgctatgcaaatggcttataggtttaatggtattggagttacacagaatgttctctatgagaaccaaaaattgattgccaaccaatttaatagtgctattggcaaaattcaagactcactttcttccacagcaagtgcacttggaaaacttcaagatgtggtcaaccaaaatgcacaagctttaaacacgcttgttaaacaacttagctccaattttggtgcaatttcaagtgttttaaatgatatcctttcacgtcttgacaaagttgaggctgaagtgcaaattgataggttgatcacaggcagacttcaaagtttgcagacatatgtgactcaacaattaattagagctgcagaaatcagagcttctgctaatcttgctgctactaaaatgtcagagtgtgtacttggacaatcaaaaagagttgatttttgtggaaagggctatcatcttatgtccttccctcagtcagcacctcatggtgtagtcttcttgcatgtgacttatgtccctgcacaagaaaagaacttcacaactgctcctgccatttgtcatgatggaaaagcacactttcctcgtgaaggtgtctttgtttcaaatggcacacactggtttgtaacacaaaggaatttttatgaaccacaaatcattactacagacaacacatttgtgtctggtaactgtgatgttgtaataggaattgtcaacaacacagtttatgatcctttgcaacctgaattagactcattcaaggaggagttagataaatattttaagaatcatacatcaccagatgttgatttaggtgacatctctggcattaatgcttcagttgtaaacattcaaaaagaaattgaccgcctcaatgaggttgccaagaatttaaatgaatctctcatcgatctccaagaacttggaaagtatgagcagtatataaaatggccatggtacatttggctaggttttatagctggcttgattgccatagtaatggtgacaattatgctttgctgtatgaccagttgctgtagttgtctcaagggctgttgttcttgtggatcctgctgcaaatttgatgaagacgactctgagccagtgctcaaaggagtcaaattacattacacataa

SEQ ID NO: 82 - RNA, 3822 nt, synthetic construct
  source 1..3822: mol_type = other RNA; note = Wild SARS-COV-2 Spike mRNA
atgtttgtttttcttgttttattgccactagtctctagtcagtgtgttaatcttacaaccagaactcaattaccccctgcatacactaattctttcacacgtggtgtttattaccctgacaaagttttcagatcctcagttttacattcaactcaggacttgttcttacctttcttttccaatgttacttggttccatgctatacatgtctctgggaccaatggtactaagaggtttgataaccctgtcctaccatttaatgatggtgtttattttgcttccactgagaagtctaacataataagaggctggatttttggtactactttagattcgaagacccagtccctacttattgttaataacgctactaatgttgttattaaagtctgtgaatttcaattttgtaatgatccatttttgggtgtttattaccacaaaaacaacaaaagttggatggaaagtgagttcagagtttattctagtgcgaataattgcacttttgaatatgtctctcagccttttcttatggaccttgaaggaaaacagggtaatttcaaaaatcttagggaatttgtgtttaagaatattgatggttattttaaaatatattctaagcacacgcctattaatttagtgcgtgatctccctcagggtttttcggctttagaaccattggtagatttgccaataggtattaacatcactaggtttcaaactttacttgctttacatagaagttatttgactcctggtgattcttcttcaggttggacagctggtgctgcagcttattatgtgggttatcttcaacctaggacttttctattaaaatataatgaaaatggaaccattacagatgctgtagactgtgcacttgaccctctctcagaaacaaagtgtacgttgaaatccttcactgtagaaaaaggaatctatcaaacttctaactttagagtccaaccaacagaatctattgttagatttcctaatattacaaacttgtgcccttttggtgaagtttttaacgccaccagatttgcatctgtttatgcttggaacaggaagagaatcagcaactgtgttgctgattattctgtcctatataattccgcatcattttccacttttaagtgttatggagtgtctcctactaaattaaatgatctctgctttactaatgtctatgcagattcatttgtaattagaggtgatgaagtcagacaaatcgctccagggcaaactggaaagattgctgattataattataaattaccagatgattttacaggctgcgttatagcttggaattctaacaatcttgattctaaggttggtggtaattataattacctgtatagattgtttaggaagtctaatctcaaaccttttgagagagatatttcaactgaaatctatcaggccggtagcacaccttgtaatggtgttgaaggttttaattgttactttcctttacaatcatatggtttccaacccactaatggtgttggttaccaaccatacagagtagtagtactttcttttgaacttctacatgcaccagcaactgtttgtggacctaaaaagtctactaatttggttaaaaacaaatgtgtcaatttcaacttcaatggtttaacaggcacaggtgttcttactgagtctaacaaaaagtttctgcctttccaacaatttggcagagacattgctgacactactgatgctgtccgtgatccacagacacttgagattcttgacattacaccatgttcttttggtggtgtcagtgttataacaccaggaacaaatacttctaaccaggttgctgttctttatcaggatgttaactgcacagaagtccctgttgctattcatgcagatcaacttactcctacttggcgtgtttattctacaggttctaatgtttttcaaacacgtgcaggctgtttaataggggctgaacatgtcaacaactcatatgagtgtgacatacccattggtgcaggtatatgcgctagttatcagactcagactaattctcctcggcgggcacgtagtgtagctagtcaatccatcattgcctacactatgtcacttggtgcagaaaattcagttgcttactctaataactctattgccatacccacaaattttactattagtgttaccacagaaattctaccagtgtctatgaccaagacatcagtagattgtacaatgtacatttgtggtgattcaactgaatgcagcaatcttttgttgcaatatggcagtttttgtacacaattaaaccgtgctttaactggaatagctgttgaacaagacaaaaacacccaagaagtttttgcacaagtcaaacaaatttacaaaacaccaccaattaaagattttggtggttttaatttttcacaaatattaccagatccatcaaaaccaagcaagaggtcatttattgaagatctacttttcaacaaagtgacacttgcagatgctggcttcatcaaacaatatggtgattgccttggtgatattgctgctagagacctcatttgtgcacaaaagtttaacggccttactgttttgccacctttgctcacagatgaaatgattgctcaatacacttctgcactgttagcgggtacaatcacttctggttggacctttggtgcaggtgctgcattacaaataccatttgctatgcaaatggcttataggtttaatggtattggagttacacagaatgttctctatgagaaccaaaaattgattgccaaccaatttaatagtgctattggcaaaattcaagactcactttcttccacagcaagtgcacttggaaaacttcaagatgtggtcaaccaaaatgcacaagctttaaacacgcttgttaaacaacttagctccaattttggtgcaatttcaagtgttttaaatgatatcctttcacgtcttgacaaagttgaggctgaagtgcaaattgataggttgatcacaggcagacttcaaagtttgcagacatatgtgactcaacaattaattagagctgcagaaatcagagcttctgctaatcttgctgctactaaaatgtcagagtgtgtacttggacaatcaaaaagagttgatttttgtggaaagggctatcatcttatgtccttccctcagtcagcacctcatggtgtagtcttcttgcatgtgacttatgtccctgcacaagaaaagaacttcacaactgctcctgccatttgtcatgatggaaaagcacactttcctcgtgaaggtgtctttgtttcaaatggcacacactggtttgtaacacaaaggaatttttatgaaccacaaatcattactacagacaacacatttgtgtctggtaactgtgatgttgtaataggaattgtcaacaacacagtttatgatcctttgcaacctgaattagactcattcaaggaggagttagataaatattttaagaatcatacatcaccagatgttgatttaggtgacatctctggcattaatgcttcagttgtaaacattcaaaaagaaattgaccgcctcaatgaggttgccaagaatttaaatgaatctctcatcgatctccaagaacttggaaagtatgagcagtatataaaatggccatggtacatttggctaggttttatagctggcttgattgccatagtaatggtgacaattatgctttgctgtatgaccagttgctgtagttgtctcaagggctgttgttcttgtggatcctgctgcaaatttgatgaagacgactctgagccagtgctcaaaggagtcaaattacattacacataa

SEQ ID NO: 83 - protein, 566 aa, Influenza A H1N1
MKAILVVMLYTFTTANADTLCIGYHANNSTDTVDTVLEKNVTVTHSVNLLEDKHNGKLCKLRGVAPLHLGKCNIAGWILGNPECESLSTARSWSYIVETSNSDNGTCYPGDFINYEELREQLSSVSSFERFEIFPKTSSWPNHDSDNGVTAACPHAGAKSFYKNLIWLVKKGKSYPKINQTYINDKGKEVLVLWGIHHPPTIADQQSLYQNADAYVFVGTSRYSKKFKPEIATRPKVRDQEGRMNYYWTLVEPGDKITFEATGNLVAPRYAFTMERDAGSGIIISDTPVHDCNTTCQTPEGAINTSLPFQNVHPITIGKCPKYVKSTKLRLATGLRNVPSIQSRGLFGAIAGFIEGGWTGMVDGWYGYHHQNEQGSGYAADLKSTQNAIDKITNKVNSVIEKMNTQFTAVGKEFNHLEKRIENLNKKVDDGFLDIWTYNAELLVLLENERTLDYHDSNVKNLYEKVRNQLKNNAKEIGNGCFEFYHKCDNTCMESVKNGTYDYPKYSEEAKLNREKIDGVKLDSTRIYQILAIYSTVASSLVLVVSLGAISFWMCSNGSLQCRICI

SEQ ID NO: 84 - protein, 566 aa, Influenza A H3N2 [sequence omitted]

SEQ ID NO: 85 - protein, 582 aa, Influenza B Victoria lineage
MKAIIVLLMVVTSNADRICTGITSSNSPHVVKTATQGEVNVTGVIPLTTTPTKSHFANLKGTETRGKLCPKCLNCTDLDVALGRPKCTGKIPSARVSILHEVRPVTSGCFPIMHDRTKIRQLPNLLRGYEHVRLSTHNVINAEDAPGRPYEIGTSGSCPNITNGNGFFATMAWAVPKNKTATNPLTIEVPYICTEGEDQITVWGFHSDNETQMAKLYGDSKPQKFTSSANGVTTHYVSQIGGFPNQTEDGGLPQSGRIVVDYMVQKSGKTGTITYQRGILLPQKVWCASGRSKVIKGSLPLIGEADCLHEKYGGLNKSKPYYTGEHAKAIGNCPIWVKTPLKLANGTKYRPPAKLLKERGFFGAIAGFLEGGWEGMIAGWHGYTSHGAHGVAVAADLKSTQEAINKITKNLNSLSELEVKNLQRLSGAMDELHNEILELDEKVDDLRADTISSQIELAVLLSNEGIINSEDEHLLALERKLKKMLGPSAVEIGNGCFETKHKCNQTCLDRIAAGTFDAGEFSLPTFDSLNITAASLNDDGLDNHTILLYYSTAASSLAVTLMIAIFVVYMVSRDNVSCSICL

SEQ ID NO: 86 - protein, 584 aa, Influenza B Yamagata lineage
MKAIIVLLMVVTSNADRICTGITSSNSPHVVKTATQGEVNVTGVIPLTTTPTKSYFANLKGTRTRGKLCPDCLNCTDLDVALGRPMCVGTTPSAKASILHEVRPVTSGCFPIMHDRTKIRQLPNLLRGYEKIRLSTQNVIDAEKAPGGPYRLGTSGSCPNATSKIGFFATMAWAVPKDNYKNATNPLTVEVPYICTEGEDQITVWGFHSDNKTQMKSLYGDSNPQKFTSSANGVTTHYVSQIGDFPDQTEDGGLPQSGRIVVDYMMQKPGKTGTIVYQRGVLLPQKVWCASGRSKVIKGSLPLIGEADCLHEEYGGLNKSKPYYTGKHAKAIGNCPIWVKTPLKLANGTKYRPPAKLLKERGFFGAIAGFLEGGWEGMIAGWHGYTSHGAHGVAVAADLKSTQEAINKITKNLNSLSELEVKNLQRLSGAMDELHNEILELDEKVDDLRADTISSQIELAVLLSNEGIINSEDEHLLALERKLKKMLGPSAVDIGNGCFETKHKCNQTCLDRIAAGTFNAGEFSLPTFDSLNITAASLNDDGLDNHTILLYYSTAASSLAVTLMLAIFIVYMVSRDNVSCSICL

SEQ ID NO: 87 - DNA, 1701 bp, synthetic construct
  source 1..1701: mol_type = other DNA; note = Influenza A H1N1
atgaaggccatcctggtggtgatgctgtacaccttcaccaccgccaacgccgacaccctgtgcatcggctaccacgccaacaacagcaccgacaccgtggacaccgtgctggagaagaacgtgaccgtgacccacagcgtgaacctgctggaggacaagcacaacggcaagctgtgcaagctgcggggcgtggcccccctgcacctgggcaagtgcaacatcgccggctggatcctgggcaaccccgagtgcgagtccctgagcaccgcccgctcctggagctacatcgtggagacctccaacagcgacaacggcacctgctaccccggggacttcatcaactacgaggagctgcgggagcagctgtccagcgtgtccagcttcgagcgcttcgagatcttccccaagacctccagctggcccaaccacgactccgacaacggcgtgaccgccgcctgcccccacgccggggccaagagcttctacaagaacctgatctggctggtgaagaagggcaagtcctaccccaagatcaaccagacctacatcaacgacaaggggaaggaggtcctcgtgctgtggggcatccaccacccccccaccatcgccgaccagcagagcctctaccagaacgccgacgcctacgtcttcgtggggacctcccggtacagcaagaagttcaagcccgagatcgccacccgccccaaggtccgggaccaggagggccgcatgaactactactggaccctggtggagccgggggacaagatcaccttcgaggccaccggcaacctcgtcgccccgcggtacgccttcacgatggagcgcgacgccgggtccggcatcatcatcagcgacacccccgtgcacgactgcaacacgacctgccagacgcccgagggggcgatcaacacctccctgccgttccagaacgtccacccgatcacgatcggcaagtgccccaagtacgtgaagtccaccaagctccggctggccacggggctccgcaacgtcccctccatccagagccggggcctgttcggggcgatcgccggcttcatcgaggggggctggaccgggatggtggacggctggtacgggtaccaccaccagaacgagcagggctccgggtacgcggccgacctcaagtcgacgcagaacgcgatcgacaagatcaccaacaaggtcaacagcgtgatcgagaagatgaacacgcagttcaccgccgtcggcaaggagttcaaccacctggagaagcgcatcgagaacctcaacaagaaggtggacgacgggttcctggacatctggacgtacaacgcggagctcctggtcctcctggagaacgagcggaccctcgactaccacgactccaacgtgaagaacctgtacgagaaggtccgcaaccagctcaagaacaacgccaaggagatcggcaacgggtgcttcgagttctaccacaagtgcgacaacacgtgcatggagtcggtgaagaacggcacctacgactacccgaagtacagcgaggaggcgaagctgaaccgggagaagatcgacggggtcaagctcgactccacgcgcatctaccagatcctggccatctactcgaccgtggcgagctccctcgtcctggtggtctcgctcggcgccatcagcttctggatgtgctccaacgggtcgctgcagtgccggatctgcatctga

SEQ ID NO: 88 - DNA, 1701 bp, synthetic construct
  source 1..1701: mol_type = other DNA; note = Influenza A H3N2
atgaagaccatcatcgccctgagctacatcctgtgcctggtgttcgcccagaagatccccggcaacgacaacagcaccgccaccctgtgcctgggccaccacgccgtgcccaacggcaccatcgtgaagaccatcaccaacgaccggatcgaggtgaccaacgccaccgagctggtgcagaactccagcatcggcgagatctgcgactccccccaccagatcctggacggcggcaactgcaccctgatcgacgccctgctgggcgacccccagtgcgacgggttccagaacaaggagtgggacctgttcgtggagcggagccgcgccaactccaactgctacccctacgacgtgcccgactacgccagcctgcggtccctggtggccagctccggcaccctggagttcaagaacgagagcttcaactggaccggggtcaagcagaacggcacctccagcgcctgcatccgcgggtccagctccagcttcttctcccggctgaactggctcacccacctgaactacacctaccccgccctcaacgtgaccatgcccaacaacgagcagttcgacaagctgtacatctggggcgtccaccaccccagcaccgacaaggaccagatctccctcttcgcccagcccagcgggcgcatcaccgtgtccacgaagcggagccagcaggccgtcatccccaacatcggctcccgcccgcggatccgcgacatccccagccggatctccatctactggacgatcgtgaagccgggggacatcctgctcatcaacagcaccggcaacctgatcgccccccgcgggtacttcaagatccggtccggcaagagctcgatcatgcgctccgacgccccgatcgggaagtgcaagagcgagtgcatcacccccaacggctcgatcccgaacgacaagcccttccagaacgtcaaccggatcacgtacggggcctgcccgcgctacgtgaagcagtccacgctcaagctggccaccggcatgcggaacgtccccgagaagcagacccgcgggatcttcggcgccatcgcggggttcatcgagaacggctgggaggggatggtggacggctggtacgggttccggcaccagaacagcgagggccgcgggcaggccgcggacctcaagtcgacgcaggccgcgatcgaccagatcaacggcaagctgaaccggctcatcgggaagacgaacgagaagttccaccagatcgagaaggagttctccgaggtcgagggccgcgtgcaggacctggagaagtacgtcgaggacaccaagatcgacctctggagctacaacgccgagctgctcgtggcgctggagaaccagcacaccatcgacctcacggactcggagatgaacaagctgttcgagaagacgaagaagcagctccgggagaacgccgaggacatggggaacggctgcttcaagatctaccacaagtgcgacaacgcgtgcatcgggtccatccgcaacgagacctacgaccacaacgtctaccgggacgaggccctgaacaaccgcttccagatcaagggcgtggagctcaagagcgggtacaaggactggatcctgtggatctcgttcgcgatgtcctgcttcctcctgtgcatcgccctcctgggcttcatcatgtgggcgtgccagaaggggaacatccggtgcaacatctgcatctga

SEQ ID NO: 89 - DNA, 1749 bp, synthetic construct
  source 1..1749: mol_type = other DNA; note = Influenza B Victoria lineage ( B/Washington/02/2019) HA CDS
atgaaggccatcatcgtgctgctgatggtggtgaccagcaacgccgaccggatctgcaccggcatcaccagctccaacagcccccacgtggtgaagaccgccacccagggcgaggtgaacgtgaccggcgtgatccccctgaccaccacccccaccaagtcccacttcgccaacctgaagggcaccgagacccggggcaagctgtgccccaagtgcctgaactgcaccgacctggacgtggccctgggccgccccaagtgcaccggcaagatccccagcgcccgggtgtccatcctgcacgaggtgcgccccgtgaccagcggctgcttccccatcatgcacgaccgcaccaagatccggcagctgcccaacctgctgcgggggtacgagcacgtccgcctgtccacccacaacgtgatcaacgccgaggacgcccccggccggccctacgagatcgggaccagcggctcctgccccaacatcaccaacgggaacggcttcttcgccaccatggcctgggccgtccccaagaacaagaccgccaccaaccccctgaccatcgaggtgccgtacatctgcaccgagggggaggaccagatcaccgtctggggcttccacagcgacaacgagacgcagatggccaagctgtacggggactccaagccccagaagttcacgagctccgccaacggcgtgaccacccactacgtcagccagatcgggggcttcccgaaccagacggaggacgggggcctgccccagtccgggcgcatcgtggtcgactacatggtgcagaagtccggcaagacggggaccatcacgtaccagcggggcatcctgctgccgcagaaggtctggtgcgcctccgggcgcagcaaggtgatcaagggctccctgcccctcatcggggaggccgactgcctgcacgagaagtacggcgggctcaacaagagcaagccgtactacaccggcgagcacgccaaggccatcgggaactgccccatctgggtcaagaccccgctgaagctcgccaacggcacgaagtaccggcccccggccaagctgctcaaggagcgcgggttcttcggcgccatcgccgggttcctggagggcgggtgggagggcatgatcgccgggtggcacggctacacgtcccacggggcccacggcgtggcggtcgccgcggacctcaagagcacccaggaggccatcaacaagatcacgaagaacctgaactccctcagcgagctggaggtgaagaacctccagcgcctgtccggggcgatggacgagctccacaacgagatcctggagctcgacgagaaggtcgacgacctgcgggccgacaccatcagctcgcagatcgagctcgcggtgctgctctccaacgagggcatcatcaacagcgaggacgagcacctgctcgccctggagcggaagctcaagaagatgctggggccctcggcggtcgagatcggcaacgggtgcttcgagaccaagcacaagtgcaaccagacgtgcctcgaccgcatcgccgcgggcacgttcgacgccggggagttctccctgccgaccttcgacagcctcaacatcacggcggcctcgctgaacgacgacggcctcgacaaccacaccatcctgctctactactccaccgcggccagctcgctggcggtgacgctcatgatcgccatcttcgtcgtgtacatggtctcccgcgacaacgtgagctgctcgatctgcctgtga

SEQ ID NO: 90 - RNA, 1755 nt, synthetic construct
  source 1..1755: mol_type = other RNA; note = Influenza B Yamagata lineage
atgaaggccatcatcgtgctgctgatggtggtgaccagcaacgccgaccggatctgcaccggcatcaccagctccaacagcccccacgtggtgaagaccgccacccagggcgaggtgaacgtgaccggcgtgatccccctgaccaccacccccaccaagtcctacttcgccaacctgaagggcacccggacccgcggcaagctgtgccccgactgcctgaactgcaccgacctggacgtggccctgggccggcccatgtgcgtgggcaccacccccagcgccaaggcctccatcctgcacgaggtgcgccccgtgaccagcggctgcttccccatcatgcacgaccgcaccaagatccggcagctgcccaacctgctgcgggggtacgagaagatccgcctgtccacccagaacgtcatcgacgccgagaaggcccccggcgggccctaccggctgggcaccagcgggtcctgccccaacgccaccagcaagatcggcttcttcgccaccatggcctgggccgtgcccaaggacaactacaagaacgccaccaaccccctgaccgtcgaggtgccctacatctgcaccgagggggaggaccagatcacggtctggggcttccactccgacaacaagacccagatgaagtccctgtacggggactccaacccgcagaagttcacgagctccgccaacggcgtgaccacgcactacgtcagccagatcggggacttcccggaccagaccgaggacggcgggctgccccagtccggccgcatcgtggtcgactacatgatgcagaagcccgggaagacgggcaccatcgtgtaccagcggggggtcctgctgccgcagaaggtgtggtgcgccagcggccgctccaaggtcatcaaggggagcctgcccctcatcggcgaggccgactgcctgcacgaggagtacgggggcctcaacaagtccaagccgtactacacggggaagcacgccaaggccatcggcaactgcccgatctgggtgaagacccccctgaagctcgccaacgggacgaagtaccggccgcccgccaagctgctcaaggagcgcggcttcttcggggccatcgccggcttcctggaggggggctgggaggggatgatcgccggctggcacgggtacaccagccacggcgcccacggggtcgcggtggccgcggacctcaagtccacgcaggaggccatcaacaagatcaccaagaacctgaacagcctctccgagctggaggtcaagaacctccagcgcctgagcggcgcgatggacgagctccacaacgagatcctggagctcgacgagaaggtggacgacctgcgggccgacacgatctcgtcccagatcgagctcgcggtcctgctcagcaacgaggggatcatcaactcggaggacgagcacctgctcgccctggagcggaagctcaagaagatgctgggcccgtccgcggtggacatcgggaacggctgcttcgagaccaagcacaagtgcaaccagacgtgcctcgaccgcatcgccgcggggaccttcaacgccggcgagttcagcctgcccacgttcgactcgctcaacatcaccgcggcctccctgaacgacgacgggctcgacaaccacacgatcctgctctactacagcaccgcggcctcgtccctggcggtcacgctcatgctggccatcttcatcgtgtacatggtcagccgcgacaacgtgtcgtgctccatctgcctctga

SEQ ID NO: 91 - DNA, 57 bp, synthetic construct
  source 1..57: mol_type = other DNA; note = 5'UTR-Moderna
gggaaataagagagaaaagaagagtaagaagaaatataagaccccggcgccgccacc

SEQ ID NO: 92 - DNA, 110 bp, synthetic construct
  source 1..110: mol_type = other DNA; note = 3'UTR-Moderna
gctggagcctcggtggcctagcttcttgccccttgggcctccccccagcccctcctccccttcctgcacccgtacccccgtggtctttgaataaagtctgagtgggcggc

SEQ ID NO: 93 - DNA, 1698 bp, synthetic construct
  source 1..1698: mol_type = other DNA; note = Influenza A H1N1 (A/Wisconsin/588/2019) HA Moderna
atgaaggccatcctggtcgtgatgctgtacaccttcaccaccgccaacgccgacaccctgtgcatcggctaccacgccaacaacagcaccgacaccgtggacaccgtgctggagaagaacgtgaccgtgacccacagcgtgaacctgctggaggacaagcacaacggcaagctgtgcaagctgaggggagtggcacccctgcacctgggcaagtgcaacatcgccggctggatcctgggcaaccccgagtgcgagagcctgagcacagcccggagctggagctacatcgtggagaccagcaacagcgacaacggcacctgttaccccggcgacttcatcaactacgaggagctgcgggagcagctgagcagcgtgagcagcttcgagcggttcgagatcttccccaagaccagcagctggcccaaccacgacagcgacaacggcgtgacagcagcctgtccacacgccggagccaagagcttctacaagaacctgatctggctggtgaagaagggcaagagctaccccaagatcaaccagacctacatcaacgacaagggcaaggaggtgctggtgctgtggggcatccaccacccacctaccatcgccgaccagcagagcctgtaccagaacgccgacgcctacgtgttcgtgggcaccagccggtacagcaagaagttcaagccagagatcgccacccggcccaaggtgagagaccaggagggccggatgaactactactggaccctggtggagcccggagacaagattaccttcgaggccaccggcaacctggtggcccctcggtacgccttcaccatggaacgggacgctggcagcggcatcatcatcagcgacactcccgtgcacgactgcaacaccacctgccagactcccgagggcgctatcaacaccagcctgcccttccagaacgtgcaccccatcaccatcggcaagtgccccaagtacgtaaagagcaccaaattgcggctggccaccggactcaggaacgtgcccagcatccaaagccggggcctgtttggcgcaatcgccggcttcatcgagggcggctggactggcatggtggacggctggtacggctaccaccaccagaacgaacaggggagcggctacgcagctgacctgaagagcacccagaacgccatcgacaagatcaccaacaaggtgaacagcgtgatcgagaagatgaacacccagttcaccgccgtgggcaaggagttcaaccacctggagaagcggatcgagaacctgaacaagaaggtggacgacggcttcctggacatctggacctacaacgccgagctgctggttctgctggagaacgagcggaccctggactatcacgacagcaacgtgaagaacctgtacgagaaggtgcggaaccagctgaagaacaacgccaaggagatcggcaacggctgcttcgagttctaccacaagtgcgacaacacctgcatggagagcgtgaagaacggcacctacgactaccccaagtacagcgaggaggccaagctgaaccgggagaagatcgacggcgtgaagctggacagcacccggatctaccagatcctggccatctacagcaccgtggccagcagcctggtgctggtggtgagcctgggcgccatcagcttctggatgtgcagcaacggcagcctgcagtgccggatctgcatc

SEQ ID NO: 94 - DNA, 1698 bp, synthetic construct
  source 1..1698: mol_type = other DNA; note = Influenza A H3N2 (A/Cambodia/e0826360/2020) HA Moderna
atgaagaccatcatcgccctgagctacatcctgtgcctggtgttcgcccagaagatccccggcaacgataacagcaccgccaccctgtgtctgggacaccacgccgtgcccaacggcaccatcgtgaagactatcaccaacgaccggatcgaggtgaccaacgccaccgagctggtgcagaacagcagcatcggcgagatctgcgacagccctcaccagatcctggacggcggcaactgcaccctgatcgacgcactgctgggcgaccctcagtgcgacggctttcagaacaaggagtgggacctgttcgtggagagatcgcgggccaacagcaactgctacccctacgacgtccccgactacgcaagcctgagaagcctcgtggcctcaagcggcaccctggagttcaagaacgagagcttcaactggaccggcgtgaagcagaacggcacctcaagcgcctgcatccggggctccagcagcagcttcttctcacggctgaactggctgacccacctgaactacacctaccccgccctgaacgtgaccatgcccaacaacgagcagttcgacaagctgtacatctggggagtgcaccatcccagcaccgacaaggaccagattagcctgttcgcccagcccagcggccggatcaccgtgagcaccaagcggagccagcaggccgtgatccccaacatcggctctcggcccagaatccgggacatccccagccggatcagcatctactggaccattgtgaagcccggcgacatcctgctgatcaactccaccggcaacctgatcgcccctcggggctatttcaagatccggagcggcaagagcagcatcatgcggagcgacgcccctatcggcaagtgcaagagcgagtgcatcacacccaacggaagcatccccaacgacaagcccttccagaacgtgaaccggataacctacggcgcctgccctagatacgtgaagcagagcaccctgaagctggccaccggcatgcggaacgtgcccgagaagcagactcggggcatcttcggcgccatcgccggcttcatcgagaacggctgggagggcatggtggacggctggtacggcttccggcaccagaactctgagggcagaggacaggccgcagacctgaagagcacccaggccgccatcgaccagatcaacggcaagctgaaccggctgatcggcaagaccaacgagaagttccaccagatcgagaaggagttcagcgaggtggagggcagggtacaggacctggagaagtacgtggaggacaccaagatcgacctgtggagctacaacgccgagctgctggtagccctggagaaccagcacaccatcgacctgaccgacagcgagatgaacaagctgttcgagaagaccaagaagcagctgcgggagaacgccgaggacatgggcaacggctgcttcaagatctaccacaagtgcgacaacgcctgcatcggcagcatccggaacgagacctacgaccacaacgtgtaccgggacgaggccctgaacaaccggttccagatcaagggcgtggagctgaagagcggctacaaggactggatcctgtggatcagcttcgccatgtcctgcttcctgctgtgcatcgccctgctgggtttcatcatgtgggcctgccagaagggcaacatccggtgcaacatctgcatc

SEQ ID NO: 95 - DNA, 1746 bp, synthetic construct
  source 1..1746: mol_type = other DNA; note = Influenza B Victoria lineage (B/Washington/02/2019) HA CDS Moderna
atgaaggccatcatcgtgctgttaatggtggtgaccagcaacgccgaccggatctgcaccggcatcacctctagcaacagccctcacgtggtgaagaccgccacacagggcgaggtgaacgtgaccggcgtgattcccctgaccaccacccctaccaagagccacttcgccaacctgaagggaaccgagacccggggcaagctgtgtcccaagtgcctgaactgcaccgacctggacgtggccctgggcagacccaagtgcaccggcaagatccccagcgcccgggtgtctatcctgcacgaagtgcggcccgtgactagcggctgcttccccatcatgcacgaccggaccaagatccggcagctgcccaacctgctgcggggctacgagcacgtgcggctgagcacccacaacgtgatcaacgccgaagacgcacccgggagaccatacgagatcggcaccagcggctcttgccccaacatcaccaacggcaacggcttcttcgctaccatggcctgggccgtgccaaagaacaagactgccaccaaccctctgaccatcgaggtgccctacatctgcaccgagggcgaggaccagatcaccgtgtggggcttccacagcgacagcgagacccagatggccaagctgtacggcgacagcaagccccagaagttcaccagcagcgccaacggcgtgaccacccactacgtgagccagatcggcggcttccccaaccagaccgaggacggcggcttaccccagagcggccggatcgtggtggactacatggtgcagaagagcggcaagaccggcaccatcacctaccagcggggcatcctgctgccacagaaggtgtggtgcgcctcagggcggtcaaaggtgatcaagggcagcctgccactgattggcgaggccgactgcctgcacgagaagtacggcggcctgaacaagagcaagccctactacaccggcgagcacgccaaggcaatcggcaactgccccatctgggtgaagacacccctgaagctggccaacggcaccaagtaccggccacccgccaaactgctgaaggagcggggcttcttcggcgccattgccggcttcctcgaaggcggttgggagggcatgatcgccggctggcacggctacactagccacggcgcacacggagtagcagtggccgccgacctgaagagcacccaggaggccatcaacaagatcaccaagaacctgaacagcctgagcgagctggaggtgaagaatctgcagcggctgtctggcgctatggacgagctgcacaacgagatcctggagctggacgagaaggtggacgacttacgggccgacaccatcagcagccagatcgagctggccgtgctgctctccaacgagggcatcatcaacagcgaggacgagcacctgctcgccctggagcggaagctgaagaagatgctgggcccttctgccgtggagatcggtaacggctgcttcgagaccaagcacaagtgcaaccagacctgcctggatcggatcgcagccggcacctttgacgccggggagttcagcctgcccaccttcgacagcctgaacatcaccgccgccagcctgaacgacgacggcctggacaaccacaccatcctgctgtactactctacagccgctagcagcctggccgtgaccctgatgatcgccatcttcgtggtgtacatggtgagccgggacaacgtgagctgcagcatctgcctg

SEQ ID NO: 96 - DNA, 1752 bp, synthetic construct
  source 1..1752: mol_type = other DNA; note = Influenza B Yamagata lineage (B/Phuket/3073/2013) HA CDS Moderna
atgaaggccatcatcgtgctactgatggtggtgaccagcaacgccgaccggatctgcaccggcatcaccagcagcaacagcccgcacgtggtgaagaccgccacccaaggcgaggtgaacgtgaccggcgtgatcccactgaccaccactcccaccaagagctacttcgccaacctgaagggcacacggactcggggcaagctgtgccccgactgcctgaactgcaccgacctggacgtggccctgggcagacccatgtgcgtgggcaccaccccttctgccaaggccagcatcctgcacgaggtgagacccgtgaccagcgggtgcttccccatcatgcacgaccggaccaagatccggcagctgcccaacctgctgcggggctacgagaagatccggctgagcacccagaacgtgatcgacgccgagaaggcccctggaggtccctaccggctgggcaccagcggaagctgccccaacgccaccagcaagatcggcttcttcgccaccatggcctgggctgtgcccaaggacaactacaagaacgccaccaatcccctgaccgtggaggtgccctacatctgcaccgagggcgaggaccagatcaccgtgtggggcttccacagcgacaacaagacccagatgaagagcctgtacggcgacagcaatccccagaagttcacaagcagcgccaacggcgtgaccacccactacgtgagccagatcggcgacttccccgaccagaccgaggacggagggctgcctcagagtggccggatcgtggtggactacatgatgcagaagcccggcaagaccggcaccatcgtgtaccagcggggcgtgctgttgcctcagaaagtttggtgtgccagcggcaggagcaaggtgatcaagggcagcctgcccctgatcggcgaggcagactgcctccacgaggagtacggcggcctgaacaagagcaagccctactacaccggcaagcacgccaaggccatcggcaactgccccatctgggtgaagacccctctgaagctggccaacggcaccaagtaccggccaccagccaagctgctgaaggagcggggcttctttggcgccattgccggcttcctcgagggaggctgggagggcatgatcgccggctggcacggctacacaagccacggcgcacacggagtggctgtggctgccgacctgaagagcacccaggaggccatcaacaagatcaccaagaacctgaacagcctgagcgagctggaggtgaagaacctgcagcggctgtcaggcgccatggacgagctgcacaacgagatcctggagctggacgagaaggtggacgacctgcgtgccgacaccatcagcagccagatcgagctggccgtgctgctgagcaacgagggcatcatcaacagcgaggacgagcacctgctggccctggagcggaaactgaagaagatgctgggaccctctgccgtggacatcggcaacggctgcttcgagaccaagcacaagtgcaaccagacctgcctggatcggatcgccgccggaaccttcaacgccggcgagttcagcctgcccaccttcgacagcctgaacatcaccgccgccagcctgaacgacgacggcctggacaaccacaccatcctgctgtactacagcactgccgcctcaagcctggccgtgaccctgatgctggccatcttcatcgtgtacatggtgagccgggacaacgtgagctgcagcatctgcctg

SEQ ID NO: 97 - DNA, 3810 bp, synthetic construct
  source 1..3810: mol_type = other DNA; note = SARS-COV-2 BA.4 Spike CDS
atgttcgtgttcctggtgctgctgcccctggtgagctctcagtgcgtgaacctgatcacaagaacacagtcgtacaccaacagcttcacaagaggcgtgtactaccccgacaaggtgttcagaagcagcgtgctgcactccacccaagacctgtttctgcccttcttcagcaacgtgacctggttccacgccatcagcggcaccaacggcaccaagagattcgacaaccccgtgctgcccttcaacgacggcgtgtacttcgctagcaccgaaaagagcaacatcatcagaggctggatcttcggcaccaccctagactccaagacacaaagcctgctgatcgttaacaacgcgaccaacgtggtgatcaaggtgtgcgagtttcagttctgcaacgaccccttcctggacgtgtactaccacaagaacaacaagagctggatggagagcgagttcagagtctacagcagcgccaacaactgcaccttcgagtacgtgtctcagcccttcctgatggacctggagggcaagcaaggcaatttcaagaacctaagagagttcgtgttcaagaacatcgacggctacttcaagatctacagcaagcacacccccatcaacctggggagagacctgccccaaggcttcagcgccctggagcccctggtggacctgcccatcggcatcaacatcacaagatttcagaccctgctggccctgcaccgtagctacctaacccccggcgatagttcctctggctggacggccggcgctgccgcctactacgtgggctacctgcagcctagaaccttcctgctgaagtacaacgagaacggcactatcactgatgccgtggactgtgccctggaccccctgagcgagaccaagtgcaccctcaagagcttcaccgtggagaagggcatctatcagacaagcaacttcagagtgcagcccaccgagagcatcgtgagattccccaacatcaccaacctgtgccccttcgacgaggtgttcaacgccacaagattcgctagcgtgtacgcgtggaacagaaagagaatcagcaactgcgtggccgactacagcgtgctgtacaacttcgctcccttcttcgccttcaagtgctatggcgtcagccccaccaagctgaacgacctgtgcttcaccaacgtgtacgccgacagcttcgtgatcagaggcaacgaggtgagccagattgcccccgggcaaaccggcaacatcgccgactacaactacaagctgcccgacgacttcaccggctgcgtgatcgcgtggaacagcaataagctggattccaaggtgggcggcaactacaactaccggtacagactgttcagaaagagcaacctgaagcccttcgagagagacatcagcaccgagatctaccaagccggcaacaagccctgcaacggcgtggcgggcgtcaactgctacttccccctgcagagctacggctttaggcccacctacggcgtgggccatcagccctacagagtggtggtgctgagcttcgagctgctgcacgcccccgcaaccgtgtgcggccccaaaaagagcaccaacctggtgaagaacaagtgcgtgaacttcaactttaatggccttaagggcacgggcgtgctgaccgagagcaacaagaagttcctgccatttcagcaattcggcagagacatcgccgacaccaccgacgcggtcagagaccctcagaccctggagatcctggacatcaccccctgtagcttcggcggcgtgagcgtgatcacccccggcactaacacaagcaaccaagtggccgtgctgtaccaaggcgtgaactgcaccgaggtgcccgtggccatccacgccgatcagctgacccccacctggagagtatacagcaccggaagcaacgtgtttcagacaagagccggctgcctgatcggcgccgagtacgtgaacaacagctacgagtgcgacatccccatcggcgccggcatctgcgctagctatcagacacagaccaagagccaccggagagctagaagcgtggcttctcagagcatcatcgcctacaccatgagcctgggcgccgagaacagcgtggcctacagcaacaacagcatcgccatccccaccaacttcaccatcagcgtgaccaccgagatcctgcccgtaagtatgaccaagacaagcgtggactgcaccatgtacatctgcggcgacagcaccgagtgcagcaacctgctgctgcagtacggcagcttctgcacacagctgaagagagccctgaccggcatcgccgtggagcaagacaagaacacccaagaggtgttcgcccaagtgaagcagatctacaagaccccccccatcaagtacttcggcggcttcaacttcagccaaatcctgcccgaccctagcaagcctagcaagcggagcttcatcgaggacctgctgttcaacaaggtgaccctggccgacgccggcttcatcaagcagtacggcgactgcctaggcgacatcgcagctagagacctgatctgcgctcagaagttcaatggactcaccgtgctcccccccctgctgaccgacgagatgatcgctcagtacacctctgccctgctggcgggaaccataacaagcggttggacatttggcgccggggccgcactgcaaatccccttcgccatgcagatggcctacagattcaacggcatcggcgtgacacagaacgtgctgtacgagaatcagaagctgatcgccaatcagttcaacagcgccatcggcaagatccaagacagcctgagcagcaccgctagcgccctgggcaagctgcaagacgtggtgaatcacaacgcccaagccctgaacaccctggtgaagcagctgagcagcaagttcggcgccatcagcagcgtattgaatgacatcctgtctagactggacccccccgaggccgaggtgcagatcgacagactgatcaccggcagactgcagagcctgcagacctacgtgacacagcagctgatcagagccgccgagatcagagctagcgccaacctggccgccaccaagatgagcgagtgcgtgctggggcagagcaagagagtggacttctgcggcaagggctaccacctgatgagcttccctcagagcgccccccacggcgtggtgttcctgcacgtgacctacgtgcccgcccaagagaagaacttcaccaccgctcccgccatctgccacgacggcaaggcccacttccctagagagggcgtgttcgtgagcaacggcacccactggttcgtgacacagagaaacttctacgagcctcagatcatcaccaccgacaacaccttcgtgagcggcaactgcgacgtggtgatcggcatagtgaacaacaccgtatacgaccccctgcagcccgagctggacagcttcaaggaggagctggacaagtacttcaaaaaccatactagccccgacgtggacctgggagacatctctggcatcaacgctagcgtggtgaacattcagaaggagatcgaccggctgaatgaggtggccaagaacctgaacgagagcctgatcgacctgcaagagctgggcaagtacgagcagtacatcaagtggccctggtacatctggctgggcttcatcgccggcctgatcgccatcgtgatggtgaccatcatgctgtgctgcatgacaagctgttgcagctgcctgaaaggttgctgcagctgtggctcgtgctgcaagttcgacgaggacgacagcgagcccgtgctgaagggcgtgaagctgcactacacctgatga

SEQ ID NO: 98 - protein, 566 aa, Influenza A H1N1
MKAILVVMLYTFTTANADTLCIGYHANNSTDTVDTVLEKNVTVTHSVNLLEDKHNGKLCKLRGVAPLHLGKCNIAGWILGNPECESLSTARSWSYIVETSNSDNGTCYPGDFINYEELREQLSSVSSFERFEIFPKTSSWPNHDSDNGVTAACPHAGAKSFYKNLIWLVKKGKSYPKINQTYINDKGKEVLVLWGIHHPPTIADQQSLYQNADAYVFVGTSRYSKKFKPEIATRPKVRDQEGRMNYYWTLVEPGDKITFEATGNLVAPRYAFTMERDAGSGIIISDTPVHDCNTTCQTPEGAINTSLPFQNVHPITIGKCPKYVKSTKLRLATGLRNVPSIQSQGLFGAIAGFIEGGWTGMVDGWYGYHHQNEQGSGYAADLKSTQNAIDKITNKVNSVIEKMNTQFTAVGKEFNHLEKRIENLNKKVDDGFLDIWTYNAELLVLLENERTLDYHDSNVKNLYEKVRNQLKNNAKEIGNGCFEFYHKCDNTCMESVKNGTYDYPKYSEEAKLNREKIDGVKLDSTRIYQILAIYSTVASSLVLVVSLGAISFWMCSNGSLQCRICI

SEQ ID NO: 99 - protein, 566 aa, Influenza A H3N2
MKTIIALSYILCLVFAQKIPGNDNSTATLCLGHHAVPNGTIVKTITNDRIEVTNATELVQNSSIGEICDSPHQILDGGNCTLIDALLGDPQCDGFQNKEWDLFVERSRANSNCYPYDVPDYASLRSLVASSGTLEFKNESFNWTGVKQNGTSSACIRGSSSSFFSRLNWLTHLNYTYPALNVTMPNNEQFDKLYIWGVHHPSTDKDQISLFAQPSGRITVSTKRSQQAVIPNIGSRPRIRDIPSRISIYWTIVKPGDILLINSTGNLIAPRGYFKIRSGKSSIMRSDAPIGKCKSECITPNGSIPNDKPFQNVNRITYGACPRYVKQSTLKLATGMRNVPEKQTQGIFGAIAGFIENGWEGMVDGWYGFRHQNSEGRGQAADLKSTQAAIDQINGKLNRLIGKTNEKFHQIEKEFSEVEGRVQDLEKYVEDTKIDLWSYNAELLVALENQHTIDLTDSEMNKLFEKTKKQLRENAEDMGNGCFKIYHKCDNACIGSIRNETYDHNVYRDEALNNRFQIKGVELKSGYKDWILWISFAMSCFLLCIALLGFIMWACQKGNIRCNICI

SEQ ID NO: 100 - protein, 582 aa, Influenza B Victoria lineage
MKAIIVLLMVVTSNADRICTGITSSNSPHVVKTATQGEVNVTGVIPLTTTPTKSHFANLKGTETRGKLCPKCLNCTDLDVALGRPKCTGKIPSARVSILHEVRPVTSGCFPIMHDRTKIRQLPNLLRGYEHVRLSTHNVINAEDAPGRPYEIGTSGSCPNITNGNGFFATMAWAVPKNKTATNPLTIEVPYICTEGEDQITVWGFHSDNETQMAKLYGDSKPQKFTSSANGVTTHYVSQIGGFPNQTEDGGLPQSGRIVVDYMVQKSGKTGTITYQRGILLPQKVWCASGRSKVIKGSLPLIGEADCLHEKYGGLNKSKPYYTGEHAKAIGNCPIWVKTPLKLANGTKYRPPAKLLKEQGFFGAIAGFLEGGWEGMIAGWHGYTSHGAHGVAVAADLKSTQEAINKITKNLNSLSELEVKNLQRLSGAMDELHNEILELDEKVDDLRADTISSQIELAVLLSNEGIINSEDEHLLALERKLKKMLGPSAVEIGNGCFETKHKCNQTCLDRIAAGTFDAGEFSLPTFDSLNITAASLNDDGLDNHTILLYYSTAASSLAVTLMIAIFVVYMVSRDNVSCSICL

SEQ ID NO: 101 - protein, 584 aa, Influenza B Yamagata lineage
MKAIIVLLMVVTSNADRICTGITSSNSPHVVKTATQGEVNVTGVIPLTTTPTKSYFANLKGTRTRGKLCPDCLNCTDLDVALGRPMCVGTTPSAKASILHEVRPVTSGCFPIMHDRTKIRQLPNLLRGYEKIRLSTQNVIDAEKAPGGPYRLGTSGSCPNATSKIGFFATMAWAVPKDNYKNATNPLTVEVPYICTEGEDQITVWGFHSDNKTQMKSLYGDSNPQKFTSSANGVTTHYVSQIGDFPDQTEDGGLPQSGRIVVDYMMQKPGKTGTIVYQRGVLLPQKVWCASGRSKVIKGSLPLIGEADCLHEEYGGLNKSKPYYTGKHAKAIGNCPIWVKTPLKLANGTKYRPPAKLLKEQGFFGAIAGFLEGGWEGMIAGWHGYTSHGAHGVAVAADLKSTQEAINKITKNLNSLSELEVKNLQRLSGAMDELHNEILELDEKVDDLRADTISSQIELAVLLSNEGIINSEDEHLLALERKLKKMLGPSAVDIGNGCFETKHKCNQTCLDRIAAGTFNAGEFSLPTFDSLNITAASLNDDGLDNHTILLYYSTAASSLAVTLMLAIFIVYMVSRDNVSCSICL

SEQ ID NO: 102 - DNA, 1701 bp, synthetic construct
  source 1..1701: mol_type = other DNA; note = Influenza A H1N1 HA0 mutant CDS
atgaaggccatcctggtggtgatgctgtacaccttcaccaccgccaacgccgacaccctgtgcatcggctaccacgccaacaacagcaccgacaccgtggacaccgtgctggagaagaacgtgaccgtgacccacagcgtgaacctgctggaggacaagcacaacggcaagctgtgcaagctgcggggcgtggcccccctgcacctgggcaagtgcaacatcgccggctggatcctgggcaaccccgagtgcgagtccctgagcaccgcccgctcctggagctacatcgtggagacctccaacagcgacaacggcacctgctaccccggggacttcatcaactacgaggagctgcgggagcagctgtccagcgtgtccagcttcgagcgcttcgagatcttccccaagacctccagctggcccaaccacgactccgacaacggcgtgaccgccgcctgcccccacgccggggccaagagcttctacaagaacctgatctggctggtgaagaagggcaagtcctaccccaagatcaaccagacctacatcaacgacaaggggaaggaggtcctcgtgctgtggggcatccaccacccccccaccatcgccgaccagcagagcctctaccagaacgccgacgcctacgtcttcgtggggacctcccggtacagcaagaagttcaagcccgagatcgccacccgccccaaggtccgggaccaggagggccgcatgaactactactggaccctggtggagccgggggacaagatcaccttcgaggccaccggcaacctcgtcgccccgcggtacgccttcacgatggagcgcgacgccgggtccggcatcatcatcagcgacacccccgtgcacgactgcaacacgacctgccagacgcccgagggggcgatcaacacctccctgccgttccagaacgtccacccgatcacgatcggcaagtgccccaagtacgtgaagtccaccaagctccggctggccacggggctccgcaacgtcccctccatccagagccagggcctgttcggggcgatcgccggcttcatcgaggggggctggaccgggatggtggacggctggtacgggtaccaccaccagaacgagcagggctccgggtacgcggccgacctcaagtcgacgcagaacgcgatcgacaagatcaccaacaaggtcaacagcgtgatcgagaagatgaacacgcagttcaccgccgtcggcaaggagttcaaccacctggagaagcgcatcgagaacctcaacaagaaggtggacgacgggttcctggacatctggacgtacaacgcggagctcctggtcctcctggagaacgagcggaccctcgactaccacgactccaacgtgaagaacctgtacgagaaggtccgcaaccagctcaagaacaacgccaaggagatcggcaacgggtgcttcgagttctaccacaagtgcgacaacacgtgcatggagtcggtgaagaacggcacctacgactacccgaagtacagcgaggaggcgaagctgaaccgggagaagatcgacggggtcaagctcgactccacgcgcatctaccagatcctggccatctactcgaccgtggcgagctccctcgtcctggtggtctcgctcggcgccatcagcttctggatgtgctccaacgggtcgctgcagtgccggatctgcatctga

SEQ ID NO: 103 - DNA, 1701 bp, synthetic construct
  source 1..1701: mol_type = other DNA; note = Influenza A H3N2 HA0 mutant CDS
atgaagaccatcatcgccctgagctacatcctgtgcctggtgttcgcccagaagatccccggcaacgacaacagcaccgccaccctgtgcctgggccaccacgccgtgcccaacggcaccatcgtgaagaccatcaccaacgaccggatcgaggtgaccaacgccaccgagctggtgcagaactccagcatcggcgagatctgcgactccccccaccagatcctggacggcggcaactgcaccctgatcgacgccctgctgggcgacccccagtgcgacgggttccagaacaaggagtgggacctgttcgtggagcggagccgcgccaactccaactgctacccctacgacgtgcccgactacgccagcctgcggtccctggtggccagctccggcaccctggagttcaagaacgagagcttcaactggaccggggtcaagcagaacggcacctccagcgcctgcatccgcgggtccagctccagcttcttctcccggctgaactggctcacccacctgaactacacctaccccgccctcaacgtgaccatgcccaacaacgagcagttcgacaagctgtacatctggggcgtccaccaccccagcaccgacaaggaccagatctccctcttcgcccagcccagcgggcgcatcaccgtgtccacgaagcggagccagcaggccgtcatccccaacatcggctcccgcccgcggatccgcgacatccccagccggatctccatctactggacgatcgtgaagccgggggacatcctgctcatcaacagcaccggcaacctgatcgccccccgcgggtacttcaagatccggtccggcaagagctcgatcatgcgctccgacgccccgatcgggaagtgcaagagcgagtgcatcacccccaacggctcgatcccgaacgacaagcccttccagaacgtcaaccggatcacgtacggggcctgcccgcgctacgtgaagcagtccacgctcaagctggccaccggcatgcggaacgtccccgagaagcagacccaggggatcttcggcgccatcgcggggttcatcgagaacggctgggaggggatggtggacggctggtacgggttccggcaccagaacagcgagggccgcgggcaggccgcggacctcaagtcgacgcaggccgcgatcgaccagatcaacggcaagctgaaccggctcatcgggaagacgaacgagaagttccaccagatcgagaaggagttctccgaggtcgagggccgcgtgcaggacctggagaagtacgtcgaggacaccaagatcgacctctggagctacaacgccgagctgctcgtggcgctggagaaccagcacaccatcgacctcacggactcggagatgaacaagctgttcgagaagacgaagaagcagctccgggagaacgccgaggacatggggaacggctgcttcaagatctaccacaagtgcgacaacgcgtgcatcgggtccatccgcaacgagacctacgaccacaacgtctaccgggacgaggccctgaacaaccgcttccagatcaagggcgtggagctcaagagcgggtacaaggactggatcctgtggatctcgttcgcgatgtcctgcttcctcctgtgcatcgccctcctgggcttcatcatgtgggcgtgccagaaggggaacatccggtgcaacatctgcatctga

SEQ ID NO: 104 - DNA, 1749 bp, synthetic construct
  source 1..1749: mol_type = other DNA; note = Influenza B Victoria HA0 mutant CDS
atgaaggccatcatcgtgctgctgatggtggtgaccagcaacgccgaccggatctgcaccggcatcaccagctccaacagcccccacgtggtgaagaccgccacccagggcgaggtgaacgtgaccggcgtgatccccctgaccaccacccccaccaagtcccacttcgccaacctgaagggcaccgagacccggggcaagctgtgccccaagtgcctgaactgcaccgacctggacgtggccctgggccgccccaagtgcaccggcaagatccccagcgcccgggtgtccatcctgcacgaggtgcgccccgtgaccagcggctgcttccccatcatgcacgaccgcaccaagatccggcagctgcccaacctgctgcgggggtacgagcacgtccgcctgtccacccacaacgtgatcaacgccgaggacgcccccggccggccctacgagatcgggaccagcggctcctgccccaacatcaccaacgggaacggcttcttcgccaccatggcctgggccgtccccaagaacaagaccgccaccaaccccctgaccatcgaggtgccgtacatctgcaccgagggggaggaccagatcaccgtctggggcttccacagcgacaacgagacgcagatggccaagctgtacggggactccaagccccagaagttcacgagctccgccaacggcgtgaccacccactacgtcagccagatcgggggcttcccgaaccagacggaggacgggggcctgccccagtccgggcgcatcgtggtcgactacatggtgcagaagtccggcaagacggggaccatcacgtaccagcggggcatcctgctgccgcagaaggtctggtgcgcctccgggcgcagcaaggtgatcaagggctccctgcccctcatcggggaggccgactgcctgcacgagaagtacggcgggctcaacaagagcaagccgtactacaccggcgagcacgccaaggccatcgggaactgccccatctgggtcaagaccccgctgaagctcgccaacggcacgaagtaccggcccccggccaagctgctcaaggagcaggggttcttcggcgccatcgccgggttcctggagggcgggtgggagggcatgatcgccgggtggcacggctacacgtcccacggggcccacggcgtggcggtcgccgcggacctcaagagcacccaggaggccatcaacaagatcacgaagaacctgaactccctcagcgagctggaggtgaagaacctccagcgcctgtccggggcgatggacgagctccacaacgagatcctggagctcgacgagaaggtcgacgacctgcgggccgacaccatcagctcgcagatcgagctcgcggtgctgctctccaacgagggcatcatcaacagcgaggacgagcacctgctcgccctggagcggaagctcaagaagatgctggggccctcggcggtcgagatcggcaacgggtgcttcgagaccaagcacaagtgcaaccagacgtgcctcgaccgcatcgccgcgggcacgttcgacgccggggagttctccctgccgaccttcgacagcctcaacatcacggcggcctcgctgaacgacgacggcctcgacaaccacaccatcctgctctactactccaccgcggccagctcgctggcggtgacgctcatgatcgccatcttcgtcgtgtacatggtctcccgcgacaacgtgagctgctcgatctgcctgtga

SEQ ID NO: 105 - DNA, 1755 bp, synthetic construct
  source 1..1755: mol_type = other DNA; note = Influenza B Yamagata HA0 mutant CDS
atgaaggccatcatcgtgctgctgatggtggtgaccagcaacgccgaccggatctgcaccggcatcaccagctccaacagcccccacgtggtgaagaccgccacccagggcgaggtgaacgtgaccggcgtgatccccctgaccaccacccccaccaagtcctacttcgccaacctgaagggcacccggacccgcggcaagctgtgccccgactgcctgaactgcaccgacctggacgtggccctgggccggcccatgtgcgtgggcaccacccccagcgccaaggcctccatcctgcacgaggtgcgccccgtgaccagcggctgcttccccatcatgcacgaccgcaccaagatccggcagctgcccaacctgctgcgggggtacgagaagatccgcctgtccacccagaacgtcatcgacgccgagaaggcccccggcgggccctaccggctgggcaccagcgggtcctgccccaacgccaccagcaagatcggcttcttcgccaccatggcctgggccgtgcccaaggacaactacaagaacgccaccaaccccctgaccgtcgaggtgccctacatctgcaccgagggggaggaccagatcacggtctggggcttccactccgacaacaagacccagatgaagtccctgtacggggactccaacccgcagaagttcacgagctccgccaacggcgtgaccacgcactacgtcagccagatcggggacttcccggaccagaccgaggacggcgggctgccccagtccggccgcatcgtggtcgactacatgatgcagaagcccgggaagacgggcaccatcgtgtaccagcggggggtcctgctgccgcagaaggtgtggtgcgccagcggccgctccaaggtcatcaaggggagcctgcccctcatcggcgaggccgactgcctgcacgaggagtacgggggcctcaacaagtccaagccgtactacacggggaagcacgccaaggccatcggcaactgcccgatctgggtgaagacccccctgaagctcgccaacgggacgaagtaccggccgcccgccaagctgctcaaggagcagggcttcttcggggccatcgccggcttcctggaggggggctgggaggggatgatcgccggctggcacgggtacaccagccacggcgcccacggggtcgcggtggccgcggacctcaagtccacgcaggaggccatcaacaagatcaccaagaacctgaacagcctctccgagctggaggtcaagaacctccagcgcctgagcggcgcgatggacgagctccacaacgagatcctggagctcgacgagaaggtggacgacctgcgggccgacacgatctcgtcccagatcgagctcgcggtcctgctcagcaacgaggggatcatcaactcggaggacgagcacctgctcgccctggagcggaagctcaagaagatgctgggcccgtccgcggtggacatcgggaacggctgcttcgagaccaagcacaagtgcaaccagacgtgcctcgaccgcatcgccgcggggaccttcaacgccggcgagttcagcctgcccacgttcgactcgctcaacatcaccgcggcctccctgaacgacgacgggctcgacaaccacacgatcctgctctactacagcaccgcggcctcgtccctggcggtcacgctcatgctggccatcttcatcgtgtacatggtcagccgcgacaacgtgtcgtgctccatctgcctctga

SEQ ID NO: 106 - RNA, 4142 nt, synthetic construct
  source 1..4142: mol_type = other RNA; note = I'-Delta24-B-120A mRNA
gagttaggagttggtggcagtttcaataacaggtcattgccgagaaaaggatagcactataatatgttcgtgttcctggtgctgctgcccctggtgagctctcagtgcgtgaacctgaggacaagaacacagctgccccccgcctacaccaacagcttcacaagaggcgtgtactaccccgacaaggtgttcagaagcagcgtgctgcactccacccaagacctgtttctgcccttcttcagcaacgtgacctggttccacgccatccacgtcagcggcaccaacggcaccaagagattcgacaaccccgtgctgcccttcaacgacggcgtgtacttcgctagcaccgaaaagagcaacatcatcagaggctggatcttcggcaccaccctagactccaagacacaaagcctgctgatcgttaacaacgcgaccaacgtggtgatcaaggtgtgcgagtttcagttctgcaacgaccccttcctggacgtgtactaccacaagaacaacaagagctggatggagagcggggtctacagcagcgccaacaactgcaccttcgagtacgtgtctcagcccttcctgatggacctggagggcaagcaaggcaatttcaagaacctaagagagttcgtgttcaagaacatcgacggctacttcaagatctacagcaagcacacccccatcaacctggtgagagacctgccccaaggcttcagcgccctggagcccctggtggacctgcccatcggcatcaacatcacaagatttcagaccctgctggccctgcaccgtagctacctaacccccggcgatagttcctctggctggacggccggcgctgccgcctactacgtgggctacctgcagcctagaaccttcctgctgaagtacaacgagaacggcactatcactgatgccgtggactgtgccctggaccccctgagcgagaccaagtgcaccctcaagagcttcaccgtggagaagggcatctatcagacaagcaacttcagagtgcagcccaccgagagcatcgtgagattccccaacatcaccaacctgtgccccttcggcgaggtgttcaacgccacaagattcgctagcgtgtacgcgtggaacagaaagagaatcagcaactgcgtggccgactacagcgtgctgtacaacagcgctagcttcagcaccttcaagtgctatggcgtcagccccaccaagctgaacgacctgtgcttcaccaacgtgtacgccgacagcttcgtgatcagaggcgacgaggtgagacagattgcccccgggcaaaccggcaagatcgccgactacaactacaagctgcccgacgacttcaccggctgcgtgatcgcgtggaacagcaataacctggattccaaggtgggcggcaactacaactaccggtacagactgttcagaaagagcaacctgaagcccttcgagagagacatcagcaccgagatctaccaagccggcagcaagccctgcaacggcgtggagggcttcaactgctacttccccctgcagagctacggctttcagcccaccaacggcgtgggctatcagccctacagagtggtggtgctgagcttcgagctgctgcacgcccccgcaaccgtgtgcggccccaaaaagagcaccaacctggtgaagaacaagtgcgtgaacttcaactttaatggccttaccggcacgggcgtgctgaccgagagcaacaagaagttcctgccatttcagcaattcggcagagacatcgccgacaccaccgacgcggtcagagaccctcagaccctggagatcctggacatcaccccctgtagcttcggcggcgtgagcgtgatcacccccggcactaacacaagcaaccaagtggccgtgctgtaccaaggcgtgaactgcaccgaggtgcccgtggccatccacgccgatcagctgacccccacctggagagtatacagcaccggaagcaacgtgtttcagacaagagccggctgcctgatcggcgccgagcacgtgaacaacagctacgagtgcgacatccccatcggcgccggcatctgcgctagctatcagacacagaccaacagccgccggagagctagaagcgtggcttctcagagcatcatcgcctacaccatgagcctgggcgccgagaacagcgtggcctacagcaacaacagcatcgccatccccaccaacttcaccatcagcgtgaccaccgagatcctgcccgtaagtatgaccaagacaagcgtggactgcaccatgtacatctgcggcgacagcaccgagtgcagcaacctgctgctgcagtacggcagcttctgcacacagctgaacagagccctgaccggcatcgccgtggagcaagacaagaacacccaagaggtgttcgcccaagtgaagcagatctacaagaccccccccatcaaggacttcggcggcttcaacttcagccaaatcctgcccgaccctagcaagcctagcaagcggagcttcatcgaggacctgctgttcaacaaggtgaccctggccgacgccggcttcatcaagcagtacggcgactgcctaggcgacatcgcagctagagacctgatctgcgctcagaagttcaatggactcaccgtgctcccccccctgctgaccgacgagatgatcgctcagtacacctctgccctgctggcgggaaccataacaagcggttggacatttggcgccggggccgcactgcaaatccccttcgccatgcagatggcctacagattcaacggcatcggcgtgacacagaacgtgctgtacgagaatcagaagctgatcgccaatcagttcaacagcgccatcggcaagatccaagacagcctgagcagcaccgctagcgccctgggcaagctgcaaaacgtggtgaatcagaacgcccaagccctgaacaccctggtgaagcagctgagcagcaacttcggcgccatcagcagcgtattgaatgacatcctgtctagactggacccccccgaggccgaggtgcagatcgacagactgatcaccggcagactgcagagcctgcagacctacgtgacacagcagctgatcagagccgccgagatcagagctagcgccaacctggccgccaccaagatgagcgagtgcgtgctggggcagagcaagagagtggacttctgcggcaagggctaccacctgatgagcttccctcagagcgccccccacggcgtggtgttcctgcacgtgacctacgtgcccgcccaagagaagaacttcaccaccgctcccgccatctgccacgacggcaaggcccacttccctagagagggcgtgttcgtgagcaacggcacccactggttcgtgacacagagaaacttctacgagcctcagatcatcaccaccgacaacaccttcgtgagcggcaactgcgacgtggtgatcggcatagtgaacaacaccgtatacgaccccctgcagcccgagctggacagcttcaaggaggagctggacaagtacttcaaaaaccatactagccccgacgtggacctgggagacatctctggcatcaacgctagcgtggtgaacattcagaaggagatcgaccggctgaatgaggtggccaagaacctgaacgagagcctgatcgacctgcaagagctgggcaagtacgagcagtacatcaagtggccctggtacatctggctgggcttcatcgccggcctgatcgccatcgtgatggtgaccatcatgctgtgctgcatgacaagctgttgcagctgcctgaaaggttgctgcagctgtggctcgtgctgcaagttcgacgaggacgacagcgagcccgtgctgaagggcgtgaagctgcactacacctgatgactcgaggctcgctttcttgctgtccaatttctattaaaggttcctttgttccctaagtccaactactaaactgggggatattatgaagggccttgagcatctggattctgcctaataaaaaacatttattttcattgcaaaaaaaaaaaaaaaaaaaaaaaaaaaaaaaaaaaaaaaaaaaaaaaaaaaaaaaaaaaaaaaaaaaaaaaaaaaaaaaaaaaaaaaaaaaaaaaaaaaaaaaaaaaaaaaaaaaaaaaaaa

SEQ ID NO: 107 - RNA, 4139 nt, synthetic construct
  source 1..4139: mol_type = other RNA; note = I'-OC24-B-120A mRNA
gagttaggagttggtggcagtttcaataacaggtcattgccgagaaaaggatagcactataatatgttcgtgttcctggtgctgctgcccctggtgagctctcagtgcgtgaacctgaccacaagaacacagctgccccccgcctacaccaacagcttcacaagaggcgtgtactaccccgacaaggtgttcagaagcagcgtgctgcactccacccaagacctgtttctgcccttcttcagcaacgtgacctggttccacgtgatcagcggcaccaacggcaccaagagattcgacaaccccgtgctgcccttcaacgacggcgtgtacttcgctagcatcgaaaagagcaacatcatcagaggctggatcttcggcaccaccctagactccaagacacaaagcctgctgatcgttaacaacgcgaccaacgtggtgatcaaggtgtgcgagtttcagttctgcaacgaccccttcctggaccacaagaacaacaagagctggatggagagcgagttcagagtgtacagcagcgccaacaactgcaccttcgagtacgtgtctcagcccttcctgatggacctggagggcaagcaaggcaatttcaagaacctaagagagttcgtgttcaagaacatcgacggctacttcaagatctacagcaagcacacccccatcatcgtgagagagcccgaggacctgccccaaggcttcagcgccctggagcccctggtggacctgcccatcggcatcaacatcacaagatttcagaccctgctggccctgcaccgtagctacctaacccccggcgatagttcctctggctggacggccggcgctgccgcctactacgtgggctacctgcagcctagaaccttcctgctgaagtacaacgagaacggcactatcactgatgccgtggactgtgccctggaccccctgagcgagaccaagtgcaccctcaagagcttcaccgtggagaagggcatctatcagacaagcaacttcagagtgcagcccaccgagagcatcgtgagattccccaacatcaccaacctgtgccccttcgacgaggtgttcaacgccaccagatttgctagcgtgtacgcctggaaccggaagagaatcagcaactgcgtggccgactacagcgtgctgtacaacctggcccccttcttcaccttcaagtgctatggcgtcagccccaccaagctgaacgacctgtgcttcaccaacgtgtacgccgacagcttcgtgatcagaggcgacgaggtgagacagatcgcccccgggcagaccggcaacatcgccgactacaactacaagctgcccgacgacttcaccggctgcgtgatcgcctggaacagcaacaagctggatagcaaggtgagcggcaactacaattacctgtacagactgttcagaaagagcaacctgaagcccttcgagagagacatcagcaccgagatctaccaagccggcaacaagccctgcaacggcgtggcgggcttcaactgctacttccccctcaggagctacagcttcagacccacctacggcgtgggccatcagccctacagagtggtcgtgctgagcttcgagctgctgcacgcccctgccacagtgtgcggccccaaaaagagcaccaacctggtgaagaacaagtgcgtgaacttcaacttcaacggcctgaagggcaccggcgtgctgaccgagagcaacaagaagttcctgccatttcagcaattcggcagagacatcgccgacaccaccgacgcggtcagagaccctcagaccctggagatcctggacatcaccccctgtagcttcggcggcgtgagcgtgatcacccccggcactaacacaagcaaccaagtggccgtgctgtaccaaggcgtgaactgcaccgaggtgcccgtggccatccacgccgatcagctgacccccacctggagagtgtatagcaccggcagcaacgtgtttcagacaagagccggctgcctgatcggcgccgagtacgtgaacaacagctacgagtgcgacatccccatcggcgccggcatctgcgctagctatcagacacagaccaagagccaccggagagctagaagcgtggctagccaaagcatcatcgcctacaccatgagcctgggcgccgagaacagcgtggcctacagcaacaacagcatcgccatccccaccaacttcaccatcagcgtgaccaccgagatcctgcccgtaagtatgaccaagacaagcgtggactgcaccatgtacatctgcggcgacagcaccgagtgcagcaacctgctcctgcagtacggcagcttctgcacacagctgaagagagccctgaccggcatcgccgtggagcaagacaagaacacccaagaggtgttcgcccaagtgaagcagatctacaagaccccccccatcaagtacttcggcggcttcaacttcagccaaatcctgcccgaccctagcaagcctagcaagcggagcttcatcgaggacctgctgttcaacaaggtgaccctggccgacgccggcttcatcaagcagtacggcgactgcctaggcgacatcgcagctagagacctgatctgcgctcagaagttcaagggactcaccgtgctcccccccctgctgaccgacgagatgatcgctcagtacacctctgccctgctggcgggaaccataacaagcggttggacatttggcgccggggccgcactgcaaatccccttcgccatgcagatggcctacagattcaacggcatcggcgtgacacagaacgtgctgtacgagaatcagaagctgatcgccaatcagttcaacagcgccatcggcaagatccaagacagcctgagcagcaccgctagcgccctgggcaagctgcaagacgtggtgaaccacaacgcccaagccctgaacaccctggtgaagcagctgagcagcaagttcggcgccatcagcagcgtgctgaatgacatcttctctagactggacccccccgaggccgaggtgcagatcgacagactgatcaccggcagactgcagagcctgcagacctacgtgacacagcagctgatcagagccgccgagatcagagctagcgccaacctggccgccaccaagatgagcgagtgcgtgctggggcagagcaagagagtggacttctgcggcaagggctaccacctgatgagcttccctcagagcgccccccacggcgtggtgttcctgcacgtgacctacgtgcccgcccaagagaagaacttcaccaccgctcccgccatctgccacgacggcaaggcccacttccctagagagggcgtgttcgtgagcaacggcacccactggttcgtgacacagagaaacttctacgagcctcagatcatcaccaccgacaacaccttcgtgagcggcaactgcgacgtggtgatcggcatagtgaacaacaccgtatacgaccccctgcagcccgagctggacagcttcaaggaggagctggacaagtacttcaaaaaccatactagccccgacgtggacctgggagacatctctggcatcaacgctagcgtggtgaacattcagaaggagatcgaccggctgaatgaggtggccaagaacctgaacgagagcctgatcgacctgcaagagctgggcaagtacgagcagtacatcaagtggccctggtacatctggctgggcttcatcgccggcctgatcgccatcgtgatggtgaccatcatgctgtgctgcatgacaagctgttgcagctgcctgaaaggttgctgcagctgtggctcgtgctgcaagttcgacgaggacgacagcgagcccgtgctgaagggcgtgaagctgcactacacctgatgactcgaggctcgctttcttgctgtccaatttctattaaaggttcctttgttccctaagtccaactactaaactgggggatattatgaagggccttgagcatctggattctgcctaataaaaaacatttattttcattgcaaaaaaaaaaaaaaaaaaaaaaaaaaaaaaaaaaaaaaaaaaaaaaaaaaaaaaaaaaaaaaaaaaaaaaaaaaaaaaaaaaaaaaaaaaaaaaaaaaaaaaaaaaaaaaaaaaaaaaaaaa

SEQ ID NO: 108 - RNA, 4133 nt, synthetic construct
  source 1..4133: mol_type = other RNA; note = I'-BA4-B-120A mRNA
gagttaggagttggtggcagtttcaataacaggtcattgccgagaaaaggatagcactataatatgttcgtgttcctggtgctgctgcccctggtgagctctcagtgcgtgaacctgatcacaagaacacagtcgtacaccaacagcttcacaagaggcgtgtactaccccgacaaggtgttcagaagcagcgtgctgcactccacccaagacctgtttctgcccttcttcagcaacgtgacctggttccacgccatcagcggcaccaacggcaccaagagattcgacaaccccgtgctgcccttcaacgacggcgtgtacttcgctagcaccgaaaagagcaacatcatcagaggctggatcttcggcaccaccctagactccaagacacaaagcctgctgatcgttaacaacgcgaccaacgtggtgatcaaggtgtgcgagtttcagttctgcaacgaccccttcctggacgtgtactaccacaagaacaacaagagctggatggagagcgagttcagagtctacagcagcgccaacaactgcaccttcgagtacgtgtctcagcccttcctgatggacctggagggcaagcaaggcaatttcaagaacctaagagagttcgtgttcaagaacatcgacggctacttcaagatctacagcaagcacacccccatcaacctggggagagacctgccccaaggcttcagcgccctggagcccctggtggacctgcccatcggcatcaacatcacaagatttcagaccctgctggccctgcaccgtagctacctaacccccggcgatagttcctctggctggacggccggcgctgccgcctactacgtgggctacctgcagcctagaaccttcctgctgaagtacaacgagaacggcactatcactgatgccgtggactgtgccctggaccccctgagcgagaccaagtgcaccctcaagagcttcaccgtggagaagggcatctatcagacaagcaacttcagagtgcagcccaccgagagcatcgtgagattccccaacatcaccaacctgtgccccttcgacgaggtgttcaacgccacaagattcgctagcgtgtacgcgtggaacagaaagagaatcagcaactgcgtggccgactacagcgtgctgtacaacttcgctcccttcttcgccttcaagtgctatggcgtcagccccaccaagctgaacgacctgtgcttcaccaacgtgtacgccgacagcttcgtgatcagaggcaacgaggtgagccagattgcccccgggcaaaccggcaacatcgccgactacaactacaagctgcccgacgacttcaccggctgcgtgatcgcgtggaacagcaataagctggattccaaggtgggcggcaactacaactaccggtacagactgttcagaaagagcaacctgaagcccttcgagagagacatcagcaccgagatctaccaagccggcaacaagccctgcaacggcgtggcgggcgtcaactgctacttccccctgcagagctacggctttaggcccacctacggcgtgggccatcagccctacagagtggtggtgctgagcttcgagctgctgcacgcccccgcaaccgtgtgcggccccaaaaagagcaccaacctggtgaagaacaagtgcgtgaacttcaactttaatggccttaagggcacgggcgtgctgaccgagagcaacaagaagttcctgccatttcagcaattcggcagagacatcgccgacaccaccgacgcggtcagagaccctcagaccctggagatcctggacatcaccccctgtagcttcggcggcgtgagcgtgatcacccccggcactaacacaagcaaccaagtggccgtgctgtaccaaggcgtgaactgcaccgaggtgcccgtggccatccacgccgatcagctgacccccacctggagagtatacagcaccggaagcaacgtgtttcagacaagagccggctgcctgatcggcgccgagtacgtgaacaacagctacgagtgcgacatccccatcggcgccggcatctgcgctagctatcagacacagaccaagagccaccggagagctagaagcgtggcttctcagagcatcatcgcctacaccatgagcctgggcgccgagaacagcgtggcctacagcaacaacagcatcgccatccccaccaacttcaccatcagcgtgaccaccgagatcctgcccgtaagtatgaccaagacaagcgtggactgcaccatgtacatctgcggcgacagcaccgagtgcagcaacctgctgctgcagtacggcagcttctgcacacagctgaagagagccctgaccggcatcgccgtggagcaagacaagaacacccaagaggtgttcgcccaagtgaagcagatctacaagaccccccccatcaagtacttcggcggcttcaacttcagccaaatcctgcccgaccctagcaagcctagcaagcggagcttcatcgaggacctgctgttcaacaaggtgaccctggccgacgccggcttcatcaagcagtacggcgactgcctaggcgacatcgcagctagagacctgatctgcgctcagaagttcaatggactcaccgtgctcccccccctgctgaccgacgagatgatcgctcagtacacctctgccctgctggcgggaaccataacaagcggttggacatttggcgccggggccgcactgcaaatccccttcgccatgcagatggcctacagattcaacggcatcggcgtgacacagaacgtgctgtacgagaatcagaagctgatcgccaatcagttcaacagcgccatcggcaagatccaagacagcctgagcagcaccgctagcgccctgggcaagctgcaagacgtggtgaatcacaacgcccaagccctgaacaccctggtgaagcagctgagcagcaagttcggcgccatcagcagcgtattgaatgacatcctgtctagactggacccccccgaggccgaggtgcagatcgacagactgatcaccggcagactgcagagcctgcagacctacgtgacacagcagctgatcagagccgccgagatcagagctagcgccaacctggccgccaccaagatgagcgagtgcgtgctggggcagagcaagagagtggacttctgcggcaagggctaccacctgatgagcttccctcagagcgccccccacggcgtggtgttcctgcacgtgacctacgtgcccgcccaagagaagaacttcaccaccgctcccgccatctgccacgacggcaaggcccacttccctagagagggcgtgttcgtgagcaacggcacccactggttcgtgacacagagaaacttctacgagcctcagatcatcaccaccgacaacaccttcgtgagcggcaactgcgacgtggtgatcggcatagtgaacaacaccgtatacgaccccctgcagcccgagctggacagcttcaaggaggagctggacaagtacttcaaaaaccatactagccccgacgtggacctgggagacatctctggcatcaacgctagcgtggtgaacattcagaaggagatcgaccggctgaatgaggtggccaagaacctgaacgagagcctgatcgacctgcaagagctgggcaagtacgagcagtacatcaagtggccctggtacatctggctgggcttcatcgccggcctgatcgccatcgtgatggtgaccatcatgctgtgctgcatgacaagctgttgcagctgcctgaaaggttgctgcagctgtggctcgtgctgcaagttcgacgaggacgacagcgagcccgtgctgaagggcgtgaagctgcactacacctgatgactcgaggctcgctttcttgctgtccaatttctattaaaggttcctttgttccctaagtccaactactaaactgggggatattatgaagggccttgagcatctggattctgcctaataaaaaacatttattttcattgcaaaaaaaaaaaaaaaaaaaaaaaaaaaaaaaaaaaaaaaaaaaaaaaaaaaaaaaaaaaaaaaaaaaaaaaaaaaaaaaaaaaaaaaaaaaaaaaaaaaaaaaaaaaaaaaaaaaaaaaaaa

SEQ ID NO: 109 - RNA, 4125 nt, synthetic construct
  source 1..4125: mol_type = other RNA; note = I'-BA4-B mRNA
gagttaggagttggtggcagtttcaataacaggtcattgccgagaaaaggatagcactataatatgttcgtgttcctggtgctgctgcccctggtgagctctcagtgcgtgaacctgatcacaagaacacagtcgtacaccaacagcttcacaagaggcgtgtactaccccgacaaggtgttcagaagcagcgtgctgcactccacccaagacctgtttctgcccttcttcagcaacgtgacctggttccacgccatcagcggcaccaacggcaccaagagattcgacaaccccgtgctgcccttcaacgacggcgtgtacttcgctagcaccgaaaagagcaacatcatcagaggctggatcttcggcaccaccctagactccaagacacaaagcctgctgatcgttaacaacgcgaccaacgtggtgatcaaggtgtgcgagtttcagttctgcaacgaccccttcctggacgtgtactaccacaagaacaacaagagctggatggagagcgagttcagagtctacagcagcgccaacaactgcaccttcgagtacgtgtctcagcccttcctgatggacctggagggcaagcaaggcaatttcaagaacctaagagagttcgtgttcaagaacatcgacggctacttcaagatctacagcaagcacacccccatcaacctggggagagacctgccccaaggcttcagcgccctggagcccctggtggacctgcccatcggcatcaacatcacaagatttcagaccctgctggccctgcaccgtagctacctaacccccggcgatagttcctctggctggacggccggcgctgccgcctactacgtgggctacctgcagcctagaaccttcctgctgaagtacaacgagaacggcactatcactgatgccgtggactgtgccctggaccccctgagcgagaccaagtgcaccctcaagagcttcaccgtggagaagggcatctatcagacaagcaacttcagagtgcagcccaccgagagcatcgtgagattccccaacatcaccaacctgtgccccttcgacgaggtgttcaacgccacaagattcgctagcgtgtacgcgtggaacagaaagagaatcagcaactgcgtggccgactacagcgtgctgtacaacttcgctcccttcttcgccttcaagtgctatggcgtcagccccaccaagctgaacgacctgtgcttcaccaacgtgtacgccgacagcttcgtgatcagaggcaacgaggtgagccagattgcccccgggcaaaccggcaacatcgccgactacaactacaagctgcccgacgacttcaccggctgcgtgatcgcgtggaacagcaataagctggattccaaggtgggcggcaactacaactaccggtacagactgttcagaaagagcaacctgaagcccttcgagagagacatcagcaccgagatctaccaagccggcaacaagccctgcaacggcgtggcgggcgtcaactgctacttccccctgcagagctacggctttaggcccacctacggcgtgggccatcagccctacagagtggtggtgctgagcttcgagctgctgcacgcccccgcaaccgtgtgcggccccaaaaagagcaccaacctggtgaagaacaagtgcgtgaacttcaactttaatggccttaagggcacgggcgtgctgaccgagagcaacaagaagttcctgccatttcagcaattcggcagagacatcgccgacaccaccgacgcggtcagagaccctcagaccctggagatcctggacatcaccccctgtagcttcggcggcgtgagcgtgatcacccccggcactaacacaagcaaccaagtggccgtgctgtaccaaggcgtgaactgcaccgaggtgcccgtggccatccacgccgatcagctgacccccacctggagagtatacagcaccggaagcaacgtgtttcagacaagagccggctgcctgatcggcgccgagtacgtgaacaacagctacgagtgcgacatccccatcggcgccggcatctgcgctagctatcagacacagaccaagagccaccggagagctagaagcgtggcttctcagagcatcatcgcctacaccatgagcctgggcgccgagaacagcgtggcctacagcaacaacagcatcgccatccccaccaacttcaccatcagcgtgaccaccgagatcctgcccgtaagtatgaccaagacaagcgtggactgcaccatgtacatctgcggcgacagcaccgagtgcagcaacctgctgctgcagtacggcagcttctgcacacagctgaagagagccctgaccggcatcgccgtggagcaagacaagaacacccaagaggtgttcgcccaagtgaagcagatctacaagaccccccccatcaagtacttcggcggcttcaacttcagccaaatcctgcccgaccctagcaagcctagcaagcggagcttcatcgaggacctgctgttcaacaaggtgaccctggccgacgccggcttcatcaagcagtacggcgactgcctaggcgacatcgcagctagagacctgatctgcgctcagaagttcaatggactcaccgtgctcccccccctgctgaccgacgagatgatcgctcagtacacctctgccctgctggcgggaaccataacaagcggttggacatttggcgccggggccgcactgcaaatccccttcgccatgcagatggcctacagattcaacggcatcggcgtgacacagaacgtgctgtacgagaatcagaagctgatcgccaatcagttcaacagcgccatcggcaagatccaagacagcctgagcagcaccgctagcgccctgggcaagctgcaagacgtggtgaatcacaacgcccaagccctgaacaccctggtgaagcagctgagcagcaagttcggcgccatcagcagcgtattgaatgacatcctgtctagactggacccccccgaggccgaggtgcagatcgacagactgatcaccggcagactgcagagcctgcagacctacgtgacacagcagctgatcagagccgccgagatcagagctagcgccaacctggccgccaccaagatgagcgagtgcgtgctggggcagagcaagagagtggacttctgcggcaagggctaccacctgatgagcttccctcagagcgccccccacggcgtggtgttcctgcacgtgacctacgtgcccgcccaagagaagaacttcaccaccgctcccgccatctgccacgacggcaaggcccacttccctagagagggcgtgttcgtgagcaacggcacccactggttcgtgacacagagaaacttctacgagcctcagatcatcaccaccgacaacaccttcgtgagcggcaactgcgacgtggtgatcggcatagtgaacaacaccgtatacgaccccctgcagcccgagctggacagcttcaaggaggagctggacaagtacttcaaaaaccatactagccccgacgtggacctgggagacatctctggcatcaacgctagcgtggtgaacattcagaaggagatcgaccggctgaatgaggtggccaagaacctgaacgagagcctgatcgacctgcaagagctgggcaagtacgagcagtacatcaagtggccctggtacatctggctgggcttcatcgccggcctgatcgccatcgtgatggtgaccatcatgctgtgctgcatgacaagctgttgcagctgcctgaaaggttgctgcagctgtggctcgtgctgcaagttcgacgaggacgacagcgagcccgtgctgaagggcgtgaagctgcactacacctgatgactcgaggctcgctttcttgctgtccaatttctattaaaggttcctttgttccctaagtccaactactaaactgggggatattatgaagggccttgagcatctggattctgcctaataaaaaacatttattttcattgcaaaaaaaaaaaaaaaaaaaaaaaaaaaaaaaagcatatgactaaaaaaaaaaaaaaaaaaaaaaaaaaaaaaaaaaaaaaaaaaaaaaaaaaaaaaaaaaaaaaaaaaaaaaaa

SEQ ID NO: 110 - RNA, 2019 nt, synthetic construct
  source 1..2019: mol_type = other RNA; note = I'-H1N1-B mRNA
gagttaggagttggtggcagtttcaataacaggtcattgccgagaaaaggatagcactataatatgaaggccatcctggtggtgatgctgtacaccttcaccaccgccaacgccgacaccctgtgcatcggctaccacgccaacaacagcaccgacaccgtggacaccgtgctggagaagaacgtgaccgtgacccacagcgtgaacctgctggaggacaagcacaacggcaagctgtgcaagctgcggggcgtggcccccctgcacctgggcaagtgcaacatcgccggctggatcctgggcaaccccgagtgcgagtccctgagcaccgcccgctcctggagctacatcgtggagacctccaacagcgacaacggcacctgctaccccggggacttcatcaactacgaggagctgcgggagcagctgtccagcgtgtccagcttcgagcgcttcgagatcttccccaagacctccagctggcccaaccacgactccgacaacggcgtgaccgccgcctgcccccacgccggggccaagagcttctacaagaacctgatctggctggtgaagaagggcaagtcctaccccaagatcaaccagacctacatcaacgacaaggggaaggaggtcctcgtgctgtggggcatccaccacccccccaccatcgccgaccagcagagcctctaccagaacgccgacgcctacgtcttcgtggggacctcccggtacagcaagaagttcaagcccgagatcgccacccgccccaaggtccgggaccaggagggccgcatgaactactactggaccctggtggagccgggggacaagatcaccttcgaggccaccggcaacctcgtcgccccgcggtacgccttcacgatggagcgcgacgccgggtccggcatcatcatcagcgacacccccgtgcacgactgcaacacgacctgccagacgcccgagggggcgatcaacacctccctgccgttccagaacgtccacccgatcacgatcggcaagtgccccaagtacgtgaagtccaccaagctccggctggccacggggctccgcaacgtcccctccatccagagccggggcctgttcggggcgatcgccggcttcatcgaggggggctggaccgggatggtggacggctggtacgggtaccaccaccagaacgagcagggctccgggtacgcggccgacctcaagtcgacgcagaacgcgatcgacaagatcaccaacaaggtcaacagcgtgatcgagaagatgaacacgcagttcaccgccgtcggcaaggagttcaaccacctggagaagcgcatcgagaacctcaacaagaaggtggacgacgggttcctggacatctggacgtacaacgcggagctcctggtcctcctggagaacgagcggaccctcgactaccacgactccaacgtgaagaacctgtacgagaaggtccgcaaccagctcaagaacaacgccaaggagatcggcaacgggtgcttcgagttctaccacaagtgcgacaacacgtgcatggagtcggtgaagaacggcacctacgactacccgaagtacagcgaggaggcgaagctgaaccgggagaagatcgacggggtcaagctcgactccacgcgcatctaccagatcctggccatctactcgaccgtggcgagctccctcgtcctggtggtctcgctcggcgccatcagcttctggatgtgctccaacgggtcgctgcagtgccggatctgcatctgatgactcgaggctcgctttcttgctgtccaatttctattaaaggttcctttgttccctaagtccaactactaaactgggggatattatgaagggccttgagcatctggattctgcctaataaaaaacatttattttcattgcaaaaaaaaaaaaaaaaaaaaaaaaaaaaaaaagcatatgactaaaaaaaaaaaaaaaaaaaaaaaaaaaaaaaaaaaaaaaaaaaaaaaaaaaaaaaaaaaaaaaaaaaaaaaa

SEQ ID NO: 111 - RNA, 2019 nt, synthetic construct
  source 1..2019: mol_type = other RNA; note = I'-H3N2-B mRNA
gagttaggagttggtggcagtttcaataacaggtcattgccgagaaaaggatagcactataatatgaagaccatcatcgccctgagctacatcctgtgcctggtgttcgcccagaagatccccggcaacgacaacagcaccgccaccctgtgcctgggccaccacgccgtgcccaacggcaccatcgtgaagaccatcaccaacgaccggatcgaggtgaccaacgccaccgagctggtgcagaactccagcatcggcgagatctgcgactccccccaccagatcctggacggcggcaactgcaccctgatcgacgccctgctgggcgacccccagtgcgacgggttccagaacaaggagtgggacctgttcgtggagcggagccgcgccaactccaactgctacccctacgacgtgcccgactacgccagcctgcggtccctggtggccagctccggcaccctggagttcaagaacgagagcttcaactggaccggggtcaagcagaacggcacctccagcgcctgcatccgcgggtccagctccagcttcttctcccggctgaactggctcacccacctgaactacacctaccccgccctcaacgtgaccatgcccaacaacgagcagttcgacaagctgtacatctggggcgtccaccaccccagcaccgacaaggaccagatctccctcttcgcccagcccagcgggcgcatcaccgtgtccacgaagcggagccagcaggccgtcatccccaacatcggctcccgcccgcggatccgcgacatccccagccggatctccatctactggacgatcgtgaagccgggggacatcctgctcatcaacagcaccggcaacctgatcgccccccgcgggtacttcaagatccggtccggcaagagctcgatcatgcgctccgacgccccgatcgggaagtgcaagagcgagtgcatcacccccaacggctcgatcccgaacgacaagcccttccagaacgtcaaccggatcacgtacggggcctgcccgcgctacgtgaagcagtccacgctcaagctggccaccggcatgcggaacgtccccgagaagcagacccgcgggatcttcggcgccatcgcggggttcatcgagaacggctgggaggggatggtggacggctggtacgggttccggcaccagaacagcgagggccgcgggcaggccgcggacctcaagtcgacgcaggccgcgatcgaccagatcaacggcaagctgaaccggctcatcgggaagacgaacgagaagttccaccagatcgagaaggagttctccgaggtcgagggccgcgtgcaggacctggagaagtacgtcgaggacaccaagatcgacctctggagctacaacgccgagctgctcgtggcgctggagaaccagcacaccatcgacctcacggactcggagatgaacaagctgttcgagaagacgaagaagcagctccgggagaacgccgaggacatggggaacggctgcttcaagatctaccacaagtgcgacaacgcgtgcatcgggtccatccgcaacgagacctacgaccacaacgtctaccgggacgaggccctgaacaaccgcttccagatcaagggcgtggagctcaagagcgggtacaaggactggatcctgtggatctcgttcgcgatgtcctgcttcctcctgtgcatcgccctcctgggcttcatcatgtgggcgtgccagaaggggaacatccggtgcaacatctgcatctgatgactcgaggctcgctttcttgctgtccaatttctattaaaggttcctttgttccctaagtccaactactaaactgggggatattatgaagggccttgagcatctggattctgcctaataaaaaacatttattttcattgcaaaaaaaaaaaaaaaaaaaaaaaaaaaaaaaagcatatgactaaaaaaaaaaaaaaaaaaaaaaaaaaaaaaaaaaaaaaaaaaaaaaaaaaaaaaaaaaaaaaaaaaaaaaaa

SEQ ID NO: 112 - RNA, 2067 nt, synthetic construct
  source 1..2067: mol_type = other RNA; note = I'-B-Victoria-B mRNA
gagttaggagttggtggcagtttcaataacaggtcattgccgagaaaaggatagcactataatatgaaggccatcatcgtgctgctgatggtggtgaccagcaacgccgaccggatctgcaccggcatcaccagctccaacagcccccacgtggtgaagaccgccacccagggcgaggtgaacgtgaccggcgtgatccccctgaccaccacccccaccaagtcccacttcgccaacctgaagggcaccgagacccggggcaagctgtgccccaagtgcctgaactgcaccgacctggacgtggccctgggccgccccaagtgcaccggcaagatccccagcgcccgggtgtccatcctgcacgaggtgcgccccgtgaccagcggctgcttccccatcatgcacgaccgcaccaagatccggcagctgcccaacctgctgcgggggtacgagcacgtccgcctgtccacccacaacgtgatcaacgccgaggacgcccccggccggccctacgagatcgggaccagcggctcctgccccaacatcaccaacgggaacggcttcttcgccaccatggcctgggccgtccccaagaacaagaccgccaccaaccccctgaccatcgaggtgccgtacatctgcaccgagggggaggaccagatcaccgtctggggcttccacagcgacaacgagacgcagatggccaagctgtacggggactccaagccccagaagttcacgagctccgccaacggcgtgaccacccactacgtcagccagatcgggggcttcccgaaccagacggaggacgggggcctgccccagtccgggcgcatcgtggtcgactacatggtgcagaagtccggcaagacggggaccatcacgtaccagcggggcatcctgctgccgcagaaggtctggtgcgcctccgggcgcagcaaggtgatcaagggctccctgcccctcatcggggaggccgactgcctgcacgagaagtacggcgggctcaacaagagcaagccgtactacaccggcgagcacgccaaggccatcgggaactgccccatctgggtcaagaccccgctgaagctcgccaacggcacgaagtaccggcccccggccaagctgctcaaggagcgcgggttcttcggcgccatcgccgggttcctggagggcgggtgggagggcatgatcgccgggtggcacggctacacgtcccacggggcccacggcgtggcggtcgccgcggacctcaagagcacccaggaggccatcaacaagatcacgaagaacctgaactccctcagcgagctggaggtgaagaacctccagcgcctgtccggggcgatggacgagctccacaacgagatcctggagctcgacgagaaggtcgacgacctgcgggccgacaccatcagctcgcagatcgagctcgcggtgctgctctccaacgagggcatcatcaacagcgaggacgagcacctgctcgccctggagcggaagctcaagaagatgctggggccctcggcggtcgagatcggcaacgggtgcttcgagaccaagcacaagtgcaaccagacgtgcctcgaccgcatcgccgcgggcacgttcgacgccggggagttctccctgccgaccttcgacagcctcaacatcacggcggcctcgctgaacgacgacggcctcgacaaccacaccatcctgctctactactccaccgcggccagctcgctggcggtgacgctcatgatcgccatcttcgtcgtgtacatggtctcccgcgacaacgtgagctgctcgatctgcctgtgatgactcgaggctcgctttcttgctgtccaatttctattaaaggttcctttgttccctaagtccaactactaaactgggggatattatgaagggccttgagcatctggattctgcctaataaaaaacatttattttcattgcaaaaaaaaaaaaaaaaaaaaaaaaaaaaaaaagcatatgactaaaaaaaaaaaaaaaaaaaaaaaaaaaaaaaaaaaaaaaaaaaaaaaaaaaaaaaaaaaaaaaaaaaaaaaa

SEQ ID NO: 113 - RNA, 2073 nt, synthetic construct
  source 1..2073: mol_type = other RNA; note = I'-B-Yamagata-B mRNA
gagttaggagttggtggcagtttcaataacaggtcattgccgagaaaaggatagcactataatatgaaggccatcatcgtgctgctgatggtggtgaccagcaacgccgaccggatctgcaccggcatcaccagctccaacagcccccacgtggtgaagaccgccacccagggcgaggtgaacgtgaccggcgtgatccccctgaccaccacccccaccaagtcctacttcgccaacctgaagggcacccggacccgcggcaagctgtgccccgactgcctgaactgcaccgacctggacgtggccctgggccggcccatgtgcgtgggcaccacccccagcgccaaggcctccatcctgcacgaggtgcgccccgtgaccagcggctgcttccccatcatgcacgaccgcaccaagatccggcagctgcccaacctgctgcgggggtacgagaagatccgcctgtccacccagaacgtcatcgacgccgagaaggcccccggcgggccctaccggctgggcaccagcgggtcctgccccaacgccaccagcaagatcggcttcttcgccaccatggcctgggccgtgcccaaggacaactacaagaacgccaccaaccccctgaccgtcgaggtgccctacatctgcaccgagggggaggaccagatcacggtctggggcttccactccgacaacaagacccagatgaagtccctgtacggggactccaacccgcagaagttcacgagctccgccaacggcgtgaccacgcactacgtcagccagatcggggacttcccggaccagaccgaggacggcgggctgccccagtccggccgcatcgtggtcgactacatgatgcagaagcccgggaagacgggcaccatcgtgtaccagcggggggtcctgctgccgcagaaggtgtggtgcgccagcggccgctccaaggtcatcaaggggagcctgcccctcatcggcgaggccgactgcctgcacgaggagtacgggggcctcaacaagtccaagccgtactacacggggaagcacgccaaggccatcggcaactgcccgatctgggtgaagacccccctgaagctcgccaacgggacgaagtaccggccgcccgccaagctgctcaaggagcgcggcttcttcggggccatcgccggcttcctggaggggggctgggaggggatgatcgccggctggcacgggtacaccagccacggcgcccacggggtcgcggtggccgcggacctcaagtccacgcaggaggccatcaacaagatcaccaagaacctgaacagcctctccgagctggaggtcaagaacctccagcgcctgagcggcgcgatggacgagctccacaacgagatcctggagctcgacgagaaggtggacgacctgcgggccgacacgatctcgtcccagatcgagctcgcggtcctgctcagcaacgaggggatcatcaactcggaggacgagcacctgctcgccctggagcggaagctcaagaagatgctgggcccgtccgcggtggacatcgggaacggctgcttcgagaccaagcacaagtgcaaccagacgtgcctcgaccgcatcgccgcggggaccttcaacgccggcgagttcagcctgcccacgttcgactcgctcaacatcaccgcggcctccctgaacgacgacgggctcgacaaccacacgatcctgctctactacagcaccgcggcctcgtccctggcggtcacgctcatgctggccatcttcatcgtgtacatggtcagccgcgacaacgtgtcgtgctccatctgcctctgatgactcgaggctcgctttcttgctgtccaatttctattaaaggttcctttgttccctaagtccaactactaaactgggggatattatgaagggccttgagcatctggattctgcctaataaaaaacatttattttcattgcaaaaaaaaaaaaaaaaaaaaaaaaaaaaaaaagcatatgactaaaaaaaaaaaaaaaaaaaaaaaaaaaaaaaaaaaaaaaaaaaaaaaaaaaaaaaaaaaaaaaaaaaaaaaa

SEQ ID NO: 114 - RNA, 2019 nt, synthetic construct
  source 1..2019: mol_type = other RNA; note = I'-H1N1-HA0-mut-B mRNA
gagttaggagttggtggcagtttcaataacaggtcattgccgagaaaaggatagcactataatatgaaggccatcctggtggtgatgctgtacaccttcaccaccgccaacgccgacaccctgtgcatcggctaccacgccaacaacagcaccgacaccgtggacaccgtgctggagaagaacgtgaccgtgacccacagcgtgaacctgctggaggacaagcacaacggcaagctgtgcaagctgcggggcgtggcccccctgcacctgggcaagtgcaacatcgccggctggatcctgggcaaccccgagtgcgagtccctgagcaccgcccgctcctggagctacatcgtggagacctccaacagcgacaacggcacctgctaccccggggacttcatcaactacgaggagctgcgggagcagctgtccagcgtgtccagcttcgagcgcttcgagatcttccccaagacctccagctggcccaaccacgactccgacaacggcgtgaccgccgcctgcccccacgccggggccaagagcttctacaagaacctgatctggctggtgaagaagggcaagtcctaccccaagatcaaccagacctacatcaacgacaaggggaaggaggtcctcgtgctgtggggcatccaccacccccccaccatcgccgaccagcagagcctctaccagaacgccgacgcctacgtcttcgtggggacctcccggtacagcaagaagttcaagcccgagatcgccacccgccccaaggtccgggaccaggagggccgcatgaactactactggaccctggtggagccgggggacaagatcaccttcgaggccaccggcaacctcgtcgccccgcggtacgccttcacgatggagcgcgacgccgggtccggcatcatcatcagcgacacccccgtgcacgactgcaacacgacctgccagacgcccgagggggcgatcaacacctccctgccgttccagaacgtccacccgatcacgatcggcaagtgccccaagtacgtgaagtccaccaagctccggctggccacggggctccgcaacgtcccctccatccagagccagggcctgttcggggcgatcgccggcttcatcgaggggggctggaccgggatggtggacggctggtacgggtaccaccaccagaacgagcagggctccgggtacgcggccgacctcaagtcgacgcagaacgcgatcgacaagatcaccaacaaggtcaacagcgtgatcgagaagatgaacacgcagttcaccgccgtcggcaaggagttcaaccacctggagaagcgcatcgagaacctcaacaagaaggtggacgacgggttcctggacatctggacgtacaacgcggagctcctggtcctcctggagaacgagcggaccctcgactaccacgactccaacgtgaagaacctgtacgagaaggtccgcaaccagctcaagaacaacgccaaggagatcggcaacgggtgcttcgagttctaccacaagtgcgacaacacgtgcatggagtcggtgaagaacggcacctacgactacccgaagtacagcgaggaggcgaagctgaaccgggagaagatcgacggggtcaagctcgactccacgcgcatctaccagatcctggccatctactcgaccgtggcgagctccctcgtcctggtggtctcgctcggcgccatcagcttctggatgtgctccaacgggtcgctgcagtgccggatctgcatctgatgactcgaggctcgctttcttgctgtccaatttctattaaaggttcctttgttccctaagtccaactactaaactgggggatattatgaagggccttgagcatctggattctgcctaataaaaaacatttattttcattgcaaaaaaaaaaaaaaaaaaaaaaaaaaaaaaaagcatatgactaaaaaaaaaaaaaaaaaaaaaaaaaaaaaaaaaaaaaaaaaaaaaaaaaaaaaaaaaaaaaaaaaaaaaaaa

SEQ ID NO: 115 - RNA, 2019 nt, synthetic construct
  source 1..2019: mol_type = other RNA; note = I'-H3N2-HA0-mut-B mRNA
gagttaggagttggtggcagtttcaataacaggtcattgccgagaaaaggatagcactataatatgaagaccatcatcgccctgagctacatcctgtgcctggtgttcgcccagaagatccccggcaacgacaacagcaccgccaccctgtgcctgggccaccacgccgtgcccaacggcaccatcgtgaagaccatcaccaacgaccggatcgaggtgaccaacgccaccgagctggtgcagaactccagcatcggcgagatctgcgactccccccaccagatcctggacggcggcaactgcaccctgatcgacgccctgctgggcgacccccagtgcgacgggttccagaacaaggagtgggacctgttcgtggagcggagccgcgccaactccaactgctacccctacgacgtgcccgactacgccagcctgcggtccctggtggccagctccggcaccctggagttcaagaacgagagcttcaactggaccggggtcaagcagaacggcacctccagcgcctgcatccgcgggtccagctccagcttcttctcccggctgaactggctcacccacctgaactacacctaccccgccctcaacgtgaccatgcccaacaacgagcagttcgacaagctgtacatctggggcgtccaccaccccagcaccgacaaggaccagatctccctcttcgcccagcccagcgggcgcatcaccgtgtccacgaagcggagccagcaggccgtcatccccaacatcggctcccgcccgcggatccgcgacatccccagccggatctccatctactggacgatcgtgaagccgggggacatcctgctcatcaacagcaccggcaacctgatcgccccccgcgggtacttcaagatccggtccggcaagagctcgatcatgcgctccgacgccccgatcgggaagtgcaagagcgagtgcatcacccccaacggctcgatcccgaacgacaagcccttccagaacgtcaaccggatcacgtacggggcctgcccgcgctacgtgaagcagtccacgctcaagctggccaccggcatgcggaacgtccccgagaagcagacccaggggatcttcggcgccatcgcggggttcatcgagaacggctgggaggggatggtggacggctggtacgggttccggcaccagaacagcgagggccgcgggcaggccgcggacctcaagtcgacgcaggccgcgatcgaccagatcaacggcaagctgaaccggctcatcgggaagacgaacgagaagttccaccagatcgagaaggagttctccgaggtcgagggccgcgtgcaggacctggagaagtacgtcgaggacaccaagatcgacctctggagctacaacgccgagctgctcgtggcgctggagaaccagcacaccatcgacctcacggactcggagatgaacaagctgttcgagaagacgaagaagcagctccgggagaacgccgaggacatggggaacggctgcttcaagatctaccacaagtgcgacaacgcgtgcatcgggtccatccgcaacgagacctacgaccacaacgtctaccgggacgaggccctgaacaaccgcttccagatcaagggcgtggagctcaagagcgggtacaaggactggatcctgtggatctcgttcgcgatgtcctgcttcctcctgtgcatcgccctcctgggcttcatcatgtgggcgtgccagaaggggaacatccggtgcaacatctgcatctgatgactcgaggctcgctttcttgctgtccaatttctattaaaggttcctttgttccctaagtccaactactaaactgggggatattatgaagggccttgagcatctggattctgcctaataaaaaacatttattttcattgcaaaaaaaaaaaaaaaaaaaaaaaaaaaaaaaagcatatgactaaaaaaaaaaaaaaaaaaaaaaaaaaaaaaaaaaaaaaaaaaaaaaaaaaaaaaaaaaaaaaaaaaaaaaaa

SEQ ID NO: 116 - RNA, 2067 nt, synthetic construct
  source 1..2067: mol_type = other RNA; note = I'-B-Victoria-HA0-mut-B mRNA
gagttaggagttggtggcagtttcaataacaggtcattgccgagaaaaggatagcactataatatgaaggccatcatcgtgctgctgatggtggtgaccagcaacgccgaccggatctgcaccggcatcaccagctccaacagcccccacgtggtgaagaccgccacccagggcgaggtgaacgtgaccggcgtgatccccctgaccaccacccccaccaagtcccacttcgccaacctgaagggcaccgagacccggggcaagctgtgccccaagtgcctgaactgcaccgacctggacgtggccctgggccgccccaagtgcaccggcaagatccccagcgcccgggtgtccatcctgcacgaggtgcgccccgtgaccagcggctgcttccccatcatgcacgaccgcaccaagatccggcagctgcccaacctgctgcgggggtacgagcacgtccgcctgtccacccacaacgtgatcaacgccgaggacgcccccggccggccctacgagatcgggaccagcggctcctgccccaacatcaccaacgggaacggcttcttcgccaccatggcctgggccgtccccaagaacaagaccgccaccaaccccctgaccatcgaggtgccgtacatctgcaccgagggggaggaccagatcaccgtctggggcttccacagcgacaacgagacgcagatggccaagctgtacggggactccaagccccagaagttcacgagctccgccaacggcgtgaccacccactacgtcagccagatcgggggcttcccgaaccagacggaggacgggggcctgccccagtccgggcgcatcgtggtcgactacatggtgcagaagtccggcaagacggggaccatcacgtaccagcggggcatcctgctgccgcagaaggtctggtgcgcctccgggcgcagcaaggtgatcaagggctccctgcccctcatcggggaggccgactgcctgcacgagaagtacggcgggctcaacaagagcaagccgtactacaccggcgagcacgccaaggccatcgggaactgccccatctgggtcaagaccccgctgaagctcgccaacggcacgaagtaccggcccccggccaagctgctcaaggagcaggggttcttcggcgccatcgccgggttcctggagggcgggtgggagggcatgatcgccgggtggcacggctacacgtcccacggggcccacggcgtggcggtcgccgcggacctcaagagcacccaggaggccatcaacaagatcacgaagaacctgaactccctcagcgagctggaggtgaagaacctccagcgcctgtccggggcgatggacgagctccacaacgagatcctggagctcgacgagaaggtcgacgacctgcgggccgacaccatcagctcgcagatcgagctcgcggtgctgctctccaacgagggcatcatcaacagcgaggacgagcacctgctcgccctggagcggaagctcaagaagatgctggggccctcggcggtcgagatcggcaacgggtgcttcgagaccaagcacaagtgcaaccagacgtgcctcgaccgcatcgccgcgggcacgttcgacgccggggagttctccctgccgaccttcgacagcctcaacatcacggcggcctcgctgaacgacgacggcctcgacaaccacaccatcctgctctactactccaccgcggccagctcgctggcggtgacgctcatgatcgccatcttcgtcgtgtacatggtctcccgcgacaacgtgagctgctcgatctgcctgtgatgactcgaggctcgctttcttgctgtccaatttctattaaaggttcctttgttccctaagtccaactactaaactgggggatattatgaagggccttgagcatctggattctgcctaataaaaaacatttattttcattgcaaaaaaaaaaaaaaaaaaaaaaaaaaaaaaaagcatatgactaaaaaaaaaaaaaaaaaaaaaaaaaaaaaaaaaaaaaaaaaaaaaaaaaaaaaaaaaaaaaaaaaaaaaaaa

SEQ ID NO: 117 - RNA, 2073 nt, synthetic construct
  source 1..2073: mol_type = other RNA; note = I'-B-Yamagata-HA0-mut-B mRNA
gagttaggagttggtggcagtttcaataacaggtcattgccgagaaaaggatagcactataatatgaaggccatcatcgtgctgctgatggtggtgaccagcaacgccgaccggatctgcaccggcatcaccagctccaacagcccccacgtggtgaagaccgccacccagggcgaggtgaacgtgaccggcgtgatccccctgaccaccacccccaccaagtcctacttcgccaacctgaagggcacccggacccgcggcaagctgtgccccgactgcctgaactgcaccgacctggacgtggccctgggccggcccatgtgcgtgggcaccacccccagcgccaaggcctccatcctgcacgaggtgcgccccgtgaccagcggctgcttccccatcatgcacgaccgcaccaagatccggcagctgcccaacctgctgcgggggtacgagaagatccgcctgtccacccagaacgtcatcgacgccgagaaggcccccggcgggccctaccggctgggcaccagcgggtcctgccccaacgccaccagcaagatcggcttcttcgccaccatggcctgggccgtgcccaaggacaactacaagaacgccaccaaccccctgaccgtcgaggtgccctacatctgcaccgagggggaggaccagatcacggtctggggcttccactccgacaacaagacccagatgaagtccctgtacggggactccaacccgcagaagttcacgagctccgccaacggcgtgaccacgcactacgtcagccagatcggggacttcccggaccagaccgaggacggcgggctgccccagtccggccgcatcgtggtcgactacatgatgcagaagcccgggaagacgggcaccatcgtgtaccagcggggggtcctgctgccgcagaaggtgtggtgcgccagcggccgctccaaggtcatcaaggggagcctgcccctcatcggcgaggccgactgcctgcacgaggagtacgggggcctcaacaagtccaagccgtactacacggggaagcacgccaaggccatcggcaactgcccgatctgggtgaagacccccctgaagctcgccaacgggacgaagtaccggccgcccgccaagctgctcaaggagcagggcttcttcggggccatcgccggcttcctggaggggggctgggaggggatgatcgccggctggcacgggtacaccagccacggcgcccacggggtcgcggtggccgcggacctcaagtccacgcaggaggccatcaacaagatcaccaagaacctgaacagcctctccgagctggaggtcaagaacctccagcgcctgagcggcgcgatggacgagctccacaacgagatcctggagctcgacgagaaggtggacgacctgcgggccgacacgatctcgtcccagatcgagctcgcggtcctgctcagcaacgaggggatcatcaactcggaggacgagcacctgctcgccctggagcggaagctcaagaagatgctgggcccgtccgcggtggacatcgggaacggctgcttcgagaccaagcacaagtgcaaccagacgtgcctcgaccgcatcgccgcggggaccttcaacgccggcgagttcagcctgcccacgttcgactcgctcaacatcaccgcggcctccctgaacgacgacgggctcgacaaccacacgatcctgctctactacagcaccgcggcctcgtccctggcggtcacgctcatgctggccatcttcatcgtgtacatggtcagccgcgacaacgtgtcgtgctccatctgcctctgatgactcgaggctcgctttcttgctgtccaatttctattaaaggttcctttgttccctaagtccaactactaaactgggggatattatgaagggccttgagcatctggattctgcctaataaaaaacatttattttcattgcaaaaaaaaaaaaaaaaaaaaaaaaaaaaaaaagcatatgactaaaaaaaaaaaaaaaaaaaaaaaaaaaaaaaaaaaaaaaaaaaaaaaaaaaaaaaaaaaaaaaaaaaaaaaa

SEQ ID NO: 118 - RNA, 2027 nt, synthetic construct
  source 1..2027: mol_type = other RNA; note = I'-H1N1-B-120A mRNA
gagttaggagttggtggcagtttcaataacaggtcattgccgagaaaaggatagcactataatatgaaggccatcctggtggtgatgctgtacaccttcaccaccgccaacgccgacaccctgtgcatcggctaccacgccaacaacagcaccgacaccgtggacaccgtgctggagaagaacgtgaccgtgacccacagcgtgaacctgctggaggacaagcacaacggcaagctgtgcaagctgcggggcgtggcccccctgcacctgggcaagtgcaacatcgccggctggatcctgggcaaccccgagtgcgagtccctgagcaccgcccgctcctggagctacatcgtggagacctccaacagcgacaacggcacctgctaccccggggacttcatcaactacgaggagctgcgggagcagctgtccagcgtgtccagcttcgagcgcttcgagatcttccccaagacctccagctggcccaaccacgactccgacaacggcgtgaccgccgcctgcccccacgccggggccaagagcttctacaagaacctgatctggctggtgaagaagggcaagtcctaccccaagatcaaccagacctacatcaacgacaaggggaaggaggtcctcgtgctgtggggcatccaccacccccccaccatcgccgaccagcagagcctctaccagaacgccgacgcctacgtcttcgtggggacctcccggtacagcaagaagttcaagcccgagatcgccacccgccccaaggtccgggaccaggagggccgcatgaactactactggaccctggtggagccgggggacaagatcaccttcgaggccaccggcaacctcgtcgccccgcggtacgccttcacgatggagcgcgacgccgggtccggcatcatcatcagcgacacccccgtgcacgactgcaacacgacctgccagacgcccgagggggcgatcaacacctccctgccgttccagaacgtccacccgatcacgatcggcaagtgccccaagtacgtgaagtccaccaagctccggctggccacggggctccgcaacgtcccctccatccagagccggggcctgttcggggcgatcgccggcttcatcgaggggggctggaccgggatggtggacggctggtacgggtaccaccaccagaacgagcagggctccgggtacgcggccgacctcaagtcgacgcagaacgcgatcgacaagatcaccaacaaggtcaacagcgtgatcgagaagatgaacacgcagttcaccgccgtcggcaaggagttcaaccacctggagaagcgcatcgagaacctcaacaagaaggtggacgacgggttcctggacatctggacgtacaacgcggagctcctggtcctcctggagaacgagcggaccctcgactaccacgactccaacgtgaagaacctgtacgagaaggtccgcaaccagctcaagaacaacgccaaggagatcggcaacgggtgcttcgagttctaccacaagtgcgacaacacgtgcatggagtcggtgaagaacggcacctacgactacccgaagtacagcgaggaggcgaagctgaaccgggagaagatcgacggggtcaagctcgactccacgcgcatctaccagatcctggccatctactcgaccgtggcgagctccctcgtcctggtggtctcgctcggcgccatcagcttctggatgtgctccaacgggtcgctgcagtgccggatctgcatctgatgactcgaggctcgctttcttgctgtccaatttctattaaaggttcctttgttccctaagtccaactactaaactgggggatattatgaagggccttgagcatctggattctgcctaataaaaaacatttattttcattgcaaaaaaaaaaaaaaaaaaaaaaaaaaaaaaaaaaaaaaaaaaaaaaaaaaaaaaaaaaaaaaaaaaaaaaaaaaaaaaaaaaaaaaaaaaaaaaaaaaaaaaaaaaaaaaaaaaaaaaaaaa

SEQ ID NO: 119 - RNA, 2027 nt, synthetic construct
  source 1..2027: mol_type = other RNA; note = I'-H3N2-B-120A mRNA
gagttaggagttggtggcagtttcaataacaggtcattgccgagaaaaggatagcactataatatgaagaccatcatcgccctgagctacatcctgtgcctggtgttcgcccagaagatccccggcaacgacaacagcaccgccaccctgtgcctgggccaccacgccgtgcccaacggcaccatcgtgaagaccatcaccaacgaccggatcgaggtgaccaacgccaccgagctggtgcagaactccagcatcggcgagatctgcgactccccccaccagatcctggacggcggcaactgcaccctgatcgacgccctgctgggcgacccccagtgcgacgggttccagaacaaggagtgggacctgttcgtggagcggagccgcgccaactccaactgctacccctacgacgtgcccgactacgccagcctgcggtccctggtggccagctccggcaccctggagttcaagaacgagagcttcaactggaccggggtcaagcagaacggcacctccagcgcctgcatccgcgggtccagctccagcttcttctcccggctgaactggctcacccacctgaactacacctaccccgccctcaacgtgaccatgcccaacaacgagcagttcgacaagctgtacatctggggcgtccaccaccccagcaccgacaaggaccagatctccctcttcgcccagcccagcgggcgcatcaccgtgtccacgaagcggagccagcaggccgtcatccccaacatcggctcccgcccgcggatccgcgacatccccagccggatctccatctactggacgatcgtgaagccgggggacatcctgctcatcaacagcaccggcaacctgatcgccccccgcgggtacttcaagatccggtccggcaagagctcgatcatgcgctccgacgccccgatcgggaagtgcaagagcgagtgcatcacccccaacggctcgatcccgaacgacaagcccttccagaacgtcaaccggatcacgtacggggcctgcccgcgctacgtgaagcagtccacgctcaagctggccaccggcatgcggaacgtccccgagaagcagacccgcgggatcttcggcgccatcgcggggttcatcgagaacggctgggaggggatggtggacggctggtacgggttccggcaccagaacagcgagggccgcgggcaggccgcggacctcaagtcgacgcaggccgcgatcgaccagatcaacggcaagctgaaccggctcatcgggaagacgaacgagaagttccaccagatcgagaaggagttctccgaggtcgagggccgcgtgcaggacctggagaagtacgtcgaggacaccaagatcgacctctggagctacaacgccgagctgctcgtggcgctggagaaccagcacaccatcgacctcacggactcggagatgaacaagctgttcgagaagacgaagaagcagctccgggagaacgccgaggacatggggaacggctgcttcaagatctaccacaagtgcgacaacgcgtgcatcgggtccatccgcaacgagacctacgaccacaacgtctaccgggacgaggccctgaacaaccgcttccagatcaagggcgtggagctcaagagcgggtacaaggactggatcctgtggatctcgttcgcgatgtcctgcttcctcctgtgcatcgccctcctgggcttcatcatgtgggcgtgccagaaggggaacatccggtgcaacatctgcatctgatgactcgaggctcgctttcttgctgtccaatttctattaaaggttcctttgttccctaagtccaactactaaactgggggatattatgaagggccttgagcatctggattctgcctaataaaaaacatttattttcattgcaaaaaaaaaaaaaaaaaaaaaaaaaaaaaaaaaaaaaaaaaaaaaaaaaaaaaaaaaaaaaaaaaaaaaaaaaaaaaaaaaaaaaaaaaaaaaaaaaaaaaaaaaaaaaaaaaaaaaaaaaa

SEQ ID NO: 120 - RNA, 2075 nt, synthetic construct
  source 1..2075: mol_type = other RNA; note = I'-B-Victoria-B-120A mRNA
gagttaggagttggtggcagtttcaataacaggtcattgccgagaaaaggatagcactataatatgaaggccatcatcgtgctgctgatggtggtgaccagcaacgccgaccggatctgcaccggcatcaccagctccaacagcccccacgtggtgaagaccgccacccagggcgaggtgaacgtgaccggcgtgatccccctgaccaccacccccaccaagtcccacttcgccaacctgaagggcaccgagacccggggcaagctgtgccccaagtgcctgaactgcaccgacctggacgtggccctgggccgccccaagtgcaccggcaagatccccagcgcccgggtgtccatcctgcacgaggtgcgccccgtgaccagcggctgcttccccatcatgcacgaccgcaccaagatccggcagctgcccaacctgctgcgggggtacgagcacgtccgcctgtccacccacaacgtgatcaacgccgaggacgcccccggccggccctacgagatcgggaccagcggctcctgccccaacatcaccaacgggaacggcttcttcgccaccatggcctgggccgtccccaagaacaagaccgccaccaaccccctgaccatcgaggtgccgtacatctgcaccgagggggaggaccagatcaccgtctggggcttccacagcgacaacgagacgcagatggccaagctgtacggggactccaagccccagaagttcacgagctccgccaacggcgtgaccacccactacgtcagccagatcgggggcttcccgaaccagacggaggacgggggcctgccccagtccgggcgcatcgtggtcgactacatggtgcagaagtccggcaagacggggaccatcacgtaccagcggggcatcctgctgccgcagaaggtctggtgcgcctccgggcgcagcaaggtgatcaagggctccctgcccctcatcggggaggccgactgcctgcacgagaagtacggcgggctcaacaagagcaagccgtactacaccggcgagcacgccaaggccatcgggaactgccccatctgggtcaagaccccgctgaagctcgccaacggcacgaagtaccggcccccggccaagctgctcaaggagcgcgggttcttcggcgccatcgccgggttcctggagggcgggtgggagggcatgatcgccgggtggcacggctacacgtcccacggggcccacggcgtggcggtcgccgcggacctcaagagcacccaggaggccatcaacaagatcacgaagaacctgaactccctcagcgagctggaggtgaagaacctccagcgcctgtccggggcgatggacgagctccacaacgagatcctggagctcgacgagaaggtcgacgacctgcgggccgacaccatcagctcgcagatcgagctcgcggtgctgctctccaacgagggcatcatcaacagcgaggacgagcacctgctcgccctggagcggaagctcaagaagatgctggggccctcggcggtcgagatcggcaacgggtgcttcgagaccaagcacaagtgcaaccagacgtgcctcgaccgcatcgccgcgggcacgttcgacgccggggagttctccctgccgaccttcgacagcctcaacatcacggcggcctcgctgaacgacgacggcctcgacaaccacaccatcctgctctactactccaccgcggccagctcgctggcggtgacgctcatgatcgccatcttcgtcgtgtacatggtctcccgcgacaacgtgagctgctcgatctgcctgtgatgactcgaggctcgctttcttgctgtccaatttctattaaaggttcctttgttccctaagtccaactactaaactgggggatattatgaagggccttgagcatctggattctgcctaataaaaaacatttattttcattgcaaaaaaaaaaaaaaaaaaaaaaaaaaaaaaaaaaaaaaaaaaaaaaaaaaaaaaaaaaaaaaaaaaaaaaaaaaaaaaaaaaaaaaaaaaaaaaaaaaaaaaaaaaaaaaaaaaaaaaaaaa

SEQ ID NO: 121 - RNA, 2081 nt, synthetic construct
  source 1..2081: mol_type = other RNA; note = I'-B-Yamagata-B-120A mRNA
gagttaggagttggtggcagtttcaataacaggtcattgccgagaaaaggatagcactataatatgaaggccatcatcgtgctgctgatggtggtgaccagcaacgccgaccggatctgcaccggcatcaccagctccaacagcccccacgtggtgaagaccgccacccagggcgaggtgaacgtgaccggcgtgatccccctgaccaccacccccaccaagtcctacttcgccaacctgaagggcacccggacccgcggcaagctgtgccccgactgcctgaactgcaccgacctggacgtggccctgggccggcccatgtgcgtgggcaccacccccagcgccaaggcctccatcctgcacgaggtgcgccccgtgaccagcggctgcttccccatcatgcacgaccgcaccaagatccggcagctgcccaacctgctgcgggggtacgagaagatccgcctgtccacccagaacgtcatcgacgccgagaaggcccccggcgggccctaccggctgggcaccagcgggtcctgccccaacgccaccagcaagatcggcttcttcgccaccatggcctgggccgtgcccaaggacaactacaagaacgccaccaaccccctgaccgtcgaggtgccctacatctgcaccgagggggaggaccagatcacggtctggggcttccactccgacaacaagacccagatgaagtccctgtacggggactccaacccgcagaagttcacgagctccgccaacggcgtgaccacgcactacgtcagccagatcggggacttcccggaccagaccgaggacggcgggctgccccagtccggccgcatcgtggtcgactacatgatgcagaagcccgggaagacgggcaccatcgtgtaccagcggggggtcctgctgccgcagaaggtgtggtgcgccagcggccgctccaaggtcatcaaggggagcctgcccctcatcggcgaggccgactgcctgcacgaggagtacgggggcctcaacaagtccaagccgtactacacggggaagcacgccaaggccatcggcaactgcccgatctgggtgaagacccccctgaagctcgccaacgggacgaagtaccggccgcccgccaagctgctcaaggagcgcggcttcttcggggccatcgccggcttcctggaggggggctgggaggggatgatcgccggctggcacgggtacaccagccacggcgcccacggggtcgcggtggccgcggacctcaagtccacgcaggaggccatcaacaagatcaccaagaacctgaacagcctctccgagctggaggtcaagaacctccagcgcctgagcggcgcgatggacgagctccacaacgagatcctggagctcgacgagaaggtggacgacctgcgggccgacacgatctcgtcccagatcgagctcgcggtcctgctcagcaacgaggggatcatcaactcggaggacgagcacctgctcgccctggagcggaagctcaagaagatgctgggcccgtccgcggtggacatcgggaacggctgcttcgagaccaagcacaagtgcaaccagacgtgcctcgaccgcatcgccgcggggaccttcaacgccggcgagttcagcctgcccacgttcgactcgctcaacatcaccgcggcctccctgaacgacgacgggctcgacaaccacacgatcctgctctactacagcaccgcggcctcgtccctggcggtcacgctcatgctggccatcttcatcgtgtacatggtcagccgcgacaacgtgtcgtgctccatctgcctctgatgactcgaggctcgctttcttgctgtccaatttctattaaaggttcctttgttccctaagtccaactactaaactgggggatattatgaagggccttgagcatctggattctgcctaataaaaaacatttattttcattgcaaaaaaaaaaaaaaaaaaaaaaaaaaaaaaaaaaaaaaaaaaaaaaaaaaaaaaaaaaaaaaaaaaaaaaaaaaaaaaaaaaaaaaaaaaaaaaaaaaaaaaaaaaaaaaaaaaaaaaaaaa

SEQ ID NO: 122 - RNA, 2027 nt, synthetic construct
  source 1..2027: mol_type = other RNA; note = I'-H1N1-HA0-mut-B-120A mRNA
gagttaggagttggtggcagtttcaataacaggtcattgccgagaaaaggatagcactataatatgaaggccatcctggtggtgatgctgtacaccttcaccaccgccaacgccgacaccctgtgcatcggctaccacgccaacaacagcaccgacaccgtggacaccgtgctggagaagaacgtgaccgtgacccacagcgtgaacctgctggaggacaagcacaacggcaagctgtgcaagctgcggggcgtggcccccctgcacctgggcaagtgcaacatcgccggctggatcctgggcaaccccgagtgcgagtccctgagcaccgcccgctcctggagctacatcgtggagacctccaacagcgacaacggcacctgctaccccggggacttcatcaactacgaggagctgcgggagcagctgtccagcgtgtccagcttcgagcgcttcgagatcttccccaagacctccagctggcccaaccacgactccgacaacggcgtgaccgccgcctgcccccacgccggggccaagagcttctacaagaacctgatctggctggtgaagaagggcaagtcctaccccaagatcaaccagacctacatcaacgacaaggggaaggaggtcctcgtgctgtggggcatccaccacccccccaccatcgccgaccagcagagcctctaccagaacgccgacgcctacgtcttcgtggggacctcccggtacagcaagaagttcaagcccgagatcgccacccgccccaaggtccgggaccaggagggccgcatgaactactactggaccctggtggagccgggggacaagatcaccttcgaggccaccggcaacctcgtcgccccgcggtacgccttcacgatggagcgcgacgccgggtccggcatcatcatcagcgacacccccgtgcacgactgcaacacgacctgccagacgcccgagggggcgatcaacacctccctgccgttccagaacgtccacccgatcacgatcggcaagtgccccaagtacgtgaagtccaccaagctccggctggccacggggctccgcaacgtcccctccatccagagccagggcctgttcggggcgatcgccggcttcatcgaggggggctggaccgggatggtggacggctggtacgggtaccaccaccagaacgagcagggctccgggtacgcggccgacctcaagtcgacgcagaacgcgatcgacaagatcaccaacaaggtcaacagcgtgatcgagaagatgaacacgcagttcaccgccgtcggcaaggagttcaaccacctggagaagcgcatcgagaacctcaacaagaaggtggacgacgggttcctggacatctggacgtacaacgcggagctcctggtcctcctggagaacgagcggaccctcgactaccacgactccaacgtgaagaacctgtacgagaaggtccgcaaccagctcaagaacaacgccaaggagatcggcaacgggtgcttcgagttctaccacaagtgcgacaacacgtgcatggagtcggtgaagaacggcacctacgactacccgaagtacagcgaggaggcgaagctgaaccgggagaagatcgacggggtcaagctcgactccacgcgcatctaccagatcctggccatctactcgaccgtggcgagctccctcgtcctggtggtctcgctcggcgccatcagcttctggatgtgctccaacgggtcgctgcagtgccggatctgcatctgatgactcgaggctcgctttcttgctgtccaatttctattaaaggttcctttgttccctaagtccaactactaaactgggggatattatgaagggccttgagcatctggattctgcctaataaaaaacatttattttcattgcaaaaaaaaaaaaaaaaaaaaaaaaaaaaaaaaaaaaaaaaaaaaaaaaaaaaaaaaaaaaaaaaaaaaaaaaaaaaaaaaaaaaaaaaaaaaaaaaaaaaaaaaaaaaaaaaaaaaaaaaaa

SEQ ID NO: 123 - RNA, 2027 nt, synthetic construct
  source 1..2027: mol_type = other RNA; note = I'-H3N2-HA0-mut-B-120A mRNA
gagttaggagttggtggcagtttcaataacaggtcattgccgagaaaaggatagcactataatatgaagaccatcatcgccctgagctacatcctgtgcctggtgttcgcccagaagatccccggcaacgacaacagcaccgccaccctgtgcctgggccaccacgccgtgcccaacggcaccatcgtgaagaccatcaccaacgaccggatcgaggtgaccaacgccaccgagctggtgcagaactccagcatcggcgagatctgcgactccccccaccagatcctggacggcggcaactgcaccctgatcgacgccctgctgggcgacccccagtgcgacgggttccagaacaaggagtgggacctgttcgtggagcggagccgcgccaactccaactgctacccctacgacgtgcccgactacgccagcctgcggtccctggtggccagctccggcaccctggagttcaagaacgagagcttcaactggaccggggtcaagcagaacggcacctccagcgcctgcatccgcgggtccagctccagcttcttctcccggctgaactggctcacccacctgaactacacctaccccgccctcaacgtgaccatgcccaacaacgagcagttcgacaagctgtacatctggggcgtccaccaccccagcaccgacaaggaccagatctccctcttcgcccagcccagcgggcgcatcaccgtgtccacgaagcggagccagcaggccgtcatccccaacatcggctcccgcccgcggatccgcgacatccccagccggatctccatctactggacgatcgtgaagccgggggacatcctgctcatcaacagcaccggcaacctgatcgccccccgcgggtacttcaagatccggtccggcaagagctcgatcatgcgctccgacgccccgatcgggaagtgcaagagcgagtgcatcacccccaacggctcgatcccgaacgacaagcccttccagaacgtcaaccggatcacgtacggggcctgcccgcgctacgtgaagcagtccacgctcaagctggccaccggcatgcggaacgtccccgagaagcagacccaggggatcttcggcgccatcgcggggttcatcgagaacggctgggaggggatggtggacggctggtacgggttccggcaccagaacagcgagggccgcgggcaggccgcggacctcaagtcgacgcaggccgcgatcgaccagatcaacggcaagctgaaccggctcatcgggaagacgaacgagaagttccaccagatcgagaaggagttctccgaggtcgagggccgcgtgcaggacctggagaagtacgtcgaggacaccaagatcgacctctggagctacaacgccgagctgctcgtggcgctggagaaccagcacaccatcgacctcacggactcggagatgaacaagctgttcgagaagacgaagaagcagctccgggagaacgccgaggacatggggaacggctgcttcaagatctaccacaagtgcgacaacgcgtgcatcgggtccatccgcaacgagacctacgaccacaacgtctaccgggacgaggccctgaacaaccgcttccagatcaagggcgtggagctcaagagcgggtacaaggactggatcctgtggatctcgttcgcgatgtcctgcttcctcctgtgcatcgccctcctgggcttcatcatgtgggcgtgccagaaggggaacatccggtgcaacatctgcatctgatgactcgaggctcgctttcttgctgtccaatttctattaaaggttcctttgttccctaagtccaactactaaactgggggatattatgaagggccttgagcatctggattctgcctaataaaaaacatttattttcattgcaaaaaaaaaaaaaaaaaaaaaaaaaaaaaaaaaaaaaaaaaaaaaaaaaaaaaaaaaaaaaaaaaaaaaaaaaaaaaaaaaaaaaaaaaaaaaaaaaaaaaaaaaaaaaaaaaaaaaaaaaa

SEQ ID NO: 124 - RNA, 2075 nt, synthetic construct
  source 1..2075: mol_type = other RNA; note = I'-B-Victoria-HA0-mut-B-120A mRNA
gagttaggagttggtggcagtttcaataacaggtcattgccgagaaaaggatagcactataatatgaaggccatcatcgtgctgctgatggtggtgaccagcaacgccgaccggatctgcaccggcatcaccagctccaacagcccccacgtggtgaagaccgccacccagggcgaggtgaacgtgaccggcgtgatccccctgaccaccacccccaccaagtcccacttcgccaacctgaagggcaccgagacccggggcaagctgtgccccaagtgcctgaactgcaccgacctggacgtggccctgggccgccccaagtgcaccggcaagatccccagcgcccgggtgtccatcctgcacgaggtgcgccccgtgaccagcggctgcttccccatcatgcacgaccgcaccaagatccggcagctgcccaacctgctgcgggggtacgagcacgtccgcctgtccacccacaacgtgatcaacgccgaggacgcccccggccggccctacgagatcgggaccagcggctcctgccccaacatcaccaacgggaacggcttcttcgccaccatggcctgggccgtccccaagaacaagaccgccaccaaccccctgaccatcgaggtgccgtacatctgcaccgagggggaggaccagatcaccgtctggggcttccacagcgacaacgagacgcagatggccaagctgtacggggactccaagccccagaagttcacgagctccgccaacggcgtgaccacccactacgtcagccagatcgggggcttcccgaaccagacggaggacgggggcctgccccagtccgggcgcatcgtggtcgactacatggtgcagaagtccggcaagacggggaccatcacgtaccagcggggcatcctgctgccgcagaaggtctggtgcgcctccgggcgcagcaaggtgatcaagggctccctgcccctcatcggggaggccgactgcctgcacgagaagtacggcgggctcaacaagagcaagccgtactacaccggcgagcacgccaaggccatcgggaactgccccatctgggtcaagaccccgctgaagctcgccaacggcacgaagtaccggcccccggccaagctgctcaaggagcaggggttcttcggcgccatcgccgggttcctggagggcgggtgggagggcatgatcgccgggtggcacggctacacgtcccacggggcccacggcgtggcggtcgccgcggacctcaagagcacccaggaggccatcaacaagatcacgaagaacctgaactccctcagcgagctggaggtgaagaacctccagcgcctgtccggggcgatggacgagctccacaacgagatcctggagctcgacgagaaggtcgacgacctgcgggccgacaccatcagctcgcagatcgagctcgcggtgctgctctccaacgagggcatcatcaacagcgaggacgagcacctgctcgccctggagcggaagctcaagaagatgctggggccctcggcggtcgagatcggcaacgggtgcttcgagaccaagcacaagtgcaaccagacgtgcctcgaccgcatcgccgcgggcacgttcgacgccggggagttctccctgccgaccttcgacagcctcaacatcacggcggcctcgctgaacgacgacggcctcgacaaccacaccatcctgctctactactccaccgcggccagctcgctggcggtgacgctcatgatcgccatcttcgtcgtgtacatggtctcccgcgacaacgtgagctgctcgatctgcctgtgatgactcgaggctcgctttcttgctgtccaatttctattaaaggttcctttgttccctaagtccaactactaaactgggggatattatgaagggccttgagcatctggattctgcctaataaaaaacatttattttcattgcaaaaaaaaaaaaaaaaaaaaaaaaaaaaaaaaaaaaaaaaaaaaaaaaaaaaaaaaaaaaaaaaaaaaaaaaaaaaaaaaaaaaaaaaaaaaaaaaaaaaaaaaaaaaaaaaaaaaaaaaaa

SEQ ID NO: 125 - RNA, 2081 nt, synthetic construct
  source 1..2081: mol_type = other RNA; note = I'-B-Yamagata-HA0-mut-B-120A mRNA
gagttaggagttggtggcagtttcaataacaggtcattgccgagaaaaggatagcactataatatgaaggccatcatcgtgctgctgatggtggtgaccagcaacgccgaccggatctgcaccggcatcaccagctccaacagcccccacgtggtgaagaccgccacccagggcgaggtgaacgtgaccggcgtgatccccctgaccaccacccccaccaagtcctacttcgccaacctgaagggcacccggacccgcggcaagctgtgccccgactgcctgaactgcaccgacctggacgtggccctgggccggcccatgtgcgtgggcaccacccccagcgccaaggcctccatcctgcacgaggtgcgccccgtgaccagcggctgcttccccatcatgcacgaccgcaccaagatccggcagctgcccaacctgctgcgggggtacgagaagatccgcctgtccacccagaacgtcatcgacgccgagaaggcccccggcgggccctaccggctgggcaccagcgggtcctgccccaacgccaccagcaagatcggcttcttcgccaccatggcctgggccgtgcccaaggacaactacaagaacgccaccaaccccctgaccgtcgaggtgccctacatctgcaccgagggggaggaccagatcacggtctggggcttccactccgacaacaagacccagatgaagtccctgtacggggactccaacccgcagaagttcacgagctccgccaacggcgtgaccacgcactacgtcagccagatcggggacttcccggaccagaccgaggacggcgggctgccccagtccggccgcatcgtggtcgactacatgatgcagaagcccgggaagacgggcaccatcgtgtaccagcggggggtcctgctgccgcagaaggtgtggtgcgccagcggccgctccaaggtcatcaaggggagcctgcccctcatcggcgaggccgactgcctgcacgaggagtacgggggcctcaacaagtccaagccgtactacacggggaagcacgccaaggccatcggcaactgcccgatctgggtgaagacccccctgaagctcgccaacgggacgaagtaccggccgcccgccaagctgctcaaggagcagggcttcttcggggccatcgccggcttcctggaggggggctgggaggggatgatcgccggctggcacgggtacaccagccacggcgcccacggggtcgcggtggccgcggacctcaagtccacgcaggaggccatcaacaagatcaccaagaacctgaacagcctctccgagctggaggtcaagaacctccagcgcctgagcggcgcgatggacgagctccacaacgagatcctggagctcgacgagaaggtggacgacctgcgggccgacacgatctcgtcccagatcgagctcgcggtcctgctcagcaacgaggggatcatcaactcggaggacgagcacctgctcgccctggagcggaagctcaagaagatgctgggcccgtccgcggtggacatcgggaacggctgcttcgagaccaagcacaagtgcaaccagacgtgcctcgaccgcatcgccgcggggaccttcaacgccggcgagttcagcctgcccacgttcgactcgctcaacatcaccgcggcctccctgaacgacgacgggctcgacaaccacacgatcctgctctactacagcaccgcggcctcgtccctggcggtcacgctcatgctggccatcttcatcgtgtacatggtcagccgcgacaacgtgtcgtgctccatctgcctctgatgactcgaggctcgctttcttgctgtccaatttctattaaaggttcctttgttccctaagtccaactactaaactgggggatattatgaagggccttgagcatctggattctgcctaataaaaaacatttattttcattgcaaaaaaaaaaaaaaaaaaaaaaaaaaaaaaaaaaaaaaaaaaaaaaaaaaaaaaaaaaaaaaaaaaaaaaaaaaaaaaaaaaaaaaaaaaaaaaaaaaaaaaaaaaaaaaaaaaaaaaaaaa

SEQ ID NO: 126 - RNA, 1701 nt, synthetic construct
  source 1..1701: mol_type = other RNA; note = Influenza A H1N1 (A/Wisconsin/588/2019) HA mRNA
atgaaggccatcctggtggtgatgctgtacaccttcaccaccgccaacgccgacaccctgtgcatcggctaccacgccaacaacagcaccgacaccgtggacaccgtgctggagaagaacgtgaccgtgacccacagcgtgaacctgctggaggacaagcacaacggcaagctgtgcaagctgcggggcgtggcccccctgcacctgggcaagtgcaacatcgccggctggatcctgggcaaccccgagtgcgagtccctgagcaccgcccgctcctggagctacatcgtggagacctccaacagcgacaacggcacctgctaccccggggacttcatcaactacgaggagctgcgggagcagctgtccagcgtgtccagcttcgagcgcttcgagatcttccccaagacctccagctggcccaaccacgactccgacaacggcgtgaccgccgcctgcccccacgccggggccaagagcttctacaagaacctgatctggctggtgaagaagggcaagtcctaccccaagatcaaccagacctacatcaacgacaaggggaaggaggtcctcgtgctgtggggcatccaccacccccccaccatcgccgaccagcagagcctctaccagaacgccgacgcctacgtcttcgtggggacctcccggtacagcaagaagttcaagcccgagatcgccacccgccccaaggtccgggaccaggagggccgcatgaactactactggaccctggtggagccgggggacaagatcaccttcgaggccaccggcaacctcgtcgccccgcggtacgccttcacgatggagcgcgacgccgggtccggcatcatcatcagcgacacccccgtgcacgactgcaacacgacctgccagacgcccgagggggcgatcaacacctccctgccgttccagaacgtccacccgatcacgatcggcaagtgccccaagtacgtgaagtccaccaagctccggctggccacggggctccgcaacgtcccctccatccagagccggggcctgttcggggcgatcgccggcttcatcgaggggggctggaccgggatggtggacggctggtacgggtaccaccaccagaacgagcagggctccgggtacgcggccgacctcaagtcgacgcagaacgcgatcgacaagatcaccaacaaggtcaacagcgtgatcgagaagatgaacacgcagttcaccgccgtcggcaaggagttcaaccacctggagaagcgcatcgagaacctcaacaagaaggtggacgacgggttcctggacatctggacgtacaacgcggagctcctggtcctcctggagaacgagcggaccctcgactaccacgactccaacgtgaagaacctgtacgagaaggtccgcaaccagctcaagaacaacgccaaggagatcggcaacgggtgcttcgagttctaccacaagtgcgacaacacgtgcatggagtcggtgaagaacggcacctacgactacccgaagtacagcgaggaggcgaagctgaaccgggagaagatcgacggggtcaagctcgactccacgcgcatctaccagatcctggccatctactcgaccgtggcgagctccctcgtcctggtggtctcgctcggcgccatcagcttctggatgtgctccaacgggtcgctgcagtgccggatctgcatctga

SEQ ID NO: 127 - RNA, 1701 nt, synthetic construct
  source 1..1701: mol_type = other RNA; note = Influenza A H3N2 (A/Cambodia/e0826360/2020) HA mRNA
atgaagaccatcatcgccctgagctacatcctgtgcctggtgttcgcccagaagatccccggcaacgacaacagcaccgccaccctgtgcctgggccaccacgccgtgcccaacggcaccatcgtgaagaccatcaccaacgaccggatcgaggtgaccaacgccaccgagctggtgcagaactccagcatcggcgagatctgcgactccccccaccagatcctggacggcggcaactgcaccctgatcgacgccctgctgggcgacccccagtgcgacgggttccagaacaaggagtgggacctgttcgtggagcggagccgcgccaactccaactgctacccctacgacgtgcccgactacgccagcctgcggtccctggtggccagctccggcaccctggagttcaagaacgagagcttcaactggaccggggtcaagcagaacggcacctccagcgcctgcatccgcgggtccagctccagcttcttctcccggctgaactggctcacccacctgaactacacctaccccgccctcaacgtgaccatgcccaacaacgagcagttcgacaagctgtacatctggggcgtccaccaccccagcaccgacaaggaccagatctccctcttcgcccagcccagcgggcgcatcaccgtgtccacgaagcggagccagcaggccgtcatccccaacatcggctcccgcccgcggatccgcgacatccccagccggatctccatctactggacgatcgtgaagccgggggacatcctgctcatcaacagcaccggcaacctgatcgccccccgcgggtacttcaagatccggtccggcaagagctcgatcatgcgctccgacgccccgatcgggaagtgcaagagcgagtgcatcacccccaacggctcgatcccgaacgacaagcccttccagaacgtcaaccggatcacgtacggggcctgcccgcgctacgtgaagcagtccacgctcaagctggccaccggcatgcggaacgtccccgagaagcagacccgcgggatcttcggcgccatcgcggggttcatcgagaacggctgggaggggatggtggacggctggtacgggttccggcaccagaacagcgagggccgcgggcaggccgcggacctcaagtcgacgcaggccgcgatcgaccagatcaacggcaagctgaaccggctcatcgggaagacgaacgagaagttccaccagatcgagaaggagttctccgaggtcgagggccgcgtgcaggacctggagaagtacgtcgaggacaccaagatcgacctctggagctacaacgccgagctgctcgtggcgctggagaaccagcacaccatcgacctcacggactcggagatgaacaagctgttcgagaagacgaagaagcagctccgggagaacgccgaggacatggggaacggctgcttcaagatctaccacaagtgcgacaacgcgtgcatcgggtccatccgcaacgagacctacgaccacaacgtctaccgggacgaggccctgaacaaccgcttccagatcaagggcgtggagctcaagagcgggtacaaggactggatcctgtggatctcgttcgcgatgtcctgcttcctcctgtgcatcgccctcctgggcttcatcatgtgggcgtgccagaaggggaacatccggtgcaacatctgcatctga

SEQ ID NO: 128 - RNA, 1749 nt, synthetic construct
  source 1..1749: mol_type = other RNA; note = Influenza B Victoria lineage ( B/Washington/02/2019) HA mRNA
atgaaggccatcatcgtgctgctgatggtggtgaccagcaacgccgaccggatctgcaccggcatcaccagctccaacagcccccacgtggtgaagaccgccacccagggcgaggtgaacgtgaccggcgtgatccccctgaccaccacccccaccaagtcccacttcgccaacctgaagggcaccgagacccggggcaagctgtgccccaagtgcctgaactgcaccgacctggacgtggccctgggccgccccaagtgcaccggcaagatccccagcgcccgggtgtccatcctgcacgaggtgcgccccgtgaccagcggctgcttccccatcatgcacgaccgcaccaagatccggcagctgcccaacctgctgcgggggtacgagcacgtccgcctgtccacccacaacgtgatcaacgccgaggacgcccccggccggccctacgagatcgggaccagcggctcctgccccaacatcaccaacgggaacggcttcttcgccaccatggcctgggccgtccccaagaacaagaccgccaccaaccccctgaccatcgaggtgccgtacatctgcaccgagggggaggaccagatcaccgtctggggcttccacagcgacaacgagacgcagatggccaagctgtacggggactccaagccccagaagttcacgagctccgccaacggcgtgaccacccactacgtcagccagatcgggggcttcccgaaccagacggaggacgggggcctgccccagtccgggcgcatcgtggtcgactacatggtgcagaagtccggcaagacggggaccatcacgtaccagcggggcatcctgctgccgcagaaggtctggtgcgcctccgggcgcagcaaggtgatcaagggctccctgcccctcatcggggaggccgactgcctgcacgagaagtacggcgggctcaacaagagcaagccgtactacaccggcgagcacgccaaggccatcgggaactgccccatctgggtcaagaccccgctgaagctcgccaacggcacgaagtaccggcccccggccaagctgctcaaggagcgcgggttcttcggcgccatcgccgggttcctggagggcgggtgggagggcatgatcgccgggtggcacggctacacgtcccacggggcccacggcgtggcggtcgccgcggacctcaagagcacccaggaggccatcaacaagatcacgaagaacctgaactccctcagcgagctggaggtgaagaacctccagcgcctgtccggggcgatggacgagctccacaacgagatcctggagctcgacgagaaggtcgacgacctgcgggccgacaccatcagctcgcagatcgagctcgcggtgctgctctccaacgagggcatcatcaacagcgaggacgagcacctgctcgccctggagcggaagctcaagaagatgctggggccctcggcggtcgagatcggcaacgggtgcttcgagaccaagcacaagtgcaaccagacgtgcctcgaccgcatcgccgcgggcacgttcgacgccggggagttctccctgccgaccttcgacagcctcaacatcacggcggcctcgctgaacgacgacggcctcgacaaccacaccatcctgctctactactccaccgcggccagctcgctggcggtgacgctcatgatcgccatcttcgtcgtgtacatggtctcccgcgacaacgtgagctgctcgatctgcctgtga

SEQ ID NO: 129 - RNA, 1755 nt, synthetic construct; identical to SEQ ID NO: 90
  source 1..1755: mol_type = other RNA; note = Influenza B Yamagata lineage (B/Phuket/3073/2013) HA mRNA

SEQ ID NO: 130 - RNA, 3810 nt, synthetic construct
  source 1..3810: mol_type = other RNA; note = SARS-COV-2 BA.4 Spike mRNA
atgttcgtgttcctggtgctgctgcccctggtgagctctcagtgcgtgaacctgatcacaagaacacagtcgtacaccaacagcttcacaagaggcgtgtactaccccgacaaggtgttcagaagcagcgtgctgcactccacccaagacctgtttctgcccttcttcagcaacgtgacctggttccacgccatcagcggcaccaacggcaccaagagattcgacaaccccgtgctgcccttcaacgacggcgtgtacttcgctagcaccgaaaagagcaacatcatcagaggctggatcttcggcaccaccctagactccaagacacaaagcctgctgatcgttaacaacgcgaccaacgtggtgatcaaggtgtgcgagtttcagttctgcaacgaccccttcctggacgtgtactaccacaagaacaacaagagctggatggagagcgagttcagagtctacagcagcgccaacaactgcaccttcgagtacgtgtctcagcccttcctgatggacctggagggcaagcaaggcaatttcaagaacctaagagagttcgtgttcaagaacatcgacggctacttcaagatctacagcaagcacacccccatcaacctggggagagacctgccccaaggcttcagcgccctggagcccctggtggacctgcccatcggcatcaacatcacaagatttcagaccctgctggccctgcaccgtagctacctaacccccggcgatagttcctctggctggacggccggcgctgccgcctactacgtgggctacctgcagcctagaaccttcctgctgaagtacaacgagaacggcactatcactgatgccgtggactgtgccctggaccccctgagcgagaccaagtgcaccctcaagagcttcaccgtggagaagggcatctatcagacaagcaacttcagagtgcagcccaccgagagcatcgtgagattccccaacatcaccaacctgtgccccttcgacgaggtgttcaacgccacaagattcgctagcgtgtacgcgtggaacagaaagagaatcagcaactgcgtggccgactacagcgtgctgtacaacttcgctcccttcttcgccttcaagtgctatggcgtcagccccaccaagctgaacgacctgtgcttcaccaacgtgtacgccgacagcttcgtgatcagaggcaacgaggtgagccagattgcccccgggcaaaccggcaacatcgccgactacaactacaagctgcccgacgacttcaccggctgcgtgatcgcgtggaacagcaataagctggattccaaggtgggcggcaactacaactaccggtacagactgttcagaaagagcaacctgaagcccttcgagagagacatcagcaccgagatctaccaagccggcaacaagccctgcaacggcgtggcgggcgtcaactgctacttccccctgcagagctacggctttaggcccacctacggcgtgggccatcagccctacagagtggtggtgctgagcttcgagctgctgcacgcccccgcaaccgtgtgcggccccaaaaagagcaccaacctggtgaagaacaagtgcgtgaacttcaactttaatggccttaagggcacgggcgtgctgaccgagagcaacaagaagttcctgccatttcagcaattcggcagagacatcgccgacaccaccgacgcggtcagagaccctcagaccctggagatcctggacatcaccccctgtagcttcggcggcgtgagcgtgatcacccccggcactaacacaagcaaccaagtggccgtgctgtaccaaggcgtgaactgcaccgaggtgcccgtggccatccacgccgatcagctgacccccacctggagagtatacagcaccggaagcaacgtgtttcagacaagagccggctgcctgatcggcgccgagtacgtgaacaacagctacgagtgcgacatccccatcggcgccggcatctgcgctagctatcagacacagaccaagagccaccggagagctagaagcgtggcttctcagagcatcatcgcctacaccatgagcctgggcgccgagaacagcgtggcctacagcaacaacagcatcgccatccccaccaacttcaccatcagcgtgaccaccgagatcctgcccgtaagtatgaccaagacaagcgtggactgcaccatgtacatctgcggcgacagcaccgagtgcagcaacctgctgctgcagtacggcagcttctgcacacagctgaagagagccctgaccggcatcgccgtggagcaagacaagaacacccaagaggtgttcgcccaagtgaagcagatctacaagaccccccccatcaagtacttcggcggcttcaacttcagccaaatcctgcccgaccctagcaagcctagcaagcggagcttcatcgaggacctgctgttcaacaaggtgaccctggccgacgccggcttcatcaagcagtacggcgactgcctaggcgacatcgcagctagagacctgatctgcgctcagaagttcaatggactcaccgtgctcccccccctgctgaccgacgagatgatcgctcagtacacctctgccctgctggcgggaaccataacaagcggttggacatttggcgccggggccgcactgcaaatccccttcgccatgcagatggcctacagattcaacggcatcggcgtgacacagaacgtgctgtacgagaatcagaagctgatcgccaatcagttcaacagcgccatcggcaagatccaagacagcctgagcagcaccgctagcgccctgggcaagctgcaagacgtggtgaatcacaacgcccaagccctgaacaccctggtgaagcagctgagcagcaagttcggcgccatcagcagcgtattgaatgacatcctgtctagactggacccccccgaggccgaggtgcagatcgacagactgatcaccggcagactgcagagcctgcagacctacgtgacacagcagctgatcagagccgccgagatcagagctagcgccaacctggccgccaccaagatgagcgagtgcgtgctggggcagagcaagagagtggacttctgcggcaagggctaccacctgatgagcttccctcagagcgccccccacggcgtggtgttcctgcacgtgacctacgtgcccgcccaagagaagaacttcaccaccgctcccgccatctgccacgacggcaaggcccacttccctagagagggcgtgttcgtgagcaacggcacccactggttcgtgacacagagaaacttctacgagcctcagatcatcaccaccgacaacaccttcgtgagcggcaactgcgacgtggtgatcggcatagtgaacaacaccgtatacgaccccctgcagcccgagctggacagcttcaaggaggagctggacaagtacttcaaaaaccatactagccccgacgtggacctgggagacatctctggcatcaacgctagcgtggtgaacattcagaaggagatcgaccggctgaatgaggtggccaagaacctgaacgagagcctgatcgacctgcaagagctgggcaagtacgagcagtacatcaagtggccctggtacatctggctgggcttcatcgccggcctgatcgccatcgtgatggtgaccatcatgctgtgctgcatgacaagctgttgcagctgcctgaaaggttgctgcagctgtggctcgtgctgcaagttcgacgaggacgacagcgagcccgtgctgaagggcgtgaagctgcactacacctgatga

SEQ ID NO: 131 - RNA, 1701 nt, synthetic construct
  source 1..1701: mol_type = other RNA; note = Influenza A H1N1 HA0 mutant mRNA
atgaaggccatcctggtggtgatgctgtacaccttcaccaccgccaacgccgacaccctgtgcatcggctaccacgccaacaacagcaccgacaccgtggacaccgtgctggagaagaacgtgaccgtgacccacagcgtgaacctgctggaggacaagcacaacggcaagctgtgcaagctgcggggcgtggcccccctgcacctgggcaagtgcaacatcgccggctggatcctgggcaaccccgagtgcgagtccctgagcaccgcccgctcctggagctacatcgtggagacctccaacagcgacaacggcacctgctaccccggggacttcatcaactacgaggagctgcgggagcagctgtccagcgtgtccagcttcgagcgcttcgagatcttccccaagacctccagctggcccaaccacgactccgacaacggcgtgaccgccgcctgcccccacgccggggccaagagcttctacaagaacctgatctggctggtgaagaagggcaagtcctaccccaagatcaaccagacctacatcaacgacaaggggaaggaggtcctcgtgctgtggggcatccaccacccccccaccatcgccgaccagcagagcctctaccagaacgccgacgcctacgtcttcgtggggacctcccggtacagcaagaagttcaagcccgagatcgccacccgccccaaggtccgggaccaggagggccgcatgaactactactggaccctggtggagccgggggacaagatcaccttcgaggccaccggcaacctcgtcgccccgcggtacgccttcacgatggagcgcgacgccgggtccggcatcatcatcagcgacacccccgtgcacgactgcaacacgacctgccagacgcccgagggggcgatcaacacctccctgccgttccagaacgtccacccgatcacgatcggcaagtgccccaagtacgtgaagtccaccaagctccggctggccacggggctccgcaacgtcccctccatccagagccagggcctgttcggggcgatcgccggcttcatcgaggggggctggaccgggatggtggacggctggtacgggtaccaccaccagaacgagcagggctccgggtacgcggccgacctcaagtcgacgcagaacgcgatcgacaagatcaccaacaaggtcaacagcgtgatcgagaagatgaacacgcagttcaccgccgtcggcaaggagttcaaccacctggagaagcgcatcgagaacctcaacaagaaggtggacgacgggttcctggacatctggacgtacaacgcggagctcctggtcctcctggagaacgagcggaccctcgactaccacgactccaacgtgaagaacctgtacgagaaggtccgcaaccagctcaagaacaacgccaaggagatcggcaacgggtgcttcgagttctaccacaagtgcgacaacacgtgcatggagtcggtgaagaacggcacctacgactacccgaagtacagcgaggaggcgaagctgaaccgggagaagatcgacggggtcaagctcgactccacgcgcatctaccagatcctggccatctactcgaccgtggcgagctccctcgtcctggtggtctcgctcggcgccatcagcttctggatgtgctccaacgggtcgctgcagtgccggatctgcatctga

SEQ ID NO: 132 - RNA, 1701 nt, synthetic construct
  source 1..1701: mol_type = other RNA; note = Influenza A H3N2 HA0 mutant mRNA
atgaagaccatcatcgccctgagctacatcctgtgcctggtgttcgcccagaagatccccggcaacgacaacagcaccgccaccctgtgcctgggccaccacgccgtgcccaacggcaccatcgtgaagaccatcaccaacgaccggatcgaggtgaccaacgccaccgagctggtgcagaactccagcatcggcgagatctgcgactccccccaccagatcctggacggcggcaactgcaccctgatcgacgccctgctgggcgacccccagtgcgacgggttccagaacaaggagtgggacctgttcgtggagcggagccgcgccaactccaactgctacccctacgacgtgcccgactacgccagcctgcggtccctggtggccagctccggcaccctggagttcaagaacgagagcttcaactggaccggggtcaagcagaacggcacctccagcgcctgcatccgcgggtccagctccagcttcttctcccggctgaactggctcacccacctgaactacacctaccccgccctcaacgtgaccatgcccaacaacgagcagttcgacaagctgtacatctggggcgtccaccaccccagcaccgacaaggaccagatctccctcttcgcccagcccagcgggcgcatcaccgtgtccacgaagcggagccagcaggccgtcatccccaacatcggctcccgcccgcggatccgcgacatccccagccggatctccatctactggacgatcgtgaagccgggggacatcctgctcatcaacagcaccggcaacctgatcgccccccgcgggtacttcaagatccggtccggcaagagctcgatcatgcgctccgacgccccgatcgggaagtgcaagagcgagtgcatcacccccaacggctcgatcccgaacgacaagcccttccagaacgtcaaccggatcacgtacggggcctgcccgcgctacgtgaagcagtccacgctcaagctggccaccggcatgcggaacgtccccgagaagcagacccaggggatcttcggcgccatcgcggggttcatcgagaacggctgggaggggatggtggacggctggtacgggttccggcaccagaacagcgagggccgcgggcaggccgcggacctcaagtcgacgcaggccgcgatcgaccagatcaacggcaagctgaaccggctcatcgggaagacgaacgagaagttccaccagatcgagaaggagttctccgaggtcgagggccgcgtgcaggacctggagaagtacgtcgaggacaccaagatcgacctctggagctacaacgccgagctgctcgtggcgctggagaaccagcacaccatcgacctcacggactcggagatgaacaagctgttcgagaagacgaagaagcagctccgggagaacgccgaggacatggggaacggctgcttcaagatctaccacaagtgcgacaacgcgtgcatcgggtccatccgcaacgagacctacgaccacaacgtctaccgggacgaggccctgaacaaccgcttccagatcaagggcgtggagctcaagagcgggtacaaggactggatcctgtggatctcgttcgcgatgtcctgcttcctcctgtgcatcgccctcctgggcttcatcatgtgggcgtgccagaaggggaacatccggtgcaacatctgcatctga

SEQ ID NO: 133 - RNA, 1749 nt, synthetic construct
  source 1..1749: mol_type = other RNA; note = Influenza B Victoria HA0 mutant mRNA
atgaaggccatcatcgtgctgctgatggtggtgaccagcaacgccgaccggatctgcaccggcatcaccagctccaacagcccccacgtggtgaagaccgccacccagggcgaggtgaacgtgaccggcgtgatccccctgaccaccacccccaccaagtcccacttcgccaacctgaagggcaccgagacccggggcaagctgtgccccaagtgcctgaactgcaccgacctggacgtggccctgggccgccccaagtgcaccggcaagatccccagcgcccgggtgtccatcctgcacgaggtgcgccccgtgaccagcggctgcttccccatcatgcacgaccgcaccaagatccggcagctgcccaacctgctgcgggggtacgagcacgtccgcctgtccacccacaacgtgatcaacgccgaggacgcccccggccggccctacgagatcgggaccagcggctcctgccccaacatcaccaacgggaacggcttcttcgccaccatggcctgggccgtccccaagaacaagaccgccaccaaccccctgaccatcgaggtgccgtacatctgcaccgagggggaggaccagatcaccgtctggggcttccacagcgacaacgagacgcagatggccaagctgtacggggactccaagccccagaagttcacgagctccgccaacggcgtgaccacccactacgtcagccagatcgggggcttcccgaaccagacggaggacgggggcctgccccagtccgggcgcatcgtggtcgactacatggtgcagaagtccggcaagacggggaccatcacgtaccagcggggcatcctgctgccgcagaaggtctggtgcgcctccgggcgcagcaaggtgatcaagggctccctgcccctcatcggggaggccgactgcctgcacgagaagtacggcgggctcaacaagagcaagccgtactacaccggcgagcacgccaaggccatcgggaactgccccatctgggtcaagaccccgctgaagctcgccaacggcacgaagtaccggcccccggccaagctgctcaaggagcaggggttcttcggcgccatcgccgggttcctggagggcgggtgggagggcatgatcgccgggtggcacggctacacgtcccacggggcccacggcgtggcggtcgccgcggacctcaagagcacccaggaggccatcaacaagatcacgaagaacctgaactccctcagcgagctggaggtgaagaacctccagcgcctgtccggggcgatggacgagctccacaacgagatcctggagctcgacgagaaggtcgacgacctgcgggccgacaccatcagctcgcagatcgagctcgcggtgctgctctccaacgagggcatcatcaacagcgaggacgagcacctgctcgccctggagcggaagctcaagaagatgctggggccctcggcggtcgagatcggcaacgggtgcttcgagaccaagcacaagtgcaaccagacgtgcctcgaccgcatcgccgcgggcacgttcgacgccggggagttctccctgccgaccttcgacagcctcaacatcacggcggcctcgctgaacgacgacggcctcgacaaccacaccatcctgctctactactccaccgcggccagctcgctggcggtgacgctcatgatcgccatcttcgtcgtgtacatggtctcccgcgacaacgtgagctgctcgatctgcctgtga

SEQ ID NO: 134 - RNA, 1755 nt, synthetic construct
  source 1..1755: mol_type = other RNA; note = Influenza B Yamagata HA0 mutant mRNA
atgaaggccatcatcgtgctgctgatggtggtgaccagcaacgccgaccggatctgcaccggcatcaccagctccaacagcccccacgtggtgaagaccgccacccagggcgaggtgaacgtgaccggcgtgatccccctgaccaccacccccaccaagtcctacttcgccaacctgaagggcacccggacccgcggcaagctgtgccccgactgcctgaactgcaccgacctggacgtggccctgggccggcccatgtgcgtgggcaccacccccagcgccaaggcctccatcctgcacgaggtgcgccccgtgaccagcggctgcttccccatcatgcacgaccgcaccaagatccggcagctgcccaacctgctgcgggggtacgagaagatccgcctgtccacccagaacgtcatcgacgccgagaaggcccccggcgggccctaccggctgggcaccagcgggtcctgccccaacgccaccagcaagatcggcttcttcgccaccatggcctgggccgtgcccaaggacaactacaagaacgccaccaaccccctgaccgtcgaggtgccctacatctgcaccgagggggaggaccagatcacggtctggggcttccactccgacaacaagacccagatgaagtccctgtacggggactccaacccgcagaagttcacgagctccgccaacggcgtgaccacgcactacgtcagccagatcggggacttcccggaccagaccgaggacggcgggctgccccagtccggccgcatcgtggtcgactacatgatgcagaagcccgggaagacgggcaccatcgtgtaccagcggggggtcctgctgccgcagaaggtgtggtgcgccagcggccgctccaaggtcatcaaggggagcctgcccctcatcggcgaggccgactgcctgcacgaggagtacgggggcctcaacaagtccaagccgtactacacggggaagcacgccaaggccatcggcaactgcccgatctgggtgaagacccccctgaagctcgccaacgggacgaagtaccggccgcccgccaagctgctcaaggagcagggcttcttcggggccatcgccggcttcctggaggggggctgggaggggatgatcgccggctggcacgggtacaccagccacggcgcccacggggtcgcggtggccgcggacctcaagtccacgcaggaggccatcaacaagatcaccaagaacctgaacagcctctccgagctggaggtcaagaacctccagcgcctgagcggcgcgatggacgagctccacaacgagatcctggagctcgacgagaaggtggacgacctgcgggccgacacgatctcgtcccagatcgagctcgcggtcctgctcagcaacgaggggatcatcaactcggaggacgagcacctgctcgccctggagcggaagctcaagaagatgctgggcccgtccgcggtggacatcgggaacggctgcttcgagaccaagcacaagtgcaaccagacgtgcctcgaccgcatcgccgcggggaccttcaacgccggcgagttcagcctgcccacgttcgactcgctcaacatcaccgcggcctccctgaacgacgacgggctcgacaaccacacgatcctgctctactacagcaccgcggcctcgtccctggcggtcacgctcatgctggccatcttcatcgtgtacatggtcagccgcgacaacgtgtcgtgctccatctgcctctga

SEQ ID NO: 135 - DNA, 120 bp, synthetic construct
  source 1..120: mol_type = other DNA; note = poly A
aaaaaaaaaaaaaaaaaaaaaaaaaaaaaaaaaaaaaaaaaaaaaaaaaaaaaaaaaaaaaaaaaaaaaaaaaaaaaaaaaaaaaaaaaaaaaaaaaaaaaaaaaaaaaaaaaaaaaaaa

SEQ ID NO: 136 - protein, 1268 aa, Severe acute respiratory syndrome coronavirus 2
  source 1..1268: note = SARS-COV-2 BA.4 Spike
MFVFLVLLPLVSSQCVNLITRTQSYTNSFTRGVYYPDKVFRSSVLHSTQDLFLPFFSNVTWFHAISGTNGTKRFDNPVLPFNDGVYFASTEKSNIIRGWIFGTTLDSKTQSLLIVNNATNVVIKVCEFQFCNDPFLDVYYHKNNKSWMESEFRVYSSANNCTFEYVSQPFLMDLEGKQGNFKNLREFVFKNIDGYFKIYSKHTPINLGRDLPQGFSALEPLVDLPIGINITRFQTLLALHRSYLTPGDXSSGWTAGAAAYYVGYLQPRTFLLKYNENGTITDAVDCALDPLSETKCTLKSFTVEKGIYQTSNFRVQPTESIVRFPNITNLCPFDEVFNATRFASVYAWNRKRISNCVADYSVLYNFAPFFAFKCYGVSPTKLNDLCFTNVYADSFVIRGNEVSQIAPGQTGNIADYNYKLPDDFTGCVIAWNSNKLDSKVGGNYNYRYRLFRKSNLKPFERDISTEIYQAGNKPCNGVAGVNCYFPLQSYGFRPTYGVGHQPYRVVVLSFELLHAPATVCGPKKSTNLVKNKCVNFNFNGLKGTGVLTESNKKFLPFQQFGRDIADTTDAVRDPQTLEILDITPCSFGGVSVITPGTNTSNQVAVLYQGVNCTEVPVAIHADQLTPTWRVYSTGSNVFQTRAGCLIGAEYVNNSYECDIPIGAGICASYQTQTKSHRRARSVASQSIIAYTMSLGAENSVAYSNNSIAIPTNFTISVTTEILPVXMTKTSVDCTMYICGDSTECSNLLLQYGSFCTQLKRALTGIAVEQDKNTQEVFAQVKQIYKTPPIKYFGGFNFSQILPDPSKPSKRSFIEDLLFNKVTLADAGFIKQYGDCLGDIAARDLICAQKFNGLTVLPPLLTDEMIAQYTSALLAGTITSGWTFGAGAALQIPFAMQMAYRFNGIGVTQNVLYENQKLIANQFNSAIGKIQDSLSSTASALGKLQDVVNHNAQALNTLVKQLSSKFGAISSVLNDILSRLDPPEAEVQIDRLITGRLQSLQTYVTQQLIRAAEIRASANLAATKMSECVLGQSKRVDFCGKGYHLMSFPQSAPHGVVFLHVTYVPAQEKNFTTAPAICHDGKAHFPREGVFVSNGTHWFVTQRNFYEPQIITTDNTFVSGNCDVVIGIVNNTVYDPLQPELDSFKEELDKYFKNHTSPDVDLGDISGINASVVNIQKEIDRLNEVAKNLNESLIDLQELGKYEQYIKWPWYIWLGFIAGLIAIVMVTIMLCCMTSCCSCLKGCCSCGSCCKFDEDDSEPVLKGVKLHYT

SEQ ID NO: 137 - DNA, 62 bp, synthetic construct
  source 1..62: mol_type = other DNA; note; note (original language) = 5'UTR I' truncation
agttaggagttggtggcagtttcaataacaggtcattgccgagaaaaggatagcactataat

SEQ ID NO: 138 - DNA, 61 bp, synthetic construct
  source 1..61: mol_type = other DNA; note; note (original language) = 5'UTR I' truncation
gttaggagttggtggcagtttcaataacaggtcattgccgagaaaaggatagcactataat

SEQ ID NO: 139 - DNA, 60 bp, synthetic construct
  source 1..60: mol_type = other DNA; note; note (original language) = 5'UTR I' truncation
ttaggagttggtggcagtttcaataacaggtcattgccgagaaaaggatagcactataat

SEQ ID NO: 140 - DNA, 58 bp, synthetic construct
  source 1..58: mol_type = other DNA; note; note (original language) = 5'UTR I' truncation
aggagttggtggcagtttcaataacaggtcattgccgagaaaaggatagcactataat

SEQ ID NO: 141 - DNA, 57 bp, synthetic construct
  source 1..57: mol_type = other DNA; note; note (original language) = 5'UTR I' truncation
ggagttggtggcagtttcaataacaggtcattgccgagaaaaggatagcactataat

SEQ ID NO: 142 - DNA, 56 bp, synthetic construct
  source 1..56: mol_type = other DNA; note; note (original language) = 5'UTR I' truncation
gagttggtggcagtttcaataacaggtcattgccgagaaaaggatagcactataat

SEQ ID NO: 143 - DNA, 54 bp, synthetic construct
  source 1..54: mol_type = other DNA; note; note (original language) = 5'UTR I' truncation
gttggtggcagtttcaataacaggtcattgccgagaaaaggatagcactataat

SEQ ID NO: 144 - DNA, 53 bp, synthetic construct
  source 1..53: mol_type = other DNA; note; note (original language) = 5'UTR I' truncation
ttggtggcagtttcaataacaggtcattgccgagaaaaggatagcactataat

SEQ ID NO: 145 - DNA, 52 bp, synthetic construct
  source 1..52: mol_type = other DNA; note; note (original language) = 5'UTR I' truncation
tggtggcagtttcaataacaggtcattgccgagaaaaggatagcactataat

SEQ ID NO: 146 - DNA, 50 bp, synthetic construct
  source 1..50: mol_type = other DNA; note; note (original language) = 5'UTR I' truncation
gtggcagtttcaataacaggtcattgccgagaaaaggatagcactataat

SEQ ID NO: 147 - DNA, 49 bp, synthetic construct
  source 1..49: mol_type = other DNA; note; note (original language) = 5'UTR I' truncation
tggcagtttcaataacaggtcattgccgagaaaaggatagcactataat

SEQ ID NO: 148 - DNA, 48 bp, synthetic construct
  source 1..48: mol_type = other DNA; note; note (original language) = 5'UTR I' truncation
ggcagtttcaataacaggtcattgccgagaaaaggatagcactataat

SEQ ID NO: 149 - DNA, 46 bp, synthetic construct
  source 1..46: mol_type = other DNA; note; note (original language) = 5'UTR I' truncation
cagtttcaataacaggtcattgccgagaaaaggatagcactataat

SEQ ID NO: 150 - DNA, 45 bp, synthetic construct
  source 1..45: mol_type = other DNA; note; note (original language) = 5'UTR I' truncation
agtttcaataacaggtcattgccgagaaaaggatagcactataat

SEQ ID NO: 151 - DNA, 44 bp, synthetic construct
  source 1..44: mol_type = other DNA; note; note (original language) = 5'UTR I' truncation
gtttcaataacaggtcattgccgagaaaaggatagcactataat

SEQ ID NO: 152 - DNA, 42 bp, synthetic construct
  source 1..42: mol_type = other DNA; note; note (original language) = 5'UTR I' truncation
ttcaataacaggtcattgccgagaaaaggatagcactataat

SEQ ID NO: 153 - DNA, 41 bp, synthetic construct
  source 1..41: mol_type = other DNA; note; note (original language) = 5'UTR I' truncation
tcaataacaggtcattgccgagaaaaggatagcactataat

SEQ ID NO: 154 - DNA, 40 bp, synthetic construct
  source 1..40: mol_type = other DNA; note; note (original language) = 5'UTR I' truncation
caataacaggtcattgccgagaaaaggatagcactataat

SEQ ID NO: 155 - DNA, 38 bp, synthetic construct
  source 1..38: mol_type = other DNA; note; note (original language) = 5'UTR I' truncation
ataacaggtcattgccgagaaaaggatagcactataat

SEQ ID NO: 156 - DNA, 37 bp, synthetic construct
  source 1..37: mol_type = other DNA; note; note (original language) = 5'UTR I' truncation
taacaggtcattgccgagaaaaggatagcactataat

SEQ ID NO: 157 - DNA, 36 bp, synthetic construct
  source 1..36: mol_type = other DNA; note; note (original language) = 5'UTR I' truncation
aacaggtcattgccgagaaaaggatagcactataat

SEQ ID NO: 158 - DNA, 34 bp, synthetic construct
  source 1..34: mol_type = other DNA; note; note (original language) = 5'UTR I' truncation
caggtcattgccgagaaaaggatagcactataat

SEQ ID NO: 159 - DNA, 33 bp, synthetic construct
  source 1..33: mol_type = other DNA; note; note (original language) = 5'UTR I' truncation
aggtcattgccgagaaaaggatagcactataat

SEQ ID NO: 160 - DNA, 32 bp, synthetic construct
  source 1..32: mol_type = other DNA; note; note (original language) = 5'UTR I' truncation
ggtcattgccgagaaaaggatagcactataat

SEQ ID NO: 161 - DNA, 30 bp, synthetic construct
  source 1..30: mol_type = other DNA; note; note (original language) = 5'UTR I' truncation
tcattgccgagaaaaggatagcactataat

SEQ ID NO: 162 - DNA, 29 bp, synthetic construct
  source 1..29: mol_type = other DNA; note; note (original language) = 5'UTR I' truncation
cattgccgagaaaaggatagcactataat

SEQ ID NO: 163 - DNA, 28 bp, synthetic construct
  source 1..28: mol_type = other DNA; note; note (original language) = 5'UTR I' truncation
attgccgagaaaaggatagcactataat

SEQ ID NO: 164 - DNA, 26 bp, synthetic construct
  source 1..26: mol_type = other DNA; note; note (original language) = 5'UTR I' truncation
tgccgagaaaaggatagcactataat

SEQ ID NO: 165 - DNA, 25 bp, synthetic construct
  source 1..25: mol_type = other DNA; note; note (original language) = 5'UTR I' truncation
gccgagaaaaggatagcactataat

SEQ ID NO: 166 - DNA, 24 bp, synthetic construct
  source 1..24: mol_type = other DNA; note; note (original language) = 5'UTR I' truncation
ccgagaaaaggatagcactataat

SEQ ID NO: 167 - DNA, 22 bp, synthetic construct
  source 1..22: mol_type = other DNA; note; note (original language) = 5'UTR I' truncation
gagaaaaggatagcactataat

SEQ ID NO: 168 - DNA, 21 bp, synthetic construct
  source 1..21: mol_type = other DNA; note; note (original language) = 5'UTR I' truncation
agaaaaggatagcactataat

SEQ ID NO: 169 - DNA, 20 bp, synthetic construct
  source 1..20: mol_type = other DNA; note; note (original language) = 5'UTR I' truncation
gaaaaggatagcactataat

SEQ ID NO: 170 - DNA, 18 bp, synthetic construct
  source 1..18: mol_type = other DNA; note; note (original language) = 5'UTR I' truncation
aaaggatagcactataat

SEQ ID NO: 171 - DNA, 17 bp, synthetic construct
  source 1..17: mol_type = other DNA; note; note (original language) = 5'UTR I' truncation
aaggatagcactataat

SEQ ID NO: 172 - DNA, 16 bp, synthetic construct
  source 1..16: mol_type = other DNA; note; note (original language) = 5'UTR I' truncation
aggatagcactataat

SEQ ID NO: 173 - DNA, 34 bp, synthetic construct
  source 1..34: mol_type = other DNA; note; note (original language) = 5'UTR I' truncation
tcaataacaggtcattgccgagaaaaggatagca

SEQ ID NO: 174 - DNA, 37 bp, synthetic construct
  source 1..37: mol_type = other DNA; note; note (original language) = 5'UTR I' truncation
tcaataacaggtcattgccgagaaaaggatagcacta

SEQ ID NO: 175 - DNA, 36 bp, synthetic construct
  source 1..36: mol_type = other DNA; note; note (original language) = 5'UTR I' truncation
tcaataacaggtcattgccgagaaaaggatagcact

SEQ ID NO: 176 - DNA, 39 bp, synthetic construct
  source 1..39: mol_type = other DNA; note; note (original language) = 5'UTR I' truncation
tcaataacaggtcattgccgagaaaaggatagcactata

SEQ ID NO: 177 - DNA, 27 bp, synthetic construct
  source 1..27: mol_type = other DNA; note; note (original language) = 5'UTR I' truncation
tcaataacaggtcattgccgagaaaag

SEQ ID NO: 178 - DNA, 31 bp, synthetic construct
  source 1..31: mol_type = other DNA; note; note (original language) = 5'UTR I' truncation
tcaataacaggtcattgccgagaaaaggata

SEQ ID NO: 179 - DNA, 30 bp, synthetic construct
  source 1..30: mol_type = other DNA; note; note (original language) = 5'UTR I' truncation
tcaataacaggtcattgccgagaaaaggat

SEQ ID NO: 180 - DNA, 33 bp, synthetic construct
  source 1..33: mol_type = other DNA; note; note (original language) = 5'UTR I' truncation
tcaataacaggtcattgccgagaaaaggatagc

SEQ ID NO: 181 - DNA, 26 bp, synthetic construct
  source 1..26: mol_type = other DNA; note; note (original language) = 5'UTR I' truncation
tcaataacaggtcattgccgagaaaa

SEQ ID NO: 182 - DNA, 28 bp, synthetic construct
  source 1..28: mol_type = other DNA; note; note (original language) = 5'UTR I' truncation
tcaataacaggtcattgccgagaaaagg

SEQ ID NO: 183 - DNA, 25 bp, synthetic construct
  source 1..25: mol_type = other DNA; note; note (original language) = 5'UTR I' truncation
tcaataacaggtcattgccgagaaa

SEQ ID NO: 184 - DNA, 16 bp, synthetic construct
  source 1..16: mol_type = other DNA; note; note (original language) = 5'UTR I' truncation
tcaataacaggtcatt

SEQ ID NO: 185 - DNA, 40 bp, synthetic construct
  source 1..40: mol_type = other DNA; note; note (original language) = 5'UTR I' truncation
tcaataacaggtcattgccgagaaaaggatagcactataa

SEQ ID NO: 186 - DNA, 29 bp, synthetic construct
  source 1..29: mol_type = other DNA; note; note (original language) = 5'UTR I' truncation
tcaataacaggtcattgccgagaaaagga

SEQ ID NO: 187 - DNA, 22 bp, synthetic construct
  source 1..22: mol_type = other DNA; note; note (original language) = 5'UTR I' truncation
tcaataacaggtcattgccgag

SEQ ID NO: 188 - DNA, 38 bp, synthetic construct
  source 1..38: mol_type = other DNA; note; note (original language) = 5'UTR I' truncation
tcaataacaggtcattgccgagaaaaggatagcactat

SEQ ID NO: 189 - DNA, 24 bp, synthetic construct
  source 1..24: mol_type = other DNA; note; note (original language) = 5'UTR I' truncation
tcaataacaggtcattgccgagaa

SEQ ID NO: 190 - DNA, 17 bp, synthetic construct
  source 1..17: mol_type = other DNA; note; note (original language) = 5'UTR I' truncation
tcaataacaggtcattg

SEQ ID NO: 191 - DNA, 32 bp, synthetic construct
  source 1..32: mol_type = other DNA; note; note (original language) = 5'UTR I' truncation
tcaataacaggtcattgccgagaaaaggatag

SEQ ID NO: 192 - DNA, 23 bp, synthetic construct
  source 1..23: mol_type = other DNA; note; note (original language) = 5'UTR I' truncation
tcaataacaggtcattgccgaga

SEQ ID NO: 193 - DNA, 15 bp, synthetic construct
  source 1..15: mol_type = other DNA; note; note (original language) = 5'UTR I' truncation
tcaataacaggtcat

SEQ ID NO: 194 - DNA, 19 bp, synthetic construct
  source 1..19: mol_type = other DNA; note; note (original language) = 5'UTR I' truncation
tcaataacaggtcattgcc

SEQ ID NO: 195 - DNA, 35 bp, synthetic construct
  source 1..35: mol_type = other DNA; note; note (original language) = 5'UTR I' truncation
tcaataacaggtcattgccgagaaaaggatagcac

SEQ ID NO: 196 - DNA, 20 bp, synthetic construct
  source 1..20: mol_type = other DNA; note; note (original language) = 5'UTR I' truncation
tcaataacaggtcattgccg